European Patent Application EP 4 711 458 A2, published March 18, 2026. Title: SELF-REPLICATING RNA AND USES THEREOF. Applicant: Seqirus Inc. The sequence listing filed with the application follows.

SEQUENCE LISTING (37 sequences)

SEQ ID NO: 1 - DNA, 3822 bp, synthetic construct
  misc_feature 1..3822: note = Nucleotide sequence of SARS-CoV-2 spike (S) protein full length wt (cleavable)
  source 1..3822: mol_type = other DNA
atgttcgtgttcctggtgctgctgcccctcgttagcagccagtgcgtgaatctgaccacccgcacccagctgccaccagcctacacaaacagcttcaccagaggagtgtattaccctgataaggtctttagatcctccgtcctgcattctacgcaggatctcttcttgccattcttcagcaacgtgacatggttccacgccatccacgtttctggcaccaacggcacaaagcgcttcgacaatcctgtgttgccgtttaacgacggcgtttacttcgccagcacagaaaagagcaacatcatccggggctggatcttcggcaccaccctggacagcaaaacccaaagcctgctcatcgtgaacaacgccaccaacgtggtgatcaaggtgtgcgagttccagttctgcaatgatccttttctgggcgtgtactatcacaagaacaacaagagctggatggaaagcgagttcagagtgtattctagcgccaacaactgcacctttgagtacgtgtcccagccctttcttatggacctggaaggcaagcagggcaacttcaagaatctgagagaattcgtgttcaagaacattgatggctacttcaagatctacagcaagcacacccctatcaacctggttcgggacctgccacaaggcttcagcgccctggaacctctggtggacctgcctatcggcatcaacatcacacggttccaaaccctgctggccctgcaccggagctacctgacccccggcgacagcagcagcggctggaccgccggcgctgccgcctattacgtgggctacctgcaacctagaaccttcctgctgaaatacaacgagaacggcacaatcaccgacgccgtggactgtgccctggaccccctgtctgagacaaagtgtaccctgaagtctttcaccgtggagaagggcatctaccagaccagcaacttccgggtgcagcctacagaatctatagtgcggttccctaacatcaccaacctgtgtccttttggcgaggtgttcaacgccactcggttcgcctctgtctacgcctggaaccggaaacggatctctaattgcgtggccgattacagcgtcctgtataactccgccagtttcagcacattcaagtgctacggcgtgtcacccaccaagctgaacgatctgtgcttcaccaatgtgtacgccgatagtttcgtgatccggggcgatgaggtgcggcagatcgcccctggacagacaggcaagatcgccgactacaactacaagctgcctgacgacttcacaggctgtgtgatcgcatggaacagcaacaacctggacagcaaggtgggcggaaactacaactacctgtacagactgttcagaaagtccaacctgaagcctttcgagagagatatatctaccgagatctaccaggccggcagcacaccctgtaatggagtggaaggctttaactgctacttccctctgcaaagctatggatttcaacctacaaatggggttggctaccagccttacagagtggtggtccttagcttcgagctgctccatgcccctgccaccgtgtgcggacctaagaagtccaccaacctggtgaaaaacaagtgcgtgaactttaattttaacggcctgaccggaacaggagtgctgacagaaagcaacaaaaagttcctgcctttccagcagttcggcagagacattgccgacaccacagatgctgttagagacccccagacgctggaaatcctggatatcaccccctgctcttttggcggcgtgagcgtgatcaccccaggcacaaacacaagcaaccaggtggctgtgctgtaccaggacgtgaactgtacagaggtccctgtggcaatccacgccgatcagctgacccctacatggcgggtgtactccactggatctaacgtgttccagacaagggccggatgcctcatcggcgctgagcacgtgaacaattcttacgagtgcgacatccctattggagcgggcatctgcgccagctaccagacacagaccaatagccctcgcagagccagaagcgtggcctcccagagcatcatcgcctacaccatgagcctgggagccgagaactctgtggcctacagcaacaacagcatcgctatccctaccaacttcaccatctctgtcaccaccgaaatcctgcccgtcagtatgaccaaaaccagcgtcgactgcaccatgtacatatgcggcgatagcaccgaatgcagcaacctgctgctgcagtatggctccttctgcacccaacttaacagagccctgactggcatcgccgtggagcaggacaagaatacccaggaggtgttcgcccaggtgaagcagatctacaagacacccccgatcaaggacttcggcggctttaatttctctcagatcctgccagacccatctaaaccctctaagcggagctttatcgaggacctgctgttcaacaaggtgactctggctgacgccggcttcatcaagcagtacggcgattgcctgggcgacattgctgctagagacctgatctgtgcccagaaattcaacggtcttactgtgctgcctcctctgctgacggatgagatgatcgcccagtacaccagcgccctgctggccggcaccatcacatccggctggacattcggcgccggcgcagccctgcagatcccttttgccatgcagatggcctaccggttcaacggaatcggagtgacacagaacgtgctctacgaaaatcagaagttgatcgccaaccagttcaacagcgccatcggcaagattcaggatagtctgagttccaccgccagcgccctgggaaagctgcaggacgtggtcaatcagaatgcccaagccctgaacaccctggtgaagcagctgagcagcaacttcggcgccatcagctctgtgctgaacgacatcctgagtagactggacaaggtggaagccgaagtgcagatcgacagattgatcaccggaagactgcaaagcctgcagacctacgtgacccagcagctgataagagctgctgaaatcagagccagcgctaatctggccgctaccaagatgagcgagtgcgttctgggccagtctaagagagtggacttctgcggaaaaggctaccacctgatgtcctttcctcagtctgccccccacggcgtggtgttcctgcacgtcacatacgtgcccgctcaagagaaaaacttcaccacggcccctgccatctgtcacgacggcaaggcccacttccccagagagggcgtgttcgtgagcaatggcacccactggtttgtgactcagagaaacttctacgagccacagattatcaccacagataacaccttcgtgtctggcaactgcgacgtggtgatcggcatcgtcaacaacacagtgtacgacccactgcaacctgagctggactcattcaaggaggaactggataagtacttcaagaatcacaccagccccgacgttgacctgggcgacatcagcggcattaacgcctctgtggtcaacatccagaaggaaatcgacagactgaatgaggtggccaagaatttgaacgagagcctgattgatctgcaggagctgggcaaatacgagcagtacatcaagtggccttggtacatctggctgggcttcatcgccgggctgatcgccatcgttatggtgacaatcatgctgtgttgcatgacaagctgttgtagctgcctgaaaggctgctgctcctgcggcagctgttgcaagtttgacgaagatgacagcgagcccgtgctgaaaggcgtcaagctgcactacacctga

SEQ ID NO: 2 - DNA, 3822 bp, synthetic construct
  misc_feature 1..3822: note = Nucleotide sequence of SARS-CoV-2 mutated spike (S) protein uncleavable (S1/S2 RRAR to QQAA mutation)
  source 1..3822: mol_type = other DNA
atgttcgtgttcctggtgctgctgcccctcgttagcagccagtgcgtgaatctgaccacccgcacccagctgccaccagcctacacaaacagcttcaccagaggagtgtattaccctgataaggtctttagatcctccgtcctgcattctacgcaggatctcttcttgccattcttcagcaacgtgacatggttccacgccatccacgtttctggcaccaacggcacaaagcgcttcgacaatcctgtgttgccgtttaacgacggcgtttacttcgccagcacagaaaagagcaacatcatccggggctggatcttcggcaccaccctggacagcaaaacccaaagcctgctcatcgtgaacaacgccaccaacgtggtgatcaaggtgtgcgagttccagttctgcaatgatccttttctgggcgtgtactatcacaagaacaacaagagctggatggaaagcgagttcagagtgtattctagcgccaacaactgcacctttgagtacgtgtcccagccctttcttatggacctggaaggcaagcagggcaacttcaagaatctgagagaattcgtgttcaagaacattgatggctacttcaagatctacagcaagcacacccctatcaacctggttcgggacctgccacaaggcttcagcgccctggaacctctggtggacctgcctatcggcatcaacatcacacggttccaaaccctgctggccctgcaccggagctacctgacccccggcgacagcagcagcggctggaccgccggcgctgccgcctattacgtgggctacctgcaacctagaaccttcctgctgaaatacaacgagaacggcacaatcaccgacgccgtggactgtgccctggaccccctgtctgagacaaagtgtaccctgaagtctttcaccgtggagaagggcatctaccagaccagcaacttccgggtgcagcctacagaatctatagtgcggttccctaacatcaccaacctgtgtccttttggcgaggtgttcaacgccactcggttcgcctctgtctacgcctggaaccggaaacggatctctaattgcgtggccgattacagcgtcctgtataactccgccagtttcagcacattcaagtgctacggcgtgtcacccaccaagctgaacgatctgtgcttcaccaatgtgtacgccgatagtttcgtgatccggggcgatgaggtgcggcagatcgcccctggacagacaggcaagatcgccgactacaactacaagctgcctgacgacttcacaggctgtgtgatcgcatggaacagcaacaacctggacagcaaggtgggcggaaactacaactacctgtacagactgttcagaaagtccaacctgaagcctttcgagagagatatatctaccgagatctaccaggccggcagcacaccctgtaatggagtggaaggctttaactgctacttccctctgcaaagctatggatttcaacctacaaatggggttggctaccagccttacagagtggtggtccttagcttcgagctgctccatgcccctgccaccgtgtgcggacctaagaagtccaccaacctggtgaaaaacaagtgcgtgaactttaattttaacggcctgaccggaacaggagtgctgacagaaagcaacaaaaagttcctgcctttccagcagttcggcagagacattgccgacaccacagatgctgttagagacccccagacgctggaaatcctggatatcaccccctgctcttttggcggcgtgagcgtgatcaccccaggcacaaacacaagcaaccaggtggctgtgctgtaccaggacgtgaactgtacagaggtccctgtggcaatccacgccgatcagctgacccctacatggcgggtgtactccactggatctaacgtgttccagacaagggccggatgcctcatcggcgctgagcacgtgaacaattcttacgagtgcgacatccctattggagcgggcatctgcgccagctaccagacacagaccaatagccctcagcaagccgctagcgtggcctcccagagcatcatcgcctacaccatgagcctgggagccgagaactctgtggcctacagcaacaacagcatcgctatccctaccaacttcaccatctctgtcaccaccgaaatcctgcccgtcagtatgaccaaaaccagcgtcgactgcaccatgtacatatgcggcgatagcaccgaatgcagcaacctgctgctgcagtatggctccttctgcacccaacttaacagagccctgactggcatcgccgtggagcaggacaagaatacccaggaggtgttcgcccaggtgaagcagatctacaagacacccccgatcaaggacttcggcggctttaatttctctcagatcctgccagacccatctaaaccctctaagcggagctttatcgaggacctgctgttcaacaaggtgactctggctgacgccggcttcatcaagcagtacggcgattgcctgggcgacattgctgctagagacctgatctgtgcccagaaattcaacggtcttactgtgctgcctcctctgctgacggatgagatgatcgcccagtacaccagcgccctgctggccggcaccatcacatccggctggacattcggcgccggcgcagccctgcagatcccttttgccatgcagatggcctaccggttcaacggaatcggagtgacacagaacgtgctctacgaaaatcagaagttgatcgccaaccagttcaacagcgccatcggcaagattcaggatagtctgagttccaccgccagcgccctgggaaagctgcaggacgtggtcaatcagaatgcccaagccctgaacaccctggtgaagcagctgagcagcaacttcggcgccatcagctctgtgctgaacgacatcctgagtagactggacaaggtggaagccgaagtgcagatcgacagattgatcaccggaagactgcaaagcctgcagacctacgtgacccagcagctgataagagctgctgaaatcagagccagcgctaatctggccgctaccaagatgagcgagtgcgttctgggccagtctaagagagtggacttctgcggaaaaggctaccacctgatgtcctttcctcagtctgccccccacggcgtggtgttcctgcacgtcacatacgtgcccgctcaagagaaaaacttcaccacggcccctgccatctgtcacgacggcaaggcccacttccccagagagggcgtgttcgtgagcaatggcacccactggtttgtgactcagagaaacttctacgagccacagattatcaccacagataacaccttcgtgtctggcaactgcgacgtggtgatcggcatcgtcaacaacacagtgtacgacccactgcaacctgagctggactcattcaaggaggaactggataagtacttcaagaatcacaccagccccgacgttgacctgggcgacatcagcggcattaacgcctctgtggtcaacatccagaaggaaatcgacagactgaatgaggtggccaagaatttgaacgagagcctgattgatctgcaggagctgggcaaatacgagcagtacatcaagtggccttggtacatctggctgggcttcatcgccgggctgatcgccatcgttatggtgacaatcatgctgtgttgcatgacaagctgttgtagctgcctgaaaggctgctgctcctgcggcagctgttgcaagtttgacgaagatgacagcgagcccgtgctgaaaggcgtcaagctgcactacacctga

SEQ ID NO: 3 - DNA, 3822 bp, synthetic construct
  misc_feature 1..3822: note = Nucleotide sequence of SARS-CoV-2 spike (S) protein uncleavable (S1/S2 RRAR to QQAA mutation and 986P/987P mutation)
  source 1..3822: mol_type = other DNA
atgttcgtgttcctggtgctgctgcccctcgttagcagccagtgcgtgaatctgaccacccgcacccagctgccaccagcctacacaaacagcttcaccagaggagtgtattaccctgataaggtctttagatcctccgtcctgcattctacgcaggatctcttcttgccattcttcagcaacgtgacatggttccacgccatccacgtttctggcaccaacggcacaaagcgcttcgacaatcctgtgttgccgtttaacgacggcgtttacttcgccagcacagaaaagagcaacatcatccggggctggatcttcggcaccaccctggacagcaaaacccaaagcctgctcatcgtgaacaacgccaccaacgtggtgatcaaggtgtgcgagttccagttctgcaatgatccttttctgggcgtgtactatcacaagaacaacaagagctggatggaaagcgagttcagagtgtattctagcgccaacaactgcacctttgagtacgtgtcccagccctttcttatggacctggaaggcaagcagggcaacttcaagaatctgagagaattcgtgttcaagaacattgatggctacttcaagatctacagcaagcacacccctatcaacctggttcgggacctgccacaaggcttcagcgccctggaacctctggtggacctgcctatcggcatcaacatcacacggttccaaaccctgctggccctgcaccggagctacctgacccccggcgacagcagcagcggctggaccgccggcgctgccgcctattacgtgggctacctgcaacctagaaccttcctgctgaaatacaacgagaacggcacaatcaccgacgccgtggactgtgccctggaccccctgtctgagacaaagtgtaccctgaagtctttcaccgtggagaagggcatctaccagaccagcaacttccgggtgcagcctacagaatctatagtgcggttccctaacatcaccaacctgtgtccttttggcgaggtgttcaacgccactcggttcgcctctgtctacgcctggaaccggaaacggatctctaattgcgtggccgattacagcgtcctgtataactccgccagtttcagcacattcaagtgctacggcgtgtcacccaccaagctgaacgatctgtgcttcaccaatgtgtacgccgatagtttcgtgatccggggcgatgaggtgcggcagatcgcccctggacagacaggcaagatcgccgactacaactacaagctgcctgacgacttcacaggctgtgtgatcgcatggaacagcaacaacctggacagcaaggtgggcggaaactacaactacctgtacagactgttcagaaagtccaacctgaagcctttcgagagagatatatctaccgagatctaccaggccggcagcacaccctgtaatggagtggaaggctttaactgctacttccctctgcaaagctatggatttcaacctacaaatggggttggctaccagccttacagagtggtggtccttagcttcgagctgctccatgcccctgccaccgtgtgcggacctaagaagtccaccaacctggtgaaaaacaagtgcgtgaactttaattttaacggcctgaccggaacaggagtgctgacagaaagcaacaaaaagttcctgcctttccagcagttcggcagagacattgccgacaccacagatgctgttagagacccccagacgctggaaatcctggatatcaccccctgctcttttggcggcgtgagcgtgatcaccccaggcacaaacacaagcaaccaggtggctgtgctgtaccaggacgtgaactgtacagaggtccctgtggcaatccacgccgatcagctgacccctacatggcgggtgtactccactggatctaacgtgttccagacaagggccggatgcctcatcggcgctgagcacgtgaacaattcttacgagtgcgacatccctattggagcgggcatctgcgccagctaccagacacagaccaatagccctcagcaagccgctagcgtggcctcccagagcatcatcgcctacaccatgagcctgggagccgagaactctgtggcctacagcaacaacagcatcgctatccctaccaacttcaccatctctgtcaccaccgaaatcctgcccgtcagtatgaccaaaaccagcgtcgactgcaccatgtacatatgcggcgatagcaccgaatgcagcaacctgctgctgcagtatggctccttctgcacccaacttaacagagccctgactggcatcgccgtggagcaggacaagaatacccaggaggtgttcgcccaggtgaagcagatctacaagacacccccgatcaaggacttcggcggctttaatttctctcagatcctgccagacccatctaaaccctctaagcggagctttatcgaggacctgctgttcaacaaggtgactctggctgacgccggcttcatcaagcagtacggcgattgcctgggcgacattgctgctagagacctgatctgtgcccagaaattcaacggtcttactgtgctgcctcctctgctgacggatgagatgatcgcccagtacaccagcgccctgctggccggcaccatcacatccggctggacattcggcgccggcgcagccctgcagatcccttttgccatgcagatggcctaccggttcaacggaatcggagtgacacagaacgtgctctacgaaaatcagaagttgatcgccaaccagttcaacagcgccatcggcaagattcaggatagtctgagttccaccgccagcgccctgggaaagctgcaggacgtggtcaatcagaatgcccaagccctgaacaccctggtgaagcagctgagcagcaacttcggcgccatcagctctgtgctgaacgacatcctgagtagactggacccacctgaagccgaagtgcagatcgacagattgatcaccggaagactgcaaagcctgcagacctacgtgacccagcagctgataagagctgctgaaatcagagccagcgctaatctggccgctaccaagatgagcgagtgcgttctgggccagtctaagagagtggacttctgcggaaaaggctaccacctgatgtcctttcctcagtctgccccccacggcgtggtgttcctgcacgtcacatacgtgcccgctcaagagaaaaacttcaccacggcccctgccatctgtcacgacggcaaggcccacttccccagagagggcgtgttcgtgagcaatggcacccactggtttgtgactcagagaaacttctacgagccacagattatcaccacagataacaccttcgtgtctggcaactgcgacgtggtgatcggcatcgtcaacaacacagtgtacgacccactgcaacctgagctggactcattcaaggaggaactggataagtacttcaagaatcacaccagccccgacgttgacctgggcgacatcagcggcattaacgcctctgtggtcaacatccagaaggaaatcgacagactgaatgaggtggccaagaatttgaacgagagcctgattgatctgcaggagctgggcaaatacgagcagtacatcaagtggccttggtacatctggctgggcttcatcgccgggctgatcgccatcgttatggtgacaatcatgctgtgttgcatgacaagctgttgtagctgcctgaaaggctgctgctcctgcggcagctgttgcaagtttgacgaagatgacagcgagcccgtgctgaaaggcgtcaagctgcactacacctga

SEQ ID NO: 4 - DNA, 3822 bp, synthetic construct
  misc_feature 1..3822: note = Nucleotide sequence of SARS-CoV-2 modified spike (S) protein uncleavable (S1/S2 RRAR to QQAA mutation and D614G mutation)
  source 1..3822: mol_type = other DNA
atgttcgtgttcctggtgctgctgcccctcgttagcagccagtgcgtgaatctgaccacccgcacccagctgccaccagcctacacaaacagcttcaccagaggagtgtattaccctgataaggtctttagatcctccgtcctgcattctacgcaggatctcttcttgccattcttcagcaacgtgacatggttccacgccatccacgtttctggcaccaacggcacaaagcgcttcgacaatcctgtgttgccgtttaacgacggcgtttacttcgccagcacagaaaagagcaacatcatccggggctggatcttcggcaccaccctggacagcaaaacccaaagcctgctcatcgtgaacaacgccaccaacgtggtgatcaaggtgtgcgagttccagttctgcaatgatccttttctgggcgtgtactatcacaagaacaacaagagctggatggaaagcgagttcagagtgtattctagcgccaacaactgcacctttgagtacgtgtcccagccctttcttatggacctggaaggcaagcagggcaacttcaagaatctgagagaattcgtgttcaagaacattgatggctacttcaagatctacagcaagcacacccctatcaacctggttcgggacctgccacaaggcttcagcgccctggaacctctggtggacctgcctatcggcatcaacatcacacggttccaaaccctgctggccctgcaccggagctacctgacccccggcgacagcagcagcggctggaccgccggcgctgccgcctattacgtgggctacctgcaacctagaaccttcctgctgaaatacaacgagaacggcacaatcaccgacgccgtggactgtgccctggaccccctgtctgagacaaagtgtaccctgaagtctttcaccgtggagaagggcatctaccagaccagcaacttccgggtgcagcctacagaatctatagtgcggttccctaacatcaccaacctgtgtccttttggcgaggtgttcaacgccactcggttcgcctctgtctacgcctggaaccggaaacggatctctaattgcgtggccgattacagcgtcctgtataactccgccagtttcagcacattcaagtgctacggcgtgtcacccaccaagctgaacgatctgtgcttcaccaatgtgtacgccgatagtttcgtgatccggggcgatgaggtgcggcagatcgcccctggacagacaggcaagatcgccgactacaactacaagctgcctgacgacttcacaggctgtgtgatcgcatggaacagcaacaacctggacagcaaggtgggcggaaactacaactacctgtacagactgttcagaaagtccaacctgaagcctttcgagagagatatatctaccgagatctaccaggccggcagcacaccctgtaatggagtggaaggctttaactgctacttccctctgcaaagctatggatttcaacctacaaatggggttggctaccagccttacagagtggtggtccttagcttcgagctgctccatgcccctgccaccgtgtgcggacctaagaagtccaccaacctggtgaaaaacaagtgcgtgaactttaattttaacggcctgaccggaacaggagtgctgacagaaagcaacaaaaagttcctgcctttccagcagttcggcagagacattgccgacaccacagatgctgttagagacccccagacgctggaaatcctggatatcaccccctgctcttttggcggcgtgagcgtgatcaccccaggcacaaacacaagcaaccaggtggctgtgctgtaccagggcgtgaactgtacagaggtccctgtggcaatccacgccgatcagctgacccctacatggcgggtgtactccactggatctaacgtgttccagacaagggccggatgcctcatcggcgctgagcacgtgaacaattcttacgagtgcgacatccctattggagcgggcatctgcgccagctaccagacacagaccaatagccctcagcaagccgctagcgtggcctcccagagcatcatcgcctacaccatgagcctgggagccgagaactctgtggcctacagcaacaacagcatcgctatccctaccaacttcaccatctctgtcaccaccgaaatcctgcccgtcagtatgaccaaaaccagcgtcgactgcaccatgtacatatgcggcgatagcaccgaatgcagcaacctgctgctgcagtatggctccttctgcacccaacttaacagagccctgactggcatcgccgtggagcaggacaagaatacccaggaggtgttcgcccaggtgaagcagatctacaagacacccccgatcaaggacttcggcggctttaatttctctcagatcctgccagacccatctaaaccctctaagcggagctttatcgaggacctgctgttcaacaaggtgactctggctgacgccggcttcatcaagcagtacggcgattgcctgggcgacattgctgctagagacctgatctgtgcccagaaattcaacggtcttactgtgctgcctcctctgctgacggatgagatgatcgcccagtacaccagcgccctgctggccggcaccatcacatccggctggacattcggcgccggcgcagccctgcagatcccttttgccatgcagatggcctaccggttcaacggaatcggagtgacacagaacgtgctctacgaaaatcagaagttgatcgccaaccagttcaacagcgccatcggcaagattcaggatagtctgagttccaccgccagcgccctgggaaagctgcaggacgtggtcaatcagaatgcccaagccctgaacaccctggtgaagcagctgagcagcaacttcggcgccatcagctctgtgctgaacgacatcctgagtagactggacaaggtggaagccgaagtgcagatcgacagattgatcaccggaagactgcaaagcctgcagacctacgtgacccagcagctgataagagctgctgaaatcagagccagcgctaatctggccgctaccaagatgagcgagtgcgttctgggccagtctaagagagtggacttctgcggaaaaggctaccacctgatgtcctttcctcagtctgccccccacggcgtggtgttcctgcacgtcacatacgtgcccgctcaagagaaaaacttcaccacggcccctgccatctgtcacgacggcaaggcccacttccccagagagggcgtgttcgtgagcaatggcacccactggtttgtgactcagagaaacttctacgagccacagattatcaccacagataacaccttcgtgtctggcaactgcgacgtggtgatcggcatcgtcaacaacacagtgtacgacccactgcaacctgagctggactcattcaaggaggaactggataagtacttcaagaatcacaccagccccgacgttgacctgggcgacatcagcggcattaacgcctctgtggtcaacatccagaaggaaatcgacagactgaatgaggtggccaagaatttgaacgagagcctgattgatctgcaggagctgggcaaatacgagcagtacatcaagtggccttggtacatctggctgggcttcatcgccgggctgatcgccatcgttatggtgacaatcatgctgtgttgcatgacaagctgttgtagctgcctgaaaggctgctgctcctgcggcagctgttgcaagtttgacgaagatgacagcgagcccgtgctgaaaggcgtcaagctgcactacacctga

SEQ ID NO: 5 - DNA, 3822 bp, synthetic construct
  misc_feature 1..3822: note = Nucleotide sequence of SARS-CoV-2 spike (S) protein uncleavable (S1/S2 RRAR to QQAA mutation and S2' mutation)
  source 1..3822: mol_type = other DNA
atgttcgtgttcctggtgctgctgcccctcgttagcagccagtgcgtgaatctgaccacccgcacccagctgccaccagcctacacaaacagcttcaccagaggagtgtattaccctgataaggtctttagatcctccgtcctgcattctacgcaggatctcttcttgccattcttcagcaacgtgacatggttccacgccatccacgtttctggcaccaacggcacaaagcgcttcgacaatcctgtgttgccgtttaacgacggcgtttacttcgccagcacagaaaagagcaacatcatccggggctggatcttcggcaccaccctggacagcaaaacccaaagcctgctcatcgtgaacaacgccaccaacgtggtgatcaaggtgtgcgagttccagttctgcaatgatccttttctgggcgtgtactatcacaagaacaacaagagctggatggaaagcgagttcagagtgtattctagcgccaacaactgcacctttgagtacgtgtcccagccctttcttatggacctggaaggcaagcagggcaacttcaagaatctgagagaattcgtgttcaagaacattgatggctacttcaagatctacagcaagcacacccctatcaacctggttcgggacctgccacaaggcttcagcgccctggaacctctggtggacctgcctatcggcatcaacatcacacggttccaaaccctgctggccctgcaccggagctacctgacccccggcgacagcagcagcggctggaccgccggcgctgccgcctattacgtgggctacctgcaacctagaaccttcctgctgaaatacaacgagaacggcacaatcaccgacgccgtggactgtgccctggaccccctgtctgagacaaagtgtaccctgaagtctttcaccgtggagaagggcatctaccagaccagcaacttccgggtgcagcctacagaatctatagtgcggttccctaacatcaccaacctgtgtccttttggcgaggtgttcaacgccactcggttcgcctctgtctacgcctggaaccggaaacggatctctaattgcgtggccgattacagcgtcctgtataactccgccagtttcagcacattcaagtgctacggcgtgtcacccaccaagctgaacgatctgtgcttcaccaatgtgtacgccgatagtttcgtgatccggggcgatgaggtgcggcagatcgcccctggacagacaggcaagatcgccgactacaactacaagctgcctgacgacttcacaggctgtgtgatcgcatggaacagcaacaacctggacagcaaggtgggcggaaactacaactacctgtacagactgttcagaaagtccaacctgaagcctttcgagagagatatatctaccgagatctaccaggccggcagcacaccctgtaatggagtggaaggctttaactgctacttccctctgcaaagctatggatttcaacctacaaatggggttggctaccagccttacagagtggtggtccttagcttcgagctgctccatgcccctgccaccgtgtgcggacctaagaagtccaccaacctggtgaaaaacaagtgcgtgaactttaattttaacggcctgaccggaacaggagtgctgacagaaagcaacaaaaagttcctgcctttccagcagttcggcagagacattgccgacaccacagatgctgttagagacccccagacgctggaaatcctggatatcaccccctgctcttttggcggcgtgagcgtgatcaccccaggcacaaacacaagcaaccaggtggctgtgctgtaccaggacgtgaactgtacagaggtccctgtggcaatccacgccgatcagctgacccctacatggcgggtgtactccactggatctaacgtgttccagacaagggccggatgcctcatcggcgctgagcacgtgaacaattcttacgagtgcgacatccctattggagcgggcatctgcgccagctaccagacacagaccaatagccctcagcaagccgctagcgtggcctcccagagcatcatcgcctacaccatgagcctgggagccgagaactctgtggcctacagcaacaacagcatcgctatccctaccaacttcaccatctctgtcaccaccgaaatcctgcccgtcagtatgaccaaaaccagcgtcgactgcaccatgtacatatgcggcgatagcaccgaatgcagcaacctgctgctgcagtatggctccttctgcacccaacttaacagagccctgactggcatcgccgtggagcaggacaagaatacccaggaggtgttcgcccaggtgaagcagatctacaagacacccccgatcaaggacttcggcggctttaatttctctcagatcctgccagacccatctaaaccctctaagaacagctttatcgaggacctgctgttcaacaaggtgactctggctgacgccggcttcatcaagcagtacggcgattgcctgggcgacattgctgctagagacctgatctgtgcccagaaattcaacggtcttactgtgctgcctcctctgctgacggatgagatgatcgcccagtacaccagcgccctgctggccggcaccatcacatccggctggacattcggcgccggcgcagccctgcagatcccttttgccatgcagatggcctaccggttcaacggaatcggagtgacacagaacgtgctctacgaaaatcagaagttgatcgccaaccagttcaacagcgccatcggcaagattcaggatagtctgagttccaccgccagcgccctgggaaagctgcaggacgtggtcaatcagaatgcccaagccctgaacaccctggtgaagcagctgagcagcaacttcggcgccatcagctctgtgctgaacgacatcctgagtagactggacaaggtggaagccgaagtgcagatcgacagattgatcaccggaagactgcaaagcctgcagacctacgtgacccagcagctgataagagctgctgaaatcagagccagcgctaatctggccgctaccaagatgagcgagtgcgttctgggccagtctaagagagtggacttctgcggaaaaggctaccacctgatgtcctttcctcagtctgccccccacggcgtggtgttcctgcacgtcacatacgtgcccgctcaagagaaaaacttcaccacggcccctgccatctgtcacgacggcaaggcccacttccccagagagggcgtgttcgtgagcaatggcacccactggtttgtgactcagagaaacttctacgagccacagattatcaccacagataacaccttcgtgtctggcaactgcgacgtggtgatcggcatcgtcaacaacacagtgtacgacccactgcaacctgagctggactcattcaaggaggaactggataagtacttcaagaatcacaccagccccgacgttgacctgggcgacatcagcggcattaacgcctctgtggtcaacatccagaaggaaatcgacagactgaatgaggtggccaagaatttgaacgagagcctgattgatctgcaggagctgggcaaatacgagcagtacatcaagtggccttggtacatctggctgggcttcatcgccgggctgatcgccatcgttatggtgacaatcatgctgtgttgcatgacaagctgttgtagctgcctgaaaggctgctgctcctgcggcagctgttgcaagtttgacgaagatgacagcgagcccgtgctgaaaggcgtcaagctgcactacacctga

SEQ ID NO: 6 - DNA, 3822 bp, synthetic construct
  misc_feature 1..3822: note = Nucleotide sequence of SARS-CoV-2 modified spike (S) protein uncleavable (S1/S2 RRAR to QQAA mutation and D614G mutation and S2' mutation)
  source 1..3822: mol_type = other DNA
atgttcgtgttcctggtgctgctgcccctcgttagcagccagtgcgtgaatctgaccacccgcacccagctgccaccagcctacacaaacagcttcaccagaggagtgtattaccctgataaggtctttagatcctccgtcctgcattctacgcaggatctcttcttgccattcttcagcaacgtgacatggttccacgccatccacgtttctggcaccaacggcacaaagcgcttcgacaatcctgtgttgccgtttaacgacggcgtttacttcgccagcacagaaaagagcaacatcatccggggctggatcttcggcaccaccctggacagcaaaacccaaagcctgctcatcgtgaacaacgccaccaacgtggtgatcaaggtgtgcgagttccagttctgcaatgatccttttctgggcgtgtactatcacaagaacaacaagagctggatggaaagcgagttcagagtgtattctagcgccaacaactgcacctttgagtacgtgtcccagccctttcttatggacctggaaggcaagcagggcaacttcaagaatctgagagaattcgtgttcaagaacattgatggctacttcaagatctacagcaagcacacccctatcaacctggttcgggacctgccacaaggcttcagcgccctggaacctctggtggacctgcctatcggcatcaacatcacacggttccaaaccctgctggccctgcaccggagctacctgacccccggcgacagcagcagcggctggaccgccggcgctgccgcctattacgtgggctacctgcaacctagaaccttcctgctgaaatacaacgagaacggcacaatcaccgacgccgtggactgtgccctggaccccctgtctgagacaaagtgtaccctgaagtctttcaccgtggagaagggcatctaccagaccagcaacttccgggtgcagcctacagaatctatagtgcggttccctaacatcaccaacctgtgtccttttggcgaggtgttcaacgccactcggttcgcctctgtctacgcctggaaccggaaacggatctctaattgcgtggccgattacagcgtcctgtataactccgccagtttcagcacattcaagtgctacggcgtgtcacccaccaagctgaacgatctgtgcttcaccaatgtgtacgccgatagtttcgtgatccggggcgatgaggtgcggcagatcgcccctggacagacaggcaagatcgccgactacaactacaagctgcctgacgacttcacaggctgtgtgatcgcatggaacagcaacaacctggacagcaaggtgggcggaaactacaactacctgtacagactgttcagaaagtccaacctgaagcctttcgagagagatatatctaccgagatctaccaggccggcagcacaccctgtaatggagtggaaggctttaactgctacttccctctgcaaagctatggatttcaacctacaaatggggttggctaccagccttacagagtggtggtccttagcttcgagctgctccatgcccctgccaccgtgtgcggacctaagaagtccaccaacctggtgaaaaacaagtgcgtgaactttaattttaacggcctgaccggaacaggagtgctgacagaaagcaacaaaaagttcctgcctttccagcagttcggcagagacattgccgacaccacagatgctgttagagacccccagacgctggaaatcctggatatcaccccctgctcttttggcggcgtgagcgtgatcaccccaggcacaaacacaagcaaccaggtggctgtgctgtaccagggcgtgaactgtacagaggtccctgtggcaatccacgccgatcagctgacccctacatggcgggtgtactccactggatctaacgtgttccagacaagggccggatgcctcatcggcgctgagcacgtgaacaattcttacgagtgcgacatccctattggagcgggcatctgcgccagctaccagacacagaccaatagccctcagcaagccgctagcgtggcctcccagagcatcatcgcctacaccatgagcctgggagccgagaactctgtggcctacagcaacaacagcatcgctatccctaccaacttcaccatctctgtcaccaccgaaatcctgcccgtcagtatgaccaaaaccagcgtcgactgcaccatgtacatatgcggcgatagcaccgaatgcagcaacctgctgctgcagtatggctccttctgcacccaacttaacagagccctgactggcatcgccgtggagcaggacaagaatacccaggaggtgttcgcccaggtgaagcagatctacaagacacccccgatcaaggacttcggcggctttaatttctctcagatcctgccagacccatctaaaccctctaagaacagctttatcgaggacctgctgttcaacaaggtgactctggctgacgccggcttcatcaagcagtacggcgattgcctgggcgacattgctgctagagacctgatctgtgcccagaaattcaacggtcttactgtgctgcctcctctgctgacggatgagatgatcgcccagtacaccagcgccctgctggccggcaccatcacatccggctggacattcggcgccggcgcagccctgcagatcccttttgccatgcagatggcctaccggttcaacggaatcggagtgacacagaacgtgctctacgaaaatcagaagttgatcgccaaccagttcaacagcgccatcggcaagattcaggatagtctgagttccaccgccagcgccctgggaaagctgcaggacgtggtcaatcagaatgcccaagccctgaacaccctggtgaagcagctgagcagcaacttcggcgccatcagctctgtgctgaacgacatcctgagtagactggacaaggtggaagccgaagtgcagatcgacagattgatcaccggaagactgcaaagcctgcagacctacgtgacccagcagctgataagagctgctgaaatcagagccagcgctaatctggccgctaccaagatgagcgagtgcgttctgggccagtctaagagagtggacttctgcggaaaaggctaccacctgatgtcctttcctcagtctgccccccacggcgtggtgttcctgcacgtcacatacgtgcccgctcaagagaaaaacttcaccacggcccctgccatctgtcacgacggcaaggcccacttccccagagagggcgtgttcgtgagcaatggcacccactggtttgtgactcagagaaacttctacgagccacagattatcaccacagataacaccttcgtgtctggcaactgcgacgtggtgatcggcatcgtcaacaacacagtgtacgacccactgcaacctgagctggactcattcaaggaggaactggataagtacttcaagaatcacaccagccccgacgttgacctgggcgacatcagcggcattaacgcctctgtggtcaacatccagaaggaaatcgacagactgaatgaggtggccaagaatttgaacgagagcctgattgatctgcaggagctgggcaaatacgagcagtacatcaagtggccttggtacatctggctgggcttcatcgccgggctgatcgccatcgttatggtgacaatcatgctgtgttgcatgacaagctgttgtagctgcctgaaaggctgctgctcctgcggcagctgttgcaagtttgacgaagatgacagcgagcccgtgctgaaaggcgtcaagctgcactacacctga

SEQ ID NO: 7 - DNA, 3822 bp, synthetic construct
  misc_feature 1..3822: note = Nucleotide sequence of SARS-CoV-2 spike (S) protein cleavable (D614G mutation)
  source 1..3822: mol_type = other DNA
atgttcgtgttcctggtgctgctgcccctcgttagcagccagtgcgtgaatctgaccacccgcacccagctgccaccagcctacacaaacagcttcaccagaggagtgtattaccctgataaggtctttagatcctccgtcctgcattctacgcaggatctcttcttgccattcttcagcaacgtgacatggttccacgccatccacgtttctggcaccaacggcacaaagcgcttcgacaatcctgtgttgccgtttaacgacggcgtttacttcgccagcacagaaaagagcaacatcatccggggctggatcttcggcaccaccctggacagcaaaacccaaagcctgctcatcgtgaacaacgccaccaacgtggtgatcaaggtgtgcgagttccagttctgcaatgatccttttctgggcgtgtactatcacaagaacaacaagagctggatggaaagcgagttcagagtgtattctagcgccaacaactgcacctttgagtacgtgtcccagccctttcttatggacctggaaggcaagcagggcaacttcaagaatctgagagaattcgtgttcaagaacattgatggctacttcaagatctacagcaagcacacccctatcaacctggttcgggacctgccacaaggcttcagcgccctggaacctctggtggacctgcctatcggcatcaacatcacacggttccaaaccctgctggccctgcaccggagctacctgacccccggcgacagcagcagcggctggaccgccggcgctgccgcctattacgtgggctacctgcaacctagaaccttcctgctgaaatacaacgagaacggcacaatcaccgacgccgtggactgtgccctggaccccctgtctgagacaaagtgtaccctgaagtctttcaccgtggagaagggcatctaccagaccagcaacttccgggtgcagcctacagaatctatagtgcggttccctaacatcaccaacctgtgtccttttggcgaggtgttcaacgccactcggttcgcctctgtctacgcctggaaccggaaacggatctctaattgcgtggccgattacagcgtcctgtataactccgccagtttcagcacattcaagtgctacggcgtgtcacccaccaagctgaacgatctgtgcttcaccaatgtgtacgccgatagtttcgtgatccggggcgatgaggtgcggcagatcgcccctggacagacaggcaagatcgccgactacaactacaagctgcctgacgacttcacaggctgtgtgatcgcatggaacagcaacaacctggacagcaaggtgggcggaaactacaactacctgtacagactgttcagaaagtccaacctgaagcctttcgagagagatatatctaccgagatctaccaggccggcagcacaccctgtaatggagtggaaggctttaactgctacttccctctgcaaagctatggatttcaacctacaaatggggttggctaccagccttacagagtggtggtccttagcttcgagctgctccatgcccctgccaccgtgtgcggacctaagaagtccaccaacctggtgaaaaacaagtgcgtgaactttaattttaacggcctgaccggaacaggagtgctgacagaaagcaacaaaaagttcctgcctttccagcagttcggcagagacattgccgacaccacagatgctgttagagacccccagacgctggaaatcctggatatcaccccctgctcttttggcggcgtgagcgtgatcaccccaggcacaaacacaagcaaccaggtggctgtgctgtaccagggcgtgaactgtacagaggtccctgtggcaatccacgccgatcagctgacccctacatggcgggtgtactccactggatctaacgtgttccagacaagggccggatgcctcatcggcgctgagcacgtgaacaattcttacgagtgcgacatccctattggagcgggcatctgcgccagctaccagacacagaccaatagccctcgcagagccagaagcgtggcctcccagagcatcatcgcctacaccatgagcctgggagccgagaactctgtggcctacagcaacaacagcatcgctatccctaccaacttcaccatctctgtcaccaccgaaatcctgcccgtcagtatgaccaaaaccagcgtcgactgcaccatgtacatatgcggcgatagcaccgaatgcagcaacctgctgctgcagtatggctccttctgcacccaacttaacagagccctgactggcatcgccgtggagcaggacaagaatacccaggaggtgttcgcccaggtgaagcagatctacaagacacccccgatcaaggacttcggcggctttaatttctctcagatcctgccagacccatctaaaccctctaagcggagctttatcgaggacctgctgttcaacaaggtgactctggctgacgccggcttcatcaagcagtacggcgattgcctgggcgacattgctgctagagacctgatctgtgcccagaaattcaacggtcttactgtgctgcctcctctgctgacggatgagatgatcgcccagtacaccagcgccctgctggccggcaccatcacatccggctggacattcggcgccggcgcagccctgcagatcccttttgccatgcagatggcctaccggttcaacggaatcggagtgacacagaacgtgctctacgaaaatcagaagttgatcgccaaccagttcaacagcgccatcggcaagattcaggatagtctgagttccaccgccagcgccctgggaaagctgcaggacgtggtcaatcagaatgcccaagccctgaacaccctggtgaagcagctgagcagcaacttcggcgccatcagctctgtgctgaacgacatcctgagtagactggacaaggtggaagccgaagtgcagatcgacagattgatcaccggaagactgcaaagcctgcagacctacgtgacccagcagctgataagagctgctgaaatcagagccagcgctaatctggccgctaccaagatgagcgagtgcgttctgggccagtctaagagagtggacttctgcggaaaaggctaccacctgatgtcctttcctcagtctgccccccacggcgtggtgttcctgcacgtcacatacgtgcccgctcaagagaaaaacttcaccacggcccctgccatctgtcacgacggcaaggcccacttccccagagagggcgtgttcgtgagcaatggcacccactggtttgtgactcagagaaacttctacgagccacagattatcaccacagataacaccttcgtgtctggcaactgcgacgtggtgatcggcatcgtcaacaacacagtgtacgacccactgcaacctgagctggactcattcaaggaggaactggataagtacttcaagaatcacaccagccccgacgttgacctgggcgacatcagcggcattaacgcctctgtggtcaacatccagaaggaaatcgacagactgaatgaggtggccaagaatttgaacgagagcctgattgatctgcaggagctgggcaaatacgagcagtacatcaagtggccttggtacatctggctgggcttcatcgccgggctgatcgccatcgttatggtgacaatcatgctgtgttgcatgacaagctgttgtagctgcctgaaaggctgctgctcctgcggcagctgttgcaagtttgacgaagatgacagcgagcccgtgctgaaaggcgtcaagctgcactacacctga

SEQ ID NO: 8 - DNA, 1260 bp, synthetic construct
  misc_feature 1..1260: note = Nucleotide sequence of SARS-CoV-2 nucleocapsid (N) protein full length wt
  source 1..1260: mol_type = other DNA
atgagcgacaacggacctcagaaccagagaaatgcccctagaatcacctttggcggacctagcgacagcaccggcagcaaccagaatggcgagagaagcggcgccagatctaagcagcggcgtccacagggactgcccaacaacaccgccagctggttcaccgccctcacccagcacggcaaagaggacctgaagttcccccggggacagggcgtgccaatcaacacaaactctagccccgacgaccagatcggctactatagacgggccaccagaaggatcagaggaggtgatggcaagatgaaggacctgagccctagatggtacttctactacctgggcacaggcccagaagccggcctgccttacggcgccaacaaggacggcatcatctgggtcgccaccgagggcgctctcaacacccctaaggaccacattggaactcggaaccccgctaataacgccgctatcgtgctgcagctgcctcagggcacgaccctgcccaagggcttctacgccgaaggcagcagaggcggcagccaggcctctagccggtccagctctcggagcagaaacagcagcagaaactccacccctggcagcagccgcggcaccagccccgccagaatggccggaaatggcggcgatgccgctctggccctgctgctgctggatagactgaaccagctggaatccaagatgtctggcaagggccagcagcaacagggccagaccgtgaccaagaaaagcgcagctgaagcctctaaaaaacctcggcagaagcggaccgccacaaaggcttacaacgtgacacaggcctttggcagaagaggacctgagcagacacagggcaacttcggcgaccaggagctgatccggcagggcacagactacaagcattggcctcagatcgcccagttcgcccctagtgccagcgccttcttcggcatgagccggatcggcatggaagtgacccctagcggcacatggctgacctacaccggcgccatcaagctggacgataaggaccccaattttaaggaccaagtgatcctgctgaacaagcacatcgacgcctataagaccttcccacctacagagcctaagaaagataagaaaaagaaggccgacgagacacaagccctgccccagagacagaaaaagcaacaaacagtgaccctgctgcctgccgctgatctggatgacttcagcaagcagctgcagcaatctatgagctccgccgatagcacccaggcctga

SEQ ID NO: 9 - DNA, 49 bp, synthetic construct
  misc_feature 1..49: note = Nucleotide sequence of alphavirus native subgenomic promoter
  source 1..49: mol_type = other DNA
ctctctacggctaacctgaatggactacgacatagtctagtccgccaag

SEQ ID NO: 10 - DNA, 14014 bp, synthetic construct
  misc_feature 1..14014: note = Nucleotide sequence of construct Co5
  source 1..14014: mol_type = other DNA
ataggcggcgcatgagagaagcccagaccaattacctacccaaaatggagaaagttcacgttgacatcgaggaagacagcccattcctcagagctttgcagcggagcttcccgcagtttgaggtagaagccaagcaggtcactgataatgaccatgctaatgccagagcgttttcgcatctggcttcaaaactgatcgaaacggaggtggacccatccgacacgatccttgacattggaagtgcgcccgcccgcagaatgtattctaagcacaagtatcattgtatctgtccgatgagatgtgcggaagatccggacagattgtataagtatgcaactaagctgaagaaaaactgtaaggaaataactgataaggaattggacaagaaaatgaaggagctcgccgccgtcatgagcgaccctgacctggaaactgagactatgtgcctccacgacgacgagtcgtgtcgctacgaagggcaagtcgctgtttaccaggatgtatacgcggttgacggaccgacaagtctctatcaccaagccaataagggagttagagtcgcctactggataggctttgacaccaccccttttatgtttaagaacttggctggagcatatccatcatactctaccaactgggccgacgaaaccgtgttaacggctcgtaacataggcctatgcagctctgacgttatggagcggtcacgtagagggatgtccattcttagaaagaagtatttgaaaccatccaacaatgttctattctctgttggctcgaccatctaccacgagaagagggacttactgaggagctggcacctgccgtctgtatttcacttacgtggcaagcaaaattacacatgtcggtgtgagactatagttagttgcgacgggtacgtcgttaaaagaatagctatcagtccaggcctgtatgggaagccttcaggctatgctgctacgatgcaccgcgagggattcttgtgctgcaaagtgacagacacattgaacggggagagggtctcttttcccgtgtgcacgtatgtgccagctacattgtgtgaccaaatgactggcatactggcaacagatgtcagtgcggacgacgcgcaaaaactgctggttgggctcaaccagcgtatagtcgtcaacggtcgcacccagagaaacaccaataccatgaaaaattaccttttgcccgtagtggcccaggcatttgctaggtgggcaaaggaatataaggaagatcaagaagatgaaaggccactaggactacgagatagacagttagtcatggggtgttgttgggcttttagaaggcacaagataacatctatttataagcgcccggatacccaaaccatcatcaaagtgaacagcgatttccactcattcgtgctgcccaggataggcagtaacacattggagatcgggctgagaacaagaatcaggaaaatgttagaggagcacaaggagccgtcacctctcattaccgccgaggacgtacaagaagctaagtgcgcagccgatgaggctaaggaggtgcgtgaagccgaggagttgcgcgcagctctaccacctttggcagctgatgttgaggagcccactctggaagccgatgtcgacttgatgttacaagaggctggggccggctcagtggagacacctcgtggcttgataaaggttaccagctacgatggcgaggacaagatcggctcttacgctgtgctttctccgcaggctgtactcaagagtgaaaaattatcttgcatccaccctctcgctgaacaagtcatagtgataacacactctggccgaaaagggcgttatgccgtggaaccataccatggtaaagtagtggtgccagagggacatgcaatacccgtccaggactttcaagctctgagtgaaagtgccaccattgtgtacaacgaacgtgagttcgtaaacaggtacctgcaccatattgccacacatggaggagcgctgaacactgatgaagaatattacaaaactgtcaagcccagcgagcacgacggcgaatacctgtacgacatcgacaggaaacagtgcgtcaagaaagaactagtcactgggctagggctcacaggcgagctggtggatcctcccttccatgaattcgcctacgagagtctgagaacacgaccagccgctccttaccaagtaccaaccataggggtgtatggcgtgccaggatcaggcaagtctggcatcattaaaagcgcagtcaccaaaaaagatctagtggtgagcgccaagaaagaaaactgtgcagaaattataagggacgtcaagaaaatgaaagggctggacgtcaatgccagaactgtggactcagtgctcttgaatggatgcaaacaccccgtagagaccctgtatattgacgaagcttttgcttgtcatgcaggtactctcagagcgctcatagccattataagacctaaaaaggcagtgctctgcggggatcccaaacagtgcggtttttttaacatgatgtgcctgaaagtgcattttaaccacgagatttgcacacaagtcttccacaaaagcatctctcgccgttgcactaaatctgtgacttcggtcgtctcaaccttgttttacgacaaaaaaatgagaacgacgaatccgaaagagactaagattgtgattgacactaccggcagtaccaaacctaagcaggacgatctcattctcacttgtttcagagggtgggtgaagcagttgcaaatagattacaaaggcaacgaaataatgacggcagctgcctctcaagggctgacccgtaaaggtgtgtatgccgttcggtacaaggtgaatgaaaatcctctgtacgcacccacctcagaacatgtgaacgtcctactgacccgcacggaggaccgcatcgtgtggaaaacactagccggcgacccatggataaaaacactgactgccaagtaccctgggaatttcactgccacgatagaggagtggcaagcagagcatgatgccatcatgaggcacatcttggagagaccggaccctaccgacgtcttccagaataaggcaaacgtgtgttgggccaaggctttagtgccggtgctgaagaccgctggcatagacatgaccactgaacaatggaacactgtggattattttgaaacggacaaagctcactcagcagagatagtattgaaccaactatgcgtgaggttctttggactcgatctggactccggtctattttctgcacccactgttccgttatccattaggaataatcactgggataactccccgtcgcctaacatgtacgggctgaataaagaagtggtccgtcagctctctcgcaggtacccacaactgcctcgggcagttgccactggaagagtctatgacatgaacactggtacactgcgcaattatgatccgcgcataaacctagtacctgtaaacagaagactgcctcatgctttagtcctccaccataatgaacacccacagagtgacttttcttcattcgtcagcaaattgaagggcagaactgtcctggtggtcggggaaaagttgtccgtcccaggcaaaatggttgactggttgtcagaccggcctgaggctaccttcagagctcggctggatttaggcatcccaggtgatgtgcccaaatatgacataatatttgttaatgtgaggaccccatataaataccatcactatcagcagtgtgaagaccatgccattaagcttagcatgttgaccaagaaagcttgtctgcatctgaatcccggcggaacctgtgtcagcataggttatggttacgctgacagggccagcgaaagcatcattggtgctatagcgcggcagttcaagttttcccgggtatgcaaaccgaaatcctcacttgaagagacggaagttctgtttgtattcattgggtacgatcgcaaggcccgtacgcacaatccttacaagctttcatcaaccttgaccaacatttatacaggttccagactccacgaagccggatgtgcaccctcatatcatgtggtgcgaggggatattgccacggccaccgaaggagtgattataaatgctgctaacagcaaaggacaacctggcggaggggtgtgcggagcgctgtataagaaattcccggaaagcttcgatttacagccgatcgaagtaggaaaagcgcgactggtcaaaggtgcagctaaacatatcattcatgccgtaggaccaaacttcaacaaagtttcggaggttgaaggtgacaaacagttggcagaggcttatgagtccatcgctaagattgtcaacgataacaattacaagtcagtagcgattccactgttgtccaccggcatcttttccgggaacaaagatcgactaacccaatcattgaaccatttgctgacagctttagacaccactgatgcagatgtagccatatactgcagggacaagaaatgggaaatgactctcaaggaagcagtggctaggagagaagcagtggaggagatatgcatatccgacgactcttcagtgacagaacctgatgcagagctggtgagggtgcatccgaagagttctttggctggaaggaagggctacagcacaagcgatggcaaaactttctcatatttggaagggaccaagtttcaccaggcggccaaggatatagcagaaattaatgccatgtggcccgttgcaacggaggccaatgagcaggtatgcatgtatatcctcggagaaagcatgagcagtattaggtcgaaatgccccgtcgaagagtcggaagcctccacaccacctagcacgctgccttgcttgtgcatccatgccatgactccagaaagagtacagcgcctaaaagcctcacgtccagaacaaattactgtgtgctcatcctttccattgccgaagtatagaatcactggtgtgcagaagatccaatgctcccagcctatattgttctcaccgaaagtgcctgcgtatattcatccaaggaagtatctcgtggaaacaccaccggtagacgagactccggagccatcggcagagaaccaatccacagaggggacacctgaacaaccaccacttataaccgaggatgagaccaggactagaacgcctgagccgatcatcatcgaagaggaagaagaggatagcataagtttgctgtcagatggcccgacccaccaggtgctgcaagtcgaggcagacattcacgggccgccctctgtatctagctcatcctggtccattcctcatgcatccgactttgatgtggacagtttatccatacttgacaccctggagggagctagcgtgaccagcggggcaacgtcagccgagactaactcttacttcgcaaagagtatggagtttctggcgcgaccggtgcctgcgcctcgaacagtattcaggaaccctccacatcccgctccgcgcacaagaacaccgtcacttgcacccagcagggcctgctcgagaaccagcctagtttccaccccgccaggcgtgaatagggtgatcactagagaggagctcgaggcgcttaccccgtcacgcactcctagcaggtcggtctcgagaaccagcctggtctccaacccgccaggcgtaaatagggtgattacaagagaggagtttgaggcgttcgtagcacaacaacaatgacggtttgatgcgggtgcatacatcttttcctccgacaccggtcaagggcatttacaacaaaaatcagtaaggcaaacggtgctatccgaagtggtgttggagaggaccgaattggagatttcgtatgccccgcgcctcgaccaagaaaaagaagaattactacgcaagaaattacagttaaatcccacacctgctaacagaagcagataccagtccaggaaggtggagaacatgaaagccataacagctagacgtattctgcaaggcctagggcattatttgaaggcagaaggaaaagtggagtgctaccgaaccctgcatcctgttcctttgtattcatctagtgtgaaccgtgccttttcaagccccaaggtcgcagtggaagcctgtaacgccatgttgaaagagaactttccgactgtggcttcttactgtattattccagagtacgatgcctatttggacatggttgacggagcttcatgctgcttagacactgccagtttttgccctgcaaagctgcgcagctttccaaagaaacactcctatttggaacccacaatacgatcggcagtgccttcagcgatccagaacacgctccagaacgtcctggcagctgccacaaaaagaaattgcaatgtcacgcaaatgagagaattgcccgtattggattcggcggcctttaatgtggaatgcttcaagaaatatgcgtgtaataatgaatattgggaaacgtttaaagaaaaccccatcaggcttactgaagaaaacgtggtaaattacattaccaaattaaaaggaccaaaagctgctgctctttttgcgaagacacataatttgaatatgttgcaggacataccaatggacaggtttgtaatggacttaaagagagacgtgaaagtgactccaggaacaaaacatactgaagaacggcccaaggtacaggtgatccaggctgccgatccgctagcaacagcgtatctgtgcggaatccaccgagagctggttaggagattaaatgcggtcctgcttccgaacattcatacactgtttgatatgtcggctgaagactttgacgctattatagccgagcacttccagcctggggattgtgttctggaaactgacatcgcgtcgtttgataaaagtgaggacgacgccatggctctgaccgcgttaatgattctggaagacttaggtgtggacgcagagctgttgacgctgattgaggcggctttcggcgaaatttcatcaatacatttgcccactaaaactaaatttaaattcggagccatgatgaaatctggaatgttcctcacactgtttgtgaacacagtcattaacattgtaatcgcaagcagagtgttgagagaacggctaaccggatcaccatgtgcagcattcattggagatgacaatatcgtgaaaggagtcaaatcggacaaattaatggcagacaggtgcgccacctggttgaatatggaagtcaagattatagatgctgtggtgggcgagaaagcgccttatttctgtggagggtttattttgtgtgactccgtgaccggcacagcgtgccgtgtggcagaccccctaaaaaggctgtttaagcttggcaaacctctggcagcagacgatgaacatgatgatgacaggagaagggcattgcatgaagagtcaacacgctggaaccgagtgggtattctttcagagctgtgcaaggcagtagaatcaaggtatgaaaccgtaggaacttccatcatagttatggccatgactactctagctagcagtgttaaatcattcagctacctgagaggggcccctataactctctacggctaacctgaatggactacgacatagtctagtccgccaagatgttcgtgttcctggtgctgctgcccctcgttagcagccagtgcgtgaatctgaccacccgcacccagctgccaccagcctacacaaacagcttcaccagaggagtgtattaccctgataaggtctttagatcctccgtcctgcattctacgcaggatctcttcttgccattcttcagcaacgtgacatggttccacgccatccacgtttctggcaccaacggcacaaagcgcttcgacaatcctgtgttgccgtttaacgacggcgtttacttcgccagcacagaaaagagcaacatcatccggggctggatcttcggcaccaccctggacagcaaaacccaaagcctgctcatcgtgaacaacgccaccaacgtggtgatcaaggtgtgcgagttccagttctgcaatgatccttttctgggcgtgtactatcacaagaacaacaagagctggatggaaagcgagttcagagtgtattctagcgccaacaactgcacctttgagtacgtgtcccagccctttcttatggacctggaaggcaagcagggcaacttcaagaatctgagagaattcgtgttcaagaacattgatggctacttcaagatctacagcaagcacacccctatcaacctggttcgggacctgccacaaggcttcagcgccctggaacctctggtggacctgcctatcggcatcaacatcacacggttccaaaccctgctggccctgcaccggagctacctgacccccggcgacagcagcagcggctggaccgccggcgctgccgcctattacgtgggctacctgcaacctagaaccttcctgctgaaatacaacgagaacggcacaatcaccgacgccgtggactgtgccctggaccccctgtctgagacaaagtgtaccctgaagtctttcaccgtggagaagggcatctaccagaccagcaacttccgggtgcagcctacagaatctatagtgcggttccctaacatcaccaacctgtgtccttttggcgaggtgttcaacgccactcggttcgcctctgtctacgcctggaaccggaaacggatctctaattgcgtggccgattacagcgtcctgtataactccgccagtttcagcacattcaagtgctacggcgtgtcacccaccaagctgaacgatctgtgcttcaccaatgtgtacgccgatagtttcgtgatccggggcgatgaggtgcggcagatcgcccctggacagacaggcaagatcgccgactacaactacaagctgcctgacgacttcacaggctgtgtgatcgcatggaacagcaacaacctggacagcaaggtgggcggaaactacaactacctgtacagactgttcagaaagtccaacctgaagcctttcgagagagatatatctaccgagatctaccaggccggcagcacaccctgtaatggagtggaaggctttaactgctacttccctctgcaaagctatggatttcaacctacaaatggggttggctaccagccttacagagtggtggtccttagcttcgagctgctccatgcccctgccaccgtgtgcggacctaagaagtccaccaacctggtgaaaaacaagtgcgtgaactttaattttaacggcctgaccggaacaggagtgctgacagaaagcaacaaaaagttcctgcctttccagcagttcggcagagacattgccgacaccacagatgctgttagagacccccagacgctggaaatcctggatatcaccccctgctcttttggcggcgtgagcgtgatcaccccaggcacaaacacaagcaaccaggtggctgtgctgtaccaggacgtgaactgtacagaggtccctgtggcaatccacgccgatcagctgacccctacatggcgggtgtactccactggatctaacgtgttccagacaagggccggatgcctcatcggcgctgagcacgtgaacaattcttacgagtgcgacatccctattggagcgggcatctgcgccagctaccagacacagaccaatagccctcgcagagccagaagcgtggcctcccagagcatcatcgcctacaccatgagcctgggagccgagaactctgtggcctacagcaacaacagcatcgctatccctaccaacttcaccatctctgtcaccaccgaaatcctgcccgtcagtatgaccaaaaccagcgtcgactgcaccatgtacatatgcggcgatagcaccgaatgcagcaacctgctgctgcagtatggctccttctgcacccaacttaacagagccctgactggcatcgccgtggagcaggacaagaatacccaggaggtgttcgcccaggtgaagcagatctacaagacacccccgatcaaggacttcggcggctttaatttctctcagatcctgccagacccatctaaaccctctaagcggagctttatcgaggacctgctgttcaacaaggtgactctggctgacgccggcttcatcaagcagtacggcgattgcctgggcgacattgctgctagagacctgatctgtgcccagaaattcaacggtcttactgtgctgcctcctctgctgacggatgagatgatcgcccagtacaccagcgccctgctggccggcaccatcacatccggctggacattcggcgccggcgcagccctgcagatcccttttgccatgcagatggcctaccggttcaacggaatcggagtgacacagaacgtgctctacgaaaatcagaagttgatcgccaaccagttcaacagcgccatcggcaagattcaggatagtctgagttccaccgccagcgccctgggaaagctgcaggacgtggtcaatcagaatgcccaagccctgaacaccctggtgaagcagctgagcagcaacttcggcgccatcagctctgtgctgaacgacatcctgagtagactggacaaggtggaagccgaagtgcagatcgacagattgatcaccggaagactgcaaagcctgcagacctacgtgacccagcagctgataagagctgctgaaatcagagccagcgctaatctggccgctaccaagatgagcgagtgcgttctgggccagtctaagagagtggacttctgcggaaaaggctaccacctgatgtcctttcctcagtctgccccccacggcgtggtgttcctgcacgtcacatacgtgcccgctcaagagaaaaacttcaccacggcccctgccatctgtcacgacggcaaggcccacttccccagagagggcgtgttcgtgagcaatggcacccactggtttgtgactcagagaaacttctacgagccacagattatcaccacagataacaccttcgtgtctggcaactgcgacgtggtgatcggcatcgtcaacaacacagtgtacgacccactgcaacctgagctggactcattcaaggaggaactggataagtacttcaagaatcacaccagccccgacgttgacctgggcgacatcagcggcattaacgcctctgtggtcaacatccagaaggaaatcgacagactgaatgaggtggccaagaatttgaacgagagcctgattgatctgcaggagctgggcaaatacgagcagtacatcaagtggccttggtacatctggctgggcttcatcgccgggctgatcgccatcgttatggtgacaatcatgctgtgttgcatgacaagctgttgtagctgcctgaaaggctgctgctcctgcggcagctgttgcaagtttgacgaagatgacagcgagcccgtgctgaaaggcgtcaagctgcactacacctgaggcgcgcccacccagcggccgcccgctacgccccaatgatccgaccagcaaaactcgatgtacttccgaggaactgatgtgcataatgcatcaggctggtacattagatccccgcttaccgcgggcaatatagcaacactaaaaactcgatgtacttccgaggaagcgcagtgcataatgctgcgcagtgttgccacataaccactatattaaccatttatctagcggacgccaaaaactcaatgtatttctgaggaagcgtggtgcataatgccacgcagcgtctgcataacttttattatttcttttattaatcaacaaaattttgtttttaacatttcaaaaaaaaaaaaaaaaaaaaaaaaaaaaaaaaaaaaagaagagcgtttaaacacgtgatatctggcctcatgggccttcctttcactgcccgctttccagtcgggaaacctgtcgtgccagctgcattaacatggtcatagctgtttccttgcgtattgggcgctctccgcttcctcgctcactgactcgctgcgctcggtcgttcgggtaaagcctggggtgcctaatgagcaaaaggccagcaaaaggccaggaaccgtaaaaaggccgcgttgctggcgtttttccataggctccgcccccctgacgagcatcacaaaaatcgacgctcaagtcagaggtggcgaaacccgacaggactataaagataccaggcgtttccccctggaagctccctcgtgcgctctcctgttccgaccctgccgcttaccggatacctgtccgcctttctcccttcgggaagcgtggcgctttctcatagctcacgctgtaggtatctcagttcggtgtaggtcgttcgctccaagctgggctgtgtgcacgaaccccccgttcagcccgaccgctgcgccttatccggtaactatcgtcttgagtccaacccggtaagacacgacttatcgccactggcagcagccactggtaacaggattagcagagcgaggtatgtaggcggtgctacagagttcttgaagtggtggcctaactacggctacactagaagaacagtatttggtatctgcgctctgctgaagccagttaccttcggaaaaagagttggtagctcttgatccggcaaacaaaccaccgctggtagcggtggtttttttgtttgcaggcagcagattacgcgcagaaaaaaaggatctcaagaagatcctttgatcttttctacggggtctgacgctcagtggaacgaaaactcacgttaagggattttggtcatgaatacacggtgcctgactgcgttagcaatttaactgtgataaactaccgcattaaagcttatcgatgataagctgtcaaacatgagaattcttagaaaaactcatcgagcatcaaatgaaactgcaatttattcatatcaggattatcaataccatatttttgaaaaagccgtttctgtaatgaaggagaaaactcaccgaggcagttccataggatggcaagatcctggtatcggtctgcgattccgactcgtccaacatcaatacaacctattaatttcccctcgtcaaaaataaggttatcaagtgagaaatcaccatgagtgacgactgaatccggtgagaatggcaaaagcttatgcatttctttccagacttgttcaacaggccagccattacgctcgtcatcaaaatcactcgcatcaaccaaaccgttattcattcgtgattgcgcctgagcgagacgaaatacgcgatcgctgttaaaaggacaattacaaacaggaatcgaatgcaaccggcgcaggaacactgccagcgcatcaacaatattttcacctgaatcaggatattcttctaatacctggaatgctgttttcccggggatcgcagtggtgagtaaccatgcatcatcaggagtacggataaaatgcttgatggtcggaagaggcataaattccgtcagccagtttagtctgaccatctcatctgtaacatcattggcaacgctacctttgccatgtttcagaaacaactctggcgcatcgggcttcccatacaatcgatagattgtcgcacctgattgcccgacattatcgcgagcccatttatacccatataaatcagcatccatgttggaatttaatcgcggcctcgagcaagacgtttcccgttgaatatggctcataacaccccttgtattactgtttatgtaagcagacagttttattgttcatgagcggatacatatttgaatgtatttagaaaaataaacaaataggggttccgcgcacatttccccgaaaagtgccacctaaattgtaagcgttaatattttgttaaaattcgcgttaaatttttgttaaatcagctcattttttaaccaataggccgaaatcggcaaaatcccttataaatcaaaagaatagaccgagatagggttgagtggccgctacagggcgctcccattcgccattcaggctgcgcaactgttgggaagggcgtttcggtgcgggcctcttcgctattacgccagctggcgaaagggggatgtgctgcaaggcgattaagttgggtaacgccagggttttcccagtcacacgcgtaatacgactcactatag

SEQ ID NO: 11 - DNA, 11452 bp, synthetic construct
  misc_feature 1..11452: note = Nucleotide sequence of construct Co6
  source 1..11452: mol_type = other DNA
ataggcggcgcatgagagaagcccagaccaattacctacccaaaatggagaaagttcacgttgacatcgaggaagacagcccattcctcagagctttgcagcggagcttcccgcagtttgaggtagaagccaagcaggtcactgataatgaccatgctaatgccagagcgttttcgcatctggcttcaaaactgatcgaaacggaggtggacccatccgacacgatccttgacattggaagtgcgcccgcccgcagaatgtattctaagcacaagtatcattgtatctgtccgatgagatgtgcggaagatccggacagattgtataagtatgcaactaagctgaagaaaaactgtaaggaaataactgataaggaattggacaagaaaatgaaggagctcgccgccgtcatgagcgaccctgacctggaaactgagactatgtgcctccacgacgacgagtcgtgtcgctacgaagggcaagtcgctgtttaccaggatgtatacgcggttgacggaccgacaagtctctatcaccaagccaataagggagttagagtcgcctactggataggctttgacaccaccccttttatgtttaagaacttggctggagcatatccatcatactctaccaactgggccgacgaaaccgtgttaacggctcgtaacataggcctatgcagctctgacgttatggagcggtcacgtagagggatgtccattcttagaaagaagtatttgaaaccatccaacaatgttctattctctgttggctcgaccatctaccacgagaagagggacttactgaggagctggcacctgccgtctgtatttcacttacgtggcaagcaaaattacacatgtcggtgtgagactatagttagttgcgacgggtacgtcgttaaaagaatagctatcagtccaggcctgtatgggaagccttcaggctatgctgctacgatgcaccgcgagggattcttgtgctgcaaagtgacagacacattgaacggggagagggtctcttttcccgtgtgcacgtatgtgccagctacattgtgtgaccaaatgactggcatactggcaacagatgtcagtgcggacgacgcgcaaaaactgctggttgggctcaaccagcgtatagtcgtcaacggtcgcacccagagaaacaccaataccatgaaaaattaccttttgcccgtagtggcccaggcatttgctaggtgggcaaaggaatataaggaagatcaagaagatgaaaggccactaggactacgagatagacagttagtcatggggtgttgttgggcttttagaaggcacaagataacatctatttataagcgcccggatacccaaaccatcatcaaagtgaacagcgatttccactcattcgtgctgcccaggataggcagtaacacattggagatcgggctgagaacaagaatcaggaaaatgttagaggagcacaaggagccgtcacctctcattaccgccgaggacgtacaagaagctaagtgcgcagccgatgaggctaaggaggtgcgtgaagccgaggagttgcgcgcagctctaccacctttggcagctgatgttgaggagcccactctggaagccgatgtcgacttgatgttacaagaggctggggccggctcagtggagacacctcgtggcttgataaaggttaccagctacgatggcgaggacaagatcggctcttacgctgtgctttctccgcaggctgtactcaagagtgaaaaattatcttgcatccaccctctcgctgaacaagtcatagtgataacacactctggccgaaaagggcgttatgccgtggaaccataccatggtaaagtagtggtgccagagggacatgcaatacccgtccaggactttcaagctctgagtgaaagtgccaccattgtgtacaacgaacgtgagttcgtaaacaggtacctgcaccatattgccacacatggaggagcgctgaacactgatgaagaatattacaaaactgtcaagcccagcgagcacgacggcgaatacctgtacgacatcgacaggaaacagtgcgtcaagaaagaactagtcactgggctagggctcacaggcgagctggtggatcctcccttccatgaattcgcctacgagagtctgagaacacgaccagccgctccttaccaagtaccaaccataggggtgtatggcgtgccaggatcaggcaagtctggcatcattaaaagcgcagtcaccaaaaaagatctagtggtgagcgccaagaaagaaaactgtgcagaaattataagggacgtcaagaaaatgaaagggctggacgtcaatgccagaactgtggactcagtgctcttgaatggatgcaaacaccccgtagagaccctgtatattgacgaagcttttgcttgtcatgcaggtactctcagagcgctcatagccattataagacctaaaaaggcagtgctctgcggggatcccaaacagtgcggtttttttaacatgatgtgcctgaaagtgcattttaaccacgagatttgcacacaagtcttccacaaaagcatctctcgccgttgcactaaatctgtgacttcggtcgtctcaaccttgttttacgacaaaaaaatgagaacgacgaatccgaaagagactaagattgtgattgacactaccggcagtaccaaacctaagcaggacgatctcattctcacttgtttcagagggtgggtgaagcagttgcaaatagattacaaaggcaacgaaataatgacggcagctgcctctcaagggctgacccgtaaaggtgtgtatgccgttcggtacaaggtgaatgaaaatcctctgtacgcacccacctcagaacatgtgaacgtcctactgacccgcacggaggaccgcatcgtgtggaaaacactagccggcgacccatggataaaaacactgactgccaagtaccctgggaatttcactgccacgatagaggagtggcaagcagagcatgatgccatcatgaggcacatcttggagagaccggaccctaccgacgtcttccagaataaggcaaacgtgtgttgggccaaggctttagtgccggtgctgaagaccgctggcatagacatgaccactgaacaatggaacactgtggattattttgaaacggacaaagctcactcagcagagatagtattgaaccaactatgcgtgaggttctttggactcgatctggactccggtctattttctgcacccactgttccgttatccattaggaataatcactgggataactccccgtcgcctaacatgtacgggctgaataaagaagtggtccgtcagctctctcgcaggtacccacaactgcctcgggcagttgccactggaagagtctatgacatgaacactggtacactgcgcaattatgatccgcgcataaacctagtacctgtaaacagaagactgcctcatgctttagtcctccaccataatgaacacccacagagtgacttttcttcattcgtcagcaaattgaagggcagaactgtcctggtggtcggggaaaagttgtccgtcccaggcaaaatggttgactggttgtcagaccggcctgaggctaccttcagagctcggctggatttaggcatcccaggtgatgtgcccaaatatgacataatatttgttaatgtgaggaccccatataaataccatcactatcagcagtgtgaagaccatgccattaagcttagcatgttgaccaagaaagcttgtctgcatctgaatcccggcggaacctgtgtcagcataggttatggttacgctgacagggccagcgaaagcatcattggtgctatagcgcggcagttcaagttttcccgggtatgcaaaccgaaatcctcacttgaagagacggaagttctgtttgtattcattgggtacgatcgcaaggcccgtacgcacaatccttacaagctttcatcaaccttgaccaacatttatacaggttccagactccacgaagccggatgtgcaccctcatatcatgtggtgcgaggggatattgccacggccaccgaaggagtgattataaatgctgctaacagcaaaggacaacctggcggaggggtgtgcggagcgctgtataagaaattcccggaaagcttcgatttacagccgatcgaagtaggaaaagcgcgactggtcaaaggtgcagctaaacatatcattcatgccgtaggaccaaacttcaacaaagtttcggaggttgaaggtgacaaacagttggcagaggcttatgagtccatcgctaagattgtcaacgataacaattacaagtcagtagcgattccactgttgtccaccggcatcttttccgggaacaaagatcgactaacccaatcattgaaccatttgctgacagctttagacaccactgatgcagatgtagccatatactgcagggacaagaaatgggaaatgactctcaaggaagcagtggctaggagagaagcagtggaggagatatgcatatccgacgactcttcagtgacagaacctgatgcagagctggtgagggtgcatccgaagagttctttggctggaaggaagggctacagcacaagcgatggcaaaactttctcatatttggaagggaccaagtttcaccaggcggccaaggatatagcagaaattaatgccatgtggcccgttgcaacggaggccaatgagcaggtatgcatgtatatcctcggagaaagcatgagcagtattaggtcgaaatgccccgtcgaagagtcggaagcctccacaccacctagcacgctgccttgcttgtgcatccatgccatgactccagaaagagtacagcgcctaaaagcctcacgtccagaacaaattactgtgtgctcatcctttccattgccgaagtatagaatcactggtgtgcagaagatccaatgctcccagcctatattgttctcaccgaaagtgcctgcgtatattcatccaaggaagtatctcgtggaaacaccaccggtagacgagactccggagccatcggcagagaaccaatccacagaggggacacctgaacaaccaccacttataaccgaggatgagaccaggactagaacgcctgagccgatcatcatcgaagaggaagaagaggatagcataagtttgctgtcagatggcccgacccaccaggtgctgcaagtcgaggcagacattcacgggccgccctctgtatctagctcatcctggtccattcctcatgcatccgactttgatgtggacagtttatccatacttgacaccctggagggagctagcgtgaccagcggggcaacgtcagccgagactaactcttacttcgcaaagagtatggagtttctggcgcgaccggtgcctgcgcctcgaacagtattcaggaaccctccacatcccgctccgcgcacaagaacaccgtcacttgcacccagcagggcctgctcgagaaccagcctagtttccaccccgccaggcgtgaatagggtgatcactagagaggagctcgaggcgcttaccccgtcacgcactcctagcaggtcggtctcgagaaccagcctggtctccaacccgccaggcgtaaatagggtgattacaagagaggagtttgaggcgttcgtagcacaacaacaatgacggtttgatgcgggtgcatacatcttttcctccgacaccggtcaagggcatttacaacaaaaatcagtaaggcaaacggtgctatccgaagtggtgttggagaggaccgaattggagatttcgtatgccccgcgcctcgaccaagaaaaagaagaattactacgcaagaaattacagttaaatcccacacctgctaacagaagcagataccagtccaggaaggtggagaacatgaaagccataacagctagacgtattctgcaaggcctagggcattatttgaaggcagaaggaaaagtggagtgctaccgaaccctgcatcctgttcctttgtattcatctagtgtgaaccgtgccttttcaagccccaaggtcgcagtggaagcctgtaacgccatgttgaaagagaactttccgactgtggcttcttactgtattattccagagtacgatgcctatttggacatggttgacggagcttcatgctgcttagacactgccagtttttgccctgcaaagctgcgcagctttccaaagaaacactcctatttggaacccacaatacgatcggcagtgccttcagcgatccagaacacgctccagaacgtcctggcagctgccacaaaaagaaattgcaatgtcacgcaaatgagagaattgcccgtattggattcggcggcctttaatgtggaatgcttcaagaaatatgcgtgtaataatgaatattgggaaacgtttaaagaaaaccccatcaggcttactgaagaaaacgtggtaaattacattaccaaattaaaaggaccaaaagctgctgctctttttgcgaagacacataatttgaatatgttgcaggacataccaatggacaggtttgtaatggacttaaagagagacgtgaaagtgactccaggaacaaaacatactgaagaacggcccaaggtacaggtgatccaggctgccgatccgctagcaacagcgtatctgtgcggaatccaccgagagctggttaggagattaaatgcggtcctgcttccgaacattcatacactgtttgatatgtcggctgaagactttgacgctattatagccgagcacttccagcctggggattgtgttctggaaactgacatcgcgtcgtttgataaaagtgaggacgacgccatggctctgaccgcgttaatgattctggaagacttaggtgtggacgcagagctgttgacgctgattgaggcggctttcggcgaaatttcatcaatacatttgcccactaaaactaaatttaaattcggagccatgatgaaatctggaatgttcctcacactgtttgtgaacacagtcattaacattgtaatcgcaagcagagtgttgagagaacggctaaccggatcaccatgtgcagcattcattggagatgacaatatcgtgaaaggagtcaaatcggacaaattaatggcagacaggtgcgccacctggttgaatatggaagtcaagattatagatgctgtggtgggcgagaaagcgccttatttctgtggagggtttattttgtgtgactccgtgaccggcacagcgtgccgtgtggcagaccccctaaaaaggctgtttaagcttggcaaacctctggcagcagacgatgaacatgatgatgacaggagaagggcattgcatgaagagtcaacacgctggaaccgagtgggtattctttcagagctgtgcaaggcagtagaatcaaggtatgaaaccgtaggaacttccatcatagttatggccatgactactctagctagcagtgttaaatcattcagctacctgagaggggcccctataactctctacggctaacctgaatggactacgacatagtctagtccgccaagatgagcgacaacggacctcagaaccagagaaatgcccctagaatcacctttggcggacctagcgacagcaccggcagcaaccagaatggcgagagaagcggcgccagatctaagcagcggcgtccacagggactgcccaacaacaccgccagctggttcaccgccctcacccagcacggcaaagaggacctgaagttcccccggggacagggcgtgccaatcaacacaaactctagccccgacgaccagatcggctactatagacgggccaccagaaggatcagaggaggtgatggcaagatgaaggacctgagccctagatggtacttctactacctgggcacaggcccagaagccggcctgccttacggcgccaacaaggacggcatcatctgggtcgccaccgagggcgctctcaacacccctaaggaccacattggaactcggaaccccgctaataacgccgctatcgtgctgcagctgcctcagggcacgaccctgcccaagggcttctacgccgaaggcagcagaggcggcagccaggcctctagccggtccagctctcggagcagaaacagcagcagaaactccacccctggcagcagccgcggcaccagccccgccagaatggccggaaatggcggcgatgccgctctggccctgctgctgctggatagactgaaccagctggaatccaagatgtctggcaagggccagcagcaacagggccagaccgtgaccaagaaaagcgcagctgaagcctctaaaaaacctcggcagaagcggaccgccacaaaggcttacaacgtgacacaggcctttggcagaagaggacctgagcagacacagggcaacttcggcgaccaggagctgatccggcagggcacagactacaagcattggcctcagatcgcccagttcgcccctagtgccagcgccttcttcggcatgagccggatcggcatggaagtgacccctagcggcacatggctgacctacaccggcgccatcaagctggacgataaggaccccaattttaaggaccaagtgatcctgctgaacaagcacatcgacgcctataagaccttcccacctacagagcctaagaaagataagaaaaagaaggccgacgagacacaagccctgccccagagacagaaaaagcaacaaacagtgaccctgctgcctgccgctgatctggatgacttcagcaagcagctgcagcaatctatgagctccgccgatagcacccaggcctgaggcgcgcccacccagcggccgcccgctacgccccaatgatccgaccagcaaaactcgatgtacttccgaggaactgatgtgcataatgcatcaggctggtacattagatccccgcttaccgcgggcaatatagcaacactaaaaactcgatgtacttccgaggaagcgcagtgcataatgctgcgcagtgttgccacataaccactatattaaccatttatctagcggacgccaaaaactcaatgtatttctgaggaagcgtggtgcataatgccacgcagcgtctgcataacttttattatttcttttattaatcaacaaaattttgtttttaacatttcaaaaaaaaaaaaaaaaaaaaaaaaaaaaaaaaaaaaagaagagcgtttaaacacgtgatatctggcctcatgggccttcctttcactgcccgctttccagtcgggaaacctgtcgtgccagctgcattaacatggtcatagctgtttccttgcgtattgggcgctctccgcttcctcgctcactgactcgctgcgctcggtcgttcgggtaaagcctggggtgcctaatgagcaaaaggccagcaaaaggccaggaaccgtaaaaaggccgcgttgctggcgtttttccataggctccgcccccctgacgagcatcacaaaaatcgacgctcaagtcagaggtggcgaaacccgacaggactataaagataccaggcgtttccccctggaagctccctcgtgcgctctcctgttccgaccctgccgcttaccggatacctgtccgcctttctcccttcgggaagcgtggcgctttctcatagctcacgctgtaggtatctcagttcggtgtaggtcgttcgctccaagctgggctgtgtgcacgaaccccccgttcagcccgaccgctgcgccttatccggtaactatcgtcttgagtccaacccggtaagacacgacttatcgccactggcagcagccactggtaacaggattagcagagcgaggtatgtaggcggtgctacagagttcttgaagtggtggcctaactacggctacactagaagaacagtatttggtatctgcgctctgctgaagccagttaccttcggaaaaagagttggtagctcttgatccggcaaacaaaccaccgctggtagcggtggtttttttgtttgcaggcagcagattacgcgcagaaaaaaaggatctcaagaagatcctttgatcttttctacggggtctgacgctcagtggaacgaaaactcacgttaagggattttggtcatgaatacacggtgcctgactgcgttagcaatttaactgtgataaactaccgcattaaagcttatcgatgataagctgtcaaacatgagaattcttagaaaaactcatcgagcatcaaatgaaactgcaatttattcatatcaggattatcaataccatatttttgaaaaagccgtttctgtaatgaaggagaaaactcaccgaggcagttccataggatggcaagatcctggtatcggtctgcgattccgactcgtccaacatcaatacaacctattaatttcccctcgtcaaaaataaggttatcaagtgagaaatcaccatgagtgacgactgaatccggtgagaatggcaaaagcttatgcatttctttccagacttgttcaacaggccagccattacgctcgtcatcaaaatcactcgcatcaaccaaaccgttattcattcgtgattgcgcctgagcgagacgaaatacgcgatcgctgttaaaaggacaattacaaacaggaatcgaatgcaaccggcgcaggaacactgccagcgcatcaacaatattttcacctgaatcaggatattcttctaatacctggaatgctgttttcccggggatcgcagtggtgagtaaccatgcatcatcaggagtacggataaaatgcttgatggtcggaagaggcataaattccgtcagccagtttagtctgaccatctcatctgtaacatcattggcaacgctacctttgccatgtttcagaaacaactctggcgcatcgggcttcccatacaatcgatagattgtcgcacctgattgcccgacattatcgcgagcccatttatacccatataaatcagcatccatgttggaatttaatcgcggcctcgagcaagacgtttcccgttgaatatggctcataacaccccttgtattactgtttatgtaagcagacagttttattgttcatgagcggatacatatttgaatgtatttagaaaaataaacaaataggggttccgcgcacatttccccgaaaagtgccacctaaattgtaagcgttaatattttgttaaaattcgcgttaaatttttgttaaatcagctcattttttaaccaataggccgaaatcggcaaaatcccttataaatcaaaagaatagaccgagatagggttgagtggccgctacagggcgctcccattcgccattcaggctgcgcaactgttgggaagggcgtttcggtgcgggcctcttcgctattacgccagctggcgaaagggggatgtgctgcaaggcgattaagttgggtaacgccagggttttcccagtcacacgcgtaatacgactcactatag

SEQ ID NO: 12 - DNA, 14014 bp, synthetic construct
  misc_feature 1..14014: note = Nucleotide sequence of construct Co16
  source 1..14014: mol_type = other DNA
ataggcggcgcatgagagaagcccagaccaattacctacccaaaatggagaaagttcacgttgacatcgaggaagacagcccattcctcagagctttgcagcggagcttcccgcagtttgaggtagaagccaagcaggtcactgataatgaccatgctaatgccagagcgttttcgcatctggcttcaaaactgatcgaaacggaggtggacccatccgacacgatccttgacattggaagtgcgcccgcccgcagaatgtattctaagcacaagtatcattgtatctgtccgatgagatgtgcggaagatccggacagattgtataagtatgcaactaagctgaagaaaaactgtaaggaaataactgataaggaattggacaagaaaatgaaggagctcgccgccgtcatgagcgaccctgacctggaaactgagactatgtgcctccacgacgacgagtcgtgtcgctacgaagggcaagtcgctgtttaccaggatgtatacgcggttgacggaccgacaagtctctatcaccaagccaataagggagttagagtcgcctactggataggctttgacaccaccccttttatgtttaagaacttggctggagcatatccatcatactctaccaactgggccgacgaaaccgtgttaacggctcgtaacataggcctatgcagctctgacgttatggagcggtcacgtagagggatgtccattcttagaaagaagtatttgaaaccatccaacaatgttctattctctgttggctcgaccatctaccacgagaagagggacttactgaggagctggcacctgccgtctgtatttcacttacgtggcaagcaaaattacacatgtcggtgtgagactatagttagttgcgacgggtacgtcgttaaaagaatagctatcagtccaggcctgtatgggaagccttcaggctatgctgctacgatgcaccgcgagggattcttgtgctgcaaagtgacagacacattgaacggggagagggtctcttttcccgtgtgcacgtatgtgccagctacattgtgtgaccaaatgactggcatactggcaacagatgtcagtgcggacgacgcgcaaaaactgctggttgggctcaaccagcgtatagtcgtcaacggtcgcacccagagaaacaccaataccatgaaaaattaccttttgcccgtagtggcccaggcatttgctaggtgggcaaaggaatataaggaagatcaagaagatgaaaggccactaggactacgagatagacagttagtcatggggtgttgttgggcttttagaaggcacaagataacatctatttataagcgcccggatacccaaaccatcatcaaagtgaacagcgatttccactcattcgtgctgcccaggataggcagtaacacattggagatcgggctgagaacaagaatcaggaaaatgttagaggagcacaaggagccgtcacctctcattaccgccgaggacgtacaagaagctaagtgcgcagccgatgaggctaaggaggtgcgtgaagccgaggagttgcgcgcagctctaccacctttggcagctgatgttgaggagcccactctggaagccgatgtcgacttgatgttacaagaggctggggccggctcagtggagacacctcgtggcttgataaaggttaccagctacgatggcgaggacaagatcggctcttacgctgtgctttctccgcaggctgtactcaagagtgaaaaattatcttgcatccaccctctcgctgaacaagtcatagtgataacacactctggccgaaaagggcgttatgccgtggaaccataccatggtaaagtagtggtgccagagggacatgcaatacccgtccaggactttcaagctctgagtgaaagtgccaccattgtgtacaacgaacgtgagttcgtaaacaggtacctgcaccatattgccacacatggaggagcgctgaacactgatgaagaatattacaaaactgtcaagcccagcgagcacgacggcgaatacctgtacgacatcgacaggaaacagtgcgtcaagaaagaactagtcactgggctagggctcacaggcgagctggtggatcctcccttccatgaattcgcctacgagagtctgagaacacgaccagccgctccttaccaagtaccaaccataggggtgtatggcgtgccaggatcaggcaagtctggcatcattaaaagcgcagtcaccaaaaaagatctagtggtgagcgccaagaaagaaaactgtgcagaaattataagggacgtcaagaaaatgaaagggctggacgtcaatgccagaactgtggactcagtgctcttgaatggatgcaaacaccccgtagagaccctgtatattgacgaagcttttgcttgtcatgcaggtactctcagagcgctcatagccattataagacctaaaaaggcagtgctctgcggggatcccaaacagtgcggtttttttaacatgatgtgcctgaaagtgcattttaaccacgagatttgcacacaagtcttccacaaaagcatctctcgccgttgcactaaatctgtgacttcggtcgtctcaaccttgttttacgacaaaaaaatgagaacgacgaatccgaaagagactaagattgtgattgacactaccggcagtaccaaacctaagcaggacgatctcattctcacttgtttcagagggtgggtgaagcagttgcaaatagattacaaaggcaacgaaataatgacggcagctgcctctcaagggctgacccgtaaaggtgtgtatgccgttcggtacaaggtgaatgaaaatcctctgtacgcacccacctcagaacatgtgaacgtcctactgacccgcacggaggaccgcatcgtgtggaaaacactagccggcgacccatggataaaaacactgactgccaagtaccctgggaatttcactgccacgatagaggagtggcaagcagagcatgatgccatcatgaggcacatcttggagagaccggaccctaccgacgtcttccagaataaggcaaacgtgtgttgggccaaggctttagtgccggtgctgaagaccgctggcatagacatgaccactgaacaatggaacactgtggattattttgaaacggacaaagctcactcagcagagatagtattgaaccaactatgcgtgaggttctttggactcgatctggactccggtctattttctgcacccactgttccgttatccattaggaataatcactgggataactccccgtcgcctaacatgtacgggctgaataaagaagtggtccgtcagctctctcgcaggtacccacaactgcctcgggcagttgccactggaagagtctatgacatgaacactggtacactgcgcaattatgatccgcgcataaacctagtacctgtaaacagaagactgcctcatgctttagtcctccaccataatgaacacccacagagtgacttttcttcattcgtcagcaaattgaagggcagaactgtcctggtggtcggggaaaagttgtccgtcccaggcaaaatggttgactggttgtcagaccggcctgaggctaccttcagagctcggctggatttaggcatcccaggtgatgtgcccaaatatgacataatatttgttaatgtgaggaccccatataaataccatcactatcagcagtgtgaagaccatgccattaagcttagcatgttgaccaagaaagcttgtctgcatctgaatcccggcggaacctgtgtcagcataggttatggttacgctgacagggccagcgaaagcatcattggtgctatagcgcggcagttcaagttttcccgggtatgcaaaccgaaatcctcacttgaagagacggaagttctgtttgtattcattgggtacgatcgcaaggcccgtacgcacaatccttacaagctttcatcaaccttgaccaacatttatacaggttccagactccacgaagccggatgtgcaccctcatatcatgtggtgcgaggggatattgccacggccaccgaaggagtgattataaatgctgctaacagcaaaggacaacctggcggaggggtgtgcggagcgctgtataagaaattcccggaaagcttcgatttacagccgatcgaagtaggaaaagcgcgactggtcaaaggtgcagctaaacatatcattcatgccgtaggaccaaacttcaacaaagtttcggaggttgaaggtgacaaacagttggcagaggcttatgagtccatcgctaagattgtcaacgataacaattacaagtcagtagcgattccactgttgtccaccggcatcttttccgggaacaaagatcgactaacccaatcattgaaccatttgctgacagctttagacaccactgatgcagatgtagccatatactgcagggacaagaaatgggaaatgactctcaaggaagcagtggctaggagagaagcagtggaggagatatgcatatccgacgactcttcagtgacagaacctgatgcagagctggtgagggtgcatccgaagagttctttggctggaaggaagggctacagcacaagcgatggcaaaactttctcatatttggaagggaccaagtttcaccaggcggccaaggatatagcagaaattaatgccatgtggcccgttgcaacggaggccaatgagcaggtatgcatgtatatcctcggagaaagcatgagcagtattaggtcgaaatgccccgtcgaagagtcggaagcctccacaccacctagcacgctgccttgcttgtgcatccatgccatgactccagaaagagtacagcgcctaaaagcctcacgtccagaacaaattactgtgtgctcatcctttccattgccgaagtatagaatcactggtgtgcagaagatccaatgctcccagcctatattgttctcaccgaaagtgcctgcgtatattcatccaaggaagtatctcgtggaaacaccaccggtagacgagactccggagccatcggcagagaaccaatccacagaggggacacctgaacaaccaccacttataaccgaggatgagaccaggactagaacgcctgagccgatcatcatcgaagaggaagaagaggatagcataagtttgctgtcagatggcccgacccaccaggtgctgcaagtcgaggcagacattcacgggccgccctctgtatctagctcatcctggtccattcctcatgcatccgactttgatgtggacagtttatccatacttgacaccctggagggagctagcgtgaccagcggggcaacgtcagccgagactaactcttacttcgcaaagagtatggagtttctggcgcgaccggtgcctgcgcctcgaacagtattcaggaaccctccacatcccgctccgcgcacaagaacaccgtcacttgcacccagcagggcctgctcgagaaccagcctagtttccaccccgccaggcgtgaatagggtgatcactagagaggagctcgaggcgcttaccccgtcacgcactcctagcaggtcggtctcgagaaccagcctggtctccaacccgccaggcgtaaatagggtgattacaagagaggagtttgaggcgttcgtagcacaacaacaatgacggtttgatgcgggtgcatacatcttttcctccgacaccggtcaagggcatttacaacaaaaatcagtaaggcaaacggtgctatccgaagtggtgttggagaggaccgaattggagatttcgtatgccccgcgcctcgaccaagaaaaagaagaattactacgcaagaaattacagttaaatcccacacctgctaacagaagcagataccagtccaggaaggtggagaacatgaaagccataacagctagacgtattctgcaaggcctagggcattatttgaaggcagaaggaaaagtggagtgctaccgaaccctgcatcctgttcctttgtattcatctagtgtgaaccgtgccttttcaagccccaaggtcgcagtggaagcctgtaacgccatgttgaaagagaactttccgactgtggcttcttactgtattattccagagtacgatgcctatttggacatggttgacggagcttcatgctgcttagacactgccagtttttgccctgcaaagctgcgcagctttccaaagaaacactcctatttggaacccacaatacgatcggcagtgccttcagcgatccagaacacgctccagaacgtcctggcagctgccacaaaaagaaattgcaatgtcacgcaaatgagagaattgcccgtattggattcggcggcctttaatgtggaatgcttcaagaaatatgcgtgtaataatgaatattgggaaacgtttaaagaaaaccccatcaggcttactgaagaaaacgtggtaaattacattaccaaattaaaaggaccaaaagctgctgctctttttgcgaagacacataatttgaatatgttgcaggacataccaatggacaggtttgtaatggacttaaagagagacgtgaaagtgactccaggaacaaaacatactgaagaacggcccaaggtacaggtgatccaggctgccgatccgctagcaacagcgtatctgtgcggaatccaccgagagctggttaggagattaaatgcggtcctgcttccgaacattcatacactgtttgatatgtcggctgaagactttgacgctattatagccgagcacttccagcctggggattgtgttctggaaactgacatcgcgtcgtttgataaaagtgaggacgacgccatggctctgaccgcgttaatgattctggaagacttaggtgtggacgcagagctgttgacgctgattgaggcggctttcggcgaaatttcatcaatacatttgcccactaaaactaaatttaaattcggagccatgatgaaatctggaatgttcctcacactgtttgtgaacacagtcattaacattgtaatcgcaagcagagtgttgagagaacggctaaccggatcaccatgtgcagcattcattggagatgacaatatcgtgaaaggagtcaaatcggacaaattaatggcagacaggtgcgccacctggttgaatatggaagtcaagattatagatgctgtggtgggcgagaaagcgccttatttctgtggagggtttattttgtgtgactccgtgaccggcacagcgtgccgtgtggcagaccccctaaaaaggctgtttaagcttggcaaacctctggcagcagacgatgaacatgatgatgacaggagaagggcattgcatgaagagtcaacacgctggaaccgagtgggtattctttcagagctgtgcaaggcagtagaatcaaggtatgaaaccgtaggaacttccatcatagttatggccatgactactctagctagcagtgttaaatcattcagctacctgagaggggcccctataactctctacggctaacctgaatggactacgacatagtctagtccgccaagatgttcgtgttcctggtgctgctgcccctcgttagcagccagtgcgtgaatctgaccacccgcacccagctgccaccagcctacacaaacagcttcaccagaggagtgtattaccctgataaggtctttagatcctccgtcctgcattctacgcaggatctcttcttgccattcttcagcaacgtgacatggttccacgccatccacgtttctggcaccaacggcacaaagcgcttcgacaatcctgtgttgccgtttaacgacggcgtttacttcgccagcacagaaaagagcaacatcatccggggctggatcttcggcaccaccctggacagcaaaacccaaagcctgctcatcgtgaacaacgccaccaacgtggtgatcaaggtgtgcgagttccagttctgcaatgatccttttctgggcgtgtactatcacaagaacaacaagagctggatggaaagcgagttcagagtgtattctagcgccaacaactgcacctttgagtacgtgtcccagccctttcttatggacctggaaggcaagcagggcaacttcaagaatctgagagaattcgtgttcaagaacattgatggctacttcaagatctacagcaagcacacccctatcaacctggttcgggacctgccacaaggcttcagcgccctggaacctctggtggacctgcctatcggcatcaacatcacacggttccaaaccctgctggccctgcaccggagctacctgacccccggcgacagcagcagcggctggaccgccggcgctgccgcctattacgtgggctacctgcaacctagaaccttcctgctgaaatacaacgagaacggcacaatcaccgacgccgtggactgtgccctggaccccctgtctgagacaaagtgtaccctgaagtctttcaccgtggagaagggcatctaccagaccagcaacttccgggtgcagcctacagaatctatagtgcggttccctaacatcaccaacctgtgtccttttggcgaggtgttcaacgccactcggttcgcctctgtctacgcctggaaccggaaacggatctctaattgcgtggccgattacagcgtcctgtataactccgccagtttcagcacattcaagtgctacggcgtgtcacccaccaagctgaacgatctgtgcttcaccaatgtgtacgccgatagtttcgtgatccggggcgatgaggtgcggcagatcgcccctggacagacaggcaagatcgccgactacaactacaagctgcctgacgacttcacaggctgtgtgatcgcatggaacagcaacaacctggacagcaaggtgggcggaaactacaactacctgtacagactgttcagaaagtccaacctgaagcctttcgagagagatatatctaccgagatctaccaggccggcagcacaccctgtaatggagtggaaggctttaactgctacttccctctgcaaagctatggatttcaacctacaaatggggttggctaccagccttacagagtggtggtccttagcttcgagctgctccatgcccctgccaccgtgtgcggacctaagaagtccaccaacctggtgaaaaacaagtgcgtgaactttaattttaacggcctgaccggaacaggagtgctgacagaaagcaacaaaaagttcctgcctttccagcagttcggcagagacattgccgacaccacagatgctgttagagacccccagacgctggaaatcctggatatcaccccctgctcttttggcggcgtgagcgtgatcaccccaggcacaaacacaagcaaccaggtggctgtgctgtaccaggacgtgaactgtacagaggtccctgtggcaatccacgccgatcagctgacccctacatggcgggtgtactccactggatctaacgtgttccagacaagggccggatgcctcatcggcgctgagcacgtgaacaattcttacgagtgcgacatccctattggagcgggcatctgcgccagctaccagacacagaccaatagccctcagcaagccgctagcgtggcctcccagagcatcatcgcctacaccatgagcctgggagccgagaactctgtggcctacagcaacaacagcatcgctatccctaccaacttcaccatctctgtcaccaccgaaatcctgcccgtcagtatgaccaaaaccagcgtcgactgcaccatgtacatatgcggcgatagcaccgaatgcagcaacctgctgctgcagtatggctccttctgcacccaacttaacagagccctgactggcatcgccgtggagcaggacaagaatacccaggaggtgttcgcccaggtgaagcagatctacaagacacccccgatcaaggacttcggcggctttaatttctctcagatcctgccagacccatctaaaccctctaagcggagctttatcgaggacctgctgttcaacaaggtgactctggctgacgccggcttcatcaagcagtacggcgattgcctgggcgacattgctgctagagacctgatctgtgcccagaaattcaacggtcttactgtgctgcctcctctgctgacggatgagatgatcgcccagtacaccagcgccctgctggccggcaccatcacatccggctggacattcggcgccggcgcagccctgcagatcccttttgccatgcagatggcctaccggttcaacggaatcggagtgacacagaacgtgctctacgaaaatcagaagttgatcgccaaccagttcaacagcgccatcggcaagattcaggatagtctgagttccaccgccagcgccctgggaaagctgcaggacgtggtcaatcagaatgcccaagccctgaacaccctggtgaagcagctgagcagcaacttcggcgccatcagctctgtgctgaacgacatcctgagtagactggacaaggtggaagccgaagtgcagatcgacagattgatcaccggaagactgcaaagcctgcagacctacgtgacccagcagctgataagagctgctgaaatcagagccagcgctaatctggccgctaccaagatgagcgagtgcgttctgggccagtctaagagagtggacttctgcggaaaaggctaccacctgatgtcctttcctcagtctgccccccacggcgtggtgttcctgcacgtcacatacgtgcccgctcaagagaaaaacttcaccacggcccctgccatctgtcacgacggcaaggcccacttccccagagagggcgtgttcgtgagcaatggcacccactggtttgtgactcagagaaacttctacgagccacagattatcaccacagataacaccttcgtgtctggcaactgcgacgtggtgatcggcatcgtcaacaacacagtgtacgacccactgcaacctgagctggactcattcaaggaggaactggataagtacttcaagaatcacaccagccccgacgttgacctgggcgacatcagcggcattaacgcctctgtggtcaacatccagaaggaaatcgacagactgaatgaggtggccaagaatttgaacgagagcctgattgatctgcaggagctgggcaaatacgagcagtacatcaagtggccttggtacatctggctgggcttcatcgccgggctgatcgccatcgttatggtgacaatcatgctgtgttgcatgacaagctgttgtagctgcctgaaaggctgctgctcctgcggcagctgttgcaagtttgacgaagatgacagcgagcccgtgctgaaaggcgtcaagctgcactacacctgaggcgcgcccacccagcggccgcccgctacgccccaatgatccgaccagcaaaactcgatgtacttccgaggaactgatgtgcataatgcatcaggctggtacattagatccccgcttaccgcgggcaatatagcaacactaaaaactcgatgtacttccgaggaagcgcagtgcataatgctgcgcagtgttgccacataaccactatattaaccatttatctagcggacgccaaaaactcaatgtatttctgaggaagcgtggtgcataatgccacgcagcgtctgcataacttttattatttcttttattaatcaacaaaattttgtttttaacatttcaaaaaaaaaaaaaaaaaaaaaaaaaaaaaaaaaaaaagaagagcgtttaaacacgtgatatctggcctcatgggccttcctttcactgcccgctttccagtcgggaaacctgtcgtgccagctgcattaacatggtcatagctgtttccttgcgtattgggcgctctccgcttcctcgctcactgactcgctgcgctcggtcgttcgggtaaagcctggggtgcctaatgagcaaaaggccagcaaaaggccaggaaccgtaaaaaggccgcgttgctggcgtttttccataggctccgcccccctgacgagcatcacaaaaatcgacgctcaagtcagaggtggcgaaacccgacaggactataaagataccaggcgtttccccctggaagctccctcgtgcgctctcctgttccgaccctgccgcttaccggatacctgtccgcctttctcccttcgggaagcgtggcgctttctcatagctcacgctgtaggtatctcagttcggtgtaggtcgttcgctccaagctgggctgtgtgcacgaaccccccgttcagcccgaccgctgcgccttatccggtaactatcgtcttgagtccaacccggtaagacacgacttatcgccactggcagcagccactggtaacaggattagcagagcgaggtatgtaggcggtgctacagagttcttgaagtggtggcctaactacggctacactagaagaacagtatttggtatctgcgctctgctgaagccagttaccttcggaaaaagagttggtagctcttgatccggcaaacaaaccaccgctggtagcggtggtttttttgtttgcaggcagcagattacgcgcagaaaaaaaggatctcaagaagatcctttgatcttttctacggggtctgacgctcagtggaacgaaaactcacgttaagggattttggtcatgaatacacggtgcctgactgcgttagcaatttaactgtgataaactaccgcattaaagcttatcgatgataagctgtcaaacatgagaattcttagaaaaactcatcgagcatcaaatgaaactgcaatttattcatatcaggattatcaataccatatttttgaaaaagccgtttctgtaatgaaggagaaaactcaccgaggcagttccataggatggcaagatcctggtatcggtctgcgattccgactcgtccaacatcaatacaacctattaatttcccctcgtcaaaaataaggttatcaagtgagaaatcaccatgagtgacgactgaatccggtgagaatggcaaaagcttatgcatttctttccagacttgttcaacaggccagccattacgctcgtcatcaaaatcactcgcatcaaccaaaccgttattcattcgtgattgcgcctgagcgagacgaaatacgcgatcgctgttaaaaggacaattacaaacaggaatcgaatgcaaccggcgcaggaacactgccagcgcatcaacaatattttcacctgaatcaggatattcttctaatacctggaatgctgttttcccggggatcgcagtggtgagtaaccatgcatcatcaggagtacggataaaatgcttgatggtcggaagaggcataaattccgtcagccagtttagtctgaccatctcatctgtaacatcattggcaacgctacctttgccatgtttcagaaacaactctggcgcatcgggcttcccatacaatcgatagattgtcgcacctgattgcccgacattatcgcgagcccatttatacccatataaatcagcatccatgttggaatttaatcgcggcctcgagcaagacgtttcccgttgaatatggctcataacaccccttgtattactgtttatgtaagcagacagttttattgttcatgagcggatacatatttgaatgtatttagaaaaataaacaaataggggttccgcgcacatttccccgaaaagtgccacctaaattgtaagcgttaatattttgttaaaattcgcgttaaatttttgttaaatcagctcattttttaaccaataggccgaaatcggcaaaatcccttataaatcaaaagaatagaccgagatagggttgagtggccgctacagggcgctcccattcgccattcaggctgcgcaactgttgggaagggcgtttcggtgcgggcctcttcgctattacgccagctggcgaaagggggatgtgctgcaaggcgattaagttgggtaacgccagggttttcccagtcacacgcgtaatacgactcactatag

SEQ ID NO: 13 - DNA, 14014 bp, synthetic construct
  misc_feature 1..14014: note = Nucleotide sequence of construct Co17
  source 1..14014: mol_type = other DNA
ataggcggcgcatgagagaagcccagaccaattacctacccaaaatggagaaagttcacgttgacatcgaggaagacagcccattcctcagagctttgcagcggagcttcccgcagtttgaggtagaagccaagcaggtcactgataatgaccatgctaatgccagagcgttttcgcatctggcttcaaaactgatcgaaacggaggtggacccatccgacacgatccttgacattggaagtgcgcccgcccgcagaatgtattctaagcacaagtatcattgtatctgtccgatgagatgtgcggaagatccggacagattgtataagtatgcaactaagctgaagaaaaactgtaaggaaataactgataaggaattggacaagaaaatgaaggagctcgccgccgtcatgagcgaccctgacctggaaactgagactatgtgcctccacgacgacgagtcgtgtcgctacgaagggcaagtcgctgtttaccaggatgtatacgcggttgacggaccgacaagtctctatcaccaagccaataagggagttagagtcgcctactggataggctttgacaccaccccttttatgtttaagaacttggctggagcatatccatcatactctaccaactgggccgacgaaaccgtgttaacggctcgtaacataggcctatgcagctctgacgttatggagcggtcacgtagagggatgtccattcttagaaagaagtatttgaaaccatccaacaatgttctattctctgttggctcgaccatctaccacgagaagagggacttactgaggagctggcacctgccgtctgtatttcacttacgtggcaagcaaaattacacatgtcggtgtgagactatagttagttgcgacgggtacgtcgttaaaagaatagctatcagtccaggcctgtatgggaagccttcaggctatgctgctacgatgcaccgcgagggattcttgtgctgcaaagtgacagacacattgaacggggagagggtctcttttcccgtgtgcacgtatgtgccagctacattgtgtgaccaaatgactggcatactggcaacagatgtcagtgcggacgacgcgcaaaaactgctggttgggctcaaccagcgtatagtcgtcaacggtcgcacccagagaaacaccaataccatgaaaaattaccttttgcccgtagtggcccaggcatttgctaggtgggcaaaggaatataaggaagatcaagaagatgaaaggccactaggactacgagatagacagttagtcatggggtgttgttgggcttttagaaggcacaagataacatctatttataagcgcccggatacccaaaccatcatcaaagtgaacagcgatttccactcattcgtgctgcccaggataggcagtaacacattggagatcgggctgagaacaagaatcaggaaaatgttagaggagcacaaggagccgtcacctctcattaccgccgaggacgtacaagaagctaagtgcgcagccgatgaggctaaggaggtgcgtgaagccgaggagttgcgcgcagctctaccacctttggcagctgatgttgaggagcccactctggaagccgatgtcgacttgatgttacaagaggctggggccggctcagtggagacacctcgtggcttgataaaggttaccagctacgatggcgaggacaagatcggctcttacgctgtgctttctccgcaggctgtactcaagagtgaaaaattatcttgcatccaccctctcgctgaacaagtcatagtgataacacactctggccgaaaagggcgttatgccgtggaaccataccatggtaaagtagtggtgccagagggacatgcaatacccgtccaggactttcaagctctgagtgaaagtgccaccattgtgtacaacgaacgtgagttcgtaaacaggtacctgcaccatattgccacacatggaggagcgctgaacactgatgaagaatattacaaaactgtcaagcccagcgagcacgacggcgaatacctgtacgacatcgacaggaaacagtgcgtcaagaaagaactagtcactgggctagggctcacaggcgagctggtggatcctcccttccatgaattcgcctacgagagtctgagaacacgaccagccgctccttaccaagtaccaaccataggggtgtatggcgtgccaggatcaggcaagtctggcatcattaaaagcgcagtcaccaaaaaagatctagtggtgagcgccaagaaagaaaactgtgcagaaattataagggacgtcaagaaaatgaaagggctggacgtcaatgccagaactgtggactcagtgctcttgaatggatgcaaacaccccgtagagaccctgtatattgacgaagcttttgcttgtcatgcaggtactctcagagcgctcatagccattataagacctaaaaaggcagtgctctgcggggatcccaaacagtgcggtttttttaacatgatgtgcctgaaagtgcattttaaccacgagatttgcacacaagtcttccacaaaagcatctctcgccgttgcactaaatctgtgacttcggtcgtctcaaccttgttttacgacaaaaaaatgagaacgacgaatccgaaagagactaagattgtgattgacactaccggcagtaccaaacctaagcaggacgatctcattctcacttgtttcagagggtgggtgaagcagttgcaaatagattacaaaggcaacgaaataatgacggcagctgcctctcaagggctgacccgtaaaggtgtgtatgccgttcggtacaaggtgaatgaaaatcctctgtacgcacccacctcagaacatgtgaacgtcctactgacccgcacggaggaccgcatcgtgtggaaaacactagccggcgacccatggataaaaacactgactgccaagtaccctgggaatttcactgccacgatagaggagtggcaagcagagcatgatgccatcatgaggcacatcttggagagaccggaccctaccgacgtcttccagaataaggcaaacgtgtgttgggccaaggctttagtgccggtgctgaagaccgctggcatagacatgaccactgaacaatggaacactgtggattattttgaaacggacaaagctcactcagcagagatagtattgaaccaactatgcgtgaggttctttggactcgatctggactccggtctattttctgcacccactgttccgttatccattaggaataatcactgggataactccccgtcgcctaacatgtacgggctgaataaagaagtggtccgtcagctctctcgcaggtacccacaactgcctcgggcagttgccactggaagagtctatgacatgaacactggtacactgcgcaattatgatccgcgcataaacctagtacctgtaaacagaagactgcctcatgctttagtcctccaccataatgaacacccacagagtgacttttcttcattcgtcagcaaattgaagggcagaactgtcctggtggtcggggaaaagttgtccgtcccaggcaaaatggttgactggttgtcagaccggcctgaggctaccttcagagctcggctggatttaggcatcccaggtgatgtgcccaaatatgacataatatttgttaatgtgaggaccccatataaataccatcactatcagcagtgtgaagaccatgccattaagcttagcatgttgaccaagaaagcttgtctgcatctgaatcccggcggaacctgtgtcagcataggttatggttacgctgacagggccagcgaaagcatcattggtgctatagcgcggcagttcaagttttcccgggtatgcaaaccgaaatcctcacttgaagagacggaagttctgtttgtattcattgggtacgatcgcaaggcccgtacgcacaatccttacaagctttcatcaaccttgaccaacatttatacaggttccagactccacgaagccggatgtgcaccctcatatcatgtggtgcgaggggatattgccacggccaccgaaggagtgattataaatgctgctaacagcaaaggacaacctggcggaggggtgtgcggagcgctgtataagaaattcccggaaagcttcgatttacagccgatcgaagtaggaaaagcgcgactggtcaaaggtgcagctaaacatatcattcatgccgtaggaccaaacttcaacaaagtttcggaggttgaaggtgacaaacagttggcagaggcttatgagtccatcgctaagattgtcaacgataacaattacaagtcagtagcgattccactgttgtccaccggcatcttttccgggaacaaagatcgactaacccaatcattgaaccatttgctgacagctttagacaccactgatgcagatgtagccatatactgcagggacaagaaatgggaaatgactctcaaggaagcagtggctaggagagaagcagtggaggagatatgcatatccgacgactcttcagtgacagaacctgatgcagagctggtgagggtgcatccgaagagttctttggctggaaggaagggctacagcacaagcgatggcaaaactttctcatatttggaagggaccaagtttcaccaggcggccaaggatatagcagaaattaatgccatgtggcccgttgcaacggaggccaatgagcaggtatgcatgtatatcctcggagaaagcatgagcagtattaggtcgaaatgccccgtcgaagagtcggaagcctccacaccacctagcacgctgccttgcttgtgcatccatgccatgactccagaaagagtacagcgcctaaaagcctcacgtccagaacaaattactgtgtgctcatcctttccattgccgaagtatagaatcactggtgtgcagaagatccaatgctcccagcctatattgttctcaccgaaagtgcctgcgtatattcatccaaggaagtatctcgtggaaacaccaccggtagacgagactccggagccatcggcagagaaccaatccacagaggggacacctgaacaaccaccacttataaccgaggatgagaccaggactagaacgcctgagccgatcatcatcgaagaggaagaagaggatagcataagtttgctgtcagatggcccgacccaccaggtgctgcaagtcgaggcagacattcacgggccgccctctgtatctagctcatcctggtccattcctcatgcatccgactttgatgtggacagtttatccatacttgacaccctggagggagctagcgtgaccagcggggcaacgtcagccgagactaactcttacttcgcaaagagtatggagtttctggcgcgaccggtgcctgcgcctcgaacagtattcaggaaccctccacatcccgctccgcgcacaagaacaccgtcacttgcacccagcagggcctgctcgagaaccagcctagtttccaccccgccaggcgtgaatagggtgatcactagagaggagctcgaggcgcttaccccgtcacgcactcctagcaggtcggtctcgagaaccagcctggtctccaacccgccaggcgtaaatagggtgattacaagagaggagtttgaggcgttcgtagcacaacaacaatgacggtttgatgcgggtgcatacatcttttcctccgacaccggtcaagggcatttacaacaaaaatcagtaaggcaaacggtgctatccgaagtggtgttggagaggaccgaattggagatttcgtatgccccgcgcctcgaccaagaaaaagaagaattactacgcaagaaattacagttaaatcccacacctgctaacagaagcagataccagtccaggaaggtggagaacatgaaagccataacagctagacgtattctgcaaggcctagggcattatttgaaggcagaaggaaaagtggagtgctaccgaaccctgcatcctgttcctttgtattcatctagtgtgaaccgtgccttttcaagccccaaggtcgcagtggaagcctgtaacgccatgttgaaagagaactttccgactgtggcttcttactgtattattccagagtacgatgcctatttggacatggttgacggagcttcatgctgcttagacactgccagtttttgccctgcaaagctgcgcagctttccaaagaaacactcctatttggaacccacaatacgatcggcagtgccttcagcgatccagaacacgctccagaacgtcctggcagctgccacaaaaagaaattgcaatgtcacgcaaatgagagaattgcccgtattggattcggcggcctttaatgtggaatgcttcaagaaatatgcgtgtaataatgaatattgggaaacgtttaaagaaaaccccatcaggcttactgaagaaaacgtggtaaattacattaccaaattaaaaggaccaaaagctgctgctctttttgcgaagacacataatttgaatatgttgcaggacataccaatggacaggtttgtaatggacttaaagagagacgtgaaagtgactccaggaacaaaacatactgaagaacggcccaaggtacaggtgatccaggctgccgatccgctagcaacagcgtatctgtgcggaatccaccgagagctggttaggagattaaatgcggtcctgcttccgaacattcatacactgtttgatatgtcggctgaagactttgacgctattatagccgagcacttccagcctggggattgtgttctggaaactgacatcgcgtcgtttgataaaagtgaggacgacgccatggctctgaccgcgttaatgattctggaagacttaggtgtggacgcagagctgttgacgctgattgaggcggctttcggcgaaatttcatcaatacatttgcccactaaaactaaatttaaattcggagccatgatgaaatctggaatgttcctcacactgtttgtgaacacagtcattaacattgtaatcgcaagcagagtgttgagagaacggctaaccggatcaccatgtgcagcattcattggagatgacaatatcgtgaaaggagtcaaatcggacaaattaatggcagacaggtgcgccacctggttgaatatggaagtcaagattatagatgctgtggtgggcgagaaagcgccttatttctgtggagggtttattttgtgtgactccgtgaccggcacagcgtgccgtgtggcagaccccctaaaaaggctgtttaagcttggcaaacctctggcagcagacgatgaacatgatgatgacaggagaagggcattgcatgaagagtcaacacgctggaaccgagtgggtattctttcagagctgtgcaaggcagtagaatcaaggtatgaaaccgtaggaacttccatcatagttatggccatgactactctagctagcagtgttaaatcattcagctacctgagaggggcccctataactctctacggctaacctgaatggactacgacatagtctagtccgccaagatgttcgtgttcctggtgctgctgcccctcgttagcagccagtgcgtgaatctgaccacccgcacccagctgccaccagcctacacaaacagcttcaccagaggagtgtattaccctgataaggtctttagatcctccgtcctgcattctacgcaggatctcttcttgccattcttcagcaacgtgacatggttccacgccatccacgtttctggcaccaacggcacaaagcgcttcgacaatcctgtgttgccgtttaacgacggcgtttacttcgccagcacagaaaagagcaacatcatccggggctggatcttcggcaccaccctggacagcaaaacccaaagcctgctcatcgtgaacaacgccaccaacgtggtgatcaaggtgtgcgagttccagttctgcaatgatccttttctgggcgtgtactatcacaagaacaacaagagctggatggaaagcgagttcagagtgtattctagcgccaacaactgcacctttgagtacgtgtcccagccctttcttatggacctggaaggcaagcagggcaacttcaagaatctgagagaattcgtgttcaagaacattgatggctacttcaagatctacagcaagcacacccctatcaacctggttcgggacctgccacaaggcttcagcgccctggaacctctggtggacctgcctatcggcatcaacatcacacggttccaaaccctgctggccctgcaccggagctacctgacccccggcgacagcagcagcggctggaccgccggcgctgccgcctattacgtgggctacctgcaacctagaaccttcctgctgaaatacaacgagaacggcacaatcaccgacgccgtggactgtgccctggaccccctgtctgagacaaagtgtaccctgaagtctttcaccgtggagaagggcatctaccagaccagcaacttccgggtgcagcctacagaatctatagtgcggttccctaacatcaccaacctgtgtccttttggcgaggtgttcaacgccactcggttcgcctctgtctacgcctggaaccggaaacggatctctaattgcgtggccgattacagcgtcctgtataactccgccagtttcagcacattcaagtgctacggcgtgtcacccaccaagctgaacgatctgtgcttcaccaatgtgtacgccgatagtttcgtgatccggggcgatgaggtgcggcagatcgcccctggacagacaggcaagatcgccgactacaactacaagctgcctgacgacttcacaggctgtgtgatcgcatggaacagcaacaacctggacagcaaggtgggcggaaactacaactacctgtacagactgttcagaaagtccaacctgaagcctttcgagagagatatatctaccgagatctaccaggccggcagcacaccctgtaatggagtggaaggctttaactgctacttccctctgcaaagctatggatttcaacctacaaatggggttggctaccagccttacagagtggtggtccttagcttcgagctgctccatgcccctgccaccgtgtgcggacctaagaagtccaccaacctggtgaaaaacaagtgcgtgaactttaattttaacggcctgaccggaacaggagtgctgacagaaagcaacaaaaagttcctgcctttccagcagttcggcagagacattgccgacaccacagatgctgttagagacccccagacgctggaaatcctggatatcaccccctgctcttttggcggcgtgagcgtgatcaccccaggcacaaacacaagcaaccaggtggctgtgctgtaccaggacgtgaactgtacagaggtccctgtggcaatccacgccgatcagctgacccctacatggcgggtgtactccactggatctaacgtgttccagacaagggccggatgcctcatcggcgctgagcacgtgaacaattcttacgagtgcgacatccctattggagcgggcatctgcgccagctaccagacacagaccaatagccctcagcaagccgctagcgtggcctcccagagcatcatcgcctacaccatgagcctgggagccgagaactctgtggcctacagcaacaacagcatcgctatccctaccaacttcaccatctctgtcaccaccgaaatcctgcccgtcagtatgaccaaaaccagcgtcgactgcaccatgtacatatgcggcgatagcaccgaatgcagcaacctgctgctgcagtatggctccttctgcacccaacttaacagagccctgactggcatcgccgtggagcaggacaagaatacccaggaggtgttcgcccaggtgaagcagatctacaagacacccccgatcaaggacttcggcggctttaatttctctcagatcctgccagacccatctaaaccctctaagcggagctttatcgaggacctgctgttcaacaaggtgactctggctgacgccggcttcatcaagcagtacggcgattgcctgggcgacattgctgctagagacctgatctgtgcccagaaattcaacggtcttactgtgctgcctcctctgctgacggatgagatgatcgcccagtacaccagcgccctgctggccggcaccatcacatccggctggacattcggcgccggcgcagccctgcagatcccttttgccatgcagatggcctaccggttcaacggaatcggagtgacacagaacgtgctctacgaaaatcagaagttgatcgccaaccagttcaacagcgccatcggcaagattcaggatagtctgagttccaccgccagcgccctgggaaagctgcaggacgtggtcaatcagaatgcccaagccctgaacaccctggtgaagcagctgagcagcaacttcggcgccatcagctctgtgctgaacgacatcctgagtagactggacccacctgaagccgaagtgcagatcgacagattgatcaccggaagactgcaaagcctgcagacctacgtgacccagcagctgataagagctgctgaaatcagagccagcgctaatctggccgctaccaagatgagcgagtgcgttctgggccagtctaagagagtggacttctgcggaaaaggctaccacctgatgtcctttcctcagtctgccccccacggcgtggtgttcctgcacgtcacatacgtgcccgctcaagagaaaaacttcaccacggcccctgccatctgtcacgacggcaaggcccacttccccagagagggcgtgttcgtgagcaatggcacccactggtttgtgactcagagaaacttctacgagccacagattatcaccacagataacaccttcgtgtctggcaactgcgacgtggtgatcggcatcgtcaacaacacagtgtacgacccactgcaacctgagctggactcattcaaggaggaactggataagtacttcaagaatcacaccagccccgacgttgacctgggcgacatcagcggcattaacgcctctgtggtcaacatccagaaggaaatcgacagactgaatgaggtggccaagaatttgaacgagagcctgattgatctgcaggagctgggcaaatacgagcagtacatcaagtggccttggtacatctggctgggcttcatcgccgggctgatcgccatcgttatggtgacaatcatgctgtgttgcatgacaagctgttgtagctgcctgaaaggctgctgctcctgcggcagctgttgcaagtttgacgaagatgacagcgagcccgtgctgaaaggcgtcaagctgcactacacctgaggcgcgcccacccagcggccgcccgctacgccccaatgatccgaccagcaaaactcgatgtacttccgaggaactgatgtgcataatgcatcaggctggtacattagatccccgcttaccgcgggcaatatagcaacactaaaaactcgatgtacttccgaggaagcgcagtgcataatgctgcgcagtgttgccacataaccactatattaaccatttatctagcggacgccaaaaactcaatgtatttctgaggaagcgtggtgcataatgccacgcagcgtctgcataacttttattatttcttttattaatcaacaaaattttgtttttaacatttcaaaaaaaaaaaaaaaaaaaaaaaaaaaaaaaaaaaaagaagagcgtttaaacacgtgatatctggcctcatgggccttcctttcactgcccgctttccagtcgggaaacctgtcgtgccagctgcattaacatggtcatagctgtttccttgcgtattgggcgctctccgcttcctcgctcactgactcgctgcgctcggtcgttcgggtaaagcctggggtgcctaatgagcaaaaggccagcaaaaggccaggaaccgtaaaaaggccgcgttgctggcgtttttccataggctccgcccccctgacgagcatcacaaaaatcgacgctcaagtcagaggtggcgaaacccgacaggactataaagataccaggcgtttccccctggaagctccctcgtgcgctctcctgttccgaccctgccgcttaccggatacctgtccgcctttctcccttcgggaagcgtggcgctttctcatagctcacgctgtaggtatctcagttcggtgtaggtcgttcgctccaagctgggctgtgtgcacgaaccccccgttcagcccgaccgctgcgccttatccggtaactatcgtcttgagtccaacccggtaagacacgacttatcgccactggcagcagccactggtaacaggattagcagagcgaggtatgtaggcggtgctacagagttcttgaagtggtggcctaactacggctacactagaagaacagtatttggtatctgcgctctgctgaagccagttaccttcggaaaaagagttggtagctcttgatccggcaaacaaaccaccgctggtagcggtggtttttttgtttgcaggcagcagattacgcgcagaaaaaaaggatctcaagaagatcctttgatcttttctacggggtctgacgctcagtggaacgaaaactcacgttaagggattttggtcatgaatacacggtgcctgactgcgttagcaatttaactgtgataaactaccgcattaaagcttatcgatgataagctgtcaaacatgagaattcttagaaaaactcatcgagcatcaaatgaaactgcaatttattcatatcaggattatcaataccatatttttgaaaaagccgtttctgtaatgaaggagaaaactcaccgaggcagttccataggatggcaagatcctggtatcggtctgcgattccgactcgtccaacatcaatacaacctattaatttcccctcgtcaaaaataaggttatcaagtgagaaatcaccatgagtgacgactgaatccggtgagaatggcaaaagcttatgcatttctttccagacttgttcaacaggccagccattacgctcgtcatcaaaatcactcgcatcaaccaaaccgttattcattcgtgattgcgcctgagcgagacgaaatacgcgatcgctgttaaaaggacaattacaaacaggaatcgaatgcaaccggcgcaggaacactgccagcgcatcaacaatattttcacctgaatcaggatattcttctaatacctggaatgctgttttcccggggatcgcagtggtgagtaaccatgcatcatcaggagtacggataaaatgcttgatggtcggaagaggcataaattccgtcagccagtttagtctgaccatctcatctgtaacatcattggcaacgctacctttgccatgtttcagaaacaactctggcgcatcgggcttcccatacaatcgatagattgtcgcacctgattgcccgacattatcgcgagcccatttatacccatataaatcagcatccatgttggaatttaatcgcggcctcgagcaagacgtttcccgttgaatatggctcataacaccccttgtattactgtttatgtaagcagacagttttattgttcatgagcggatacatatttgaatgtatttagaaaaataaacaaataggggttccgcgcacatttccccgaaaagtgccacctaaattgtaagcgttaatattttgttaaaattcgcgttaaatttttgttaaatcagctcattttttaaccaataggccgaaatcggcaaaatcccttataaatcaaaagaatagaccgagatagggttgagtggccgctacagggcgctcccattcgccattcaggctgcgcaactgttgggaagggcgtttcggtgcgggcctcttcgctattacgccagctggcgaaagggggatgtgctgcaaggcgattaagttgggtaacgccagggttttcccagtcacacgcgtaatacgactcactatag

SEQ ID NO: 14 - DNA, 14014 bp, synthetic construct
  misc_feature 1..14014: note = Nucleotide sequence of construct Co48
  source 1..14014: mol_type = other DNA
ataggcggcgcatgagagaagcccagaccaattacctacccaaaatggagaaagttcacgttgacatcgaggaagacagcccattcctcagagctttgcagcggagcttcccgcagtttgaggtagaagccaagcaggtcactgataatgaccatgctaatgccagagcgttttcgcatctggcttcaaaactgatcgaaacggaggtggacccatccgacacgatccttgacattggaagtgcgcccgcccgcagaatgtattctaagcacaagtatcattgtatctgtccgatgagatgtgcggaagatccggacagattgtataagtatgcaactaagctgaagaaaaactgtaaggaaataactgataaggaattggacaagaaaatgaaggagctcgccgccgtcatgagcgaccctgacctggaaactgagactatgtgcctccacgacgacgagtcgtgtcgctacgaagggcaagtcgctgtttaccaggatgtatacgcggttgacggaccgacaagtctctatcaccaagccaataagggagttagagtcgcctactggataggctttgacaccaccccttttatgtttaagaacttggctggagcatatccatcatactctaccaactgggccgacgaaaccgtgttaacggctcgtaacataggcctatgcagctctgacgttatggagcggtcacgtagagggatgtccattcttagaaagaagtatttgaaaccatccaacaatgttctattctctgttggctcgaccatctaccacgagaagagggacttactgaggagctggcacctgccgtctgtatttcacttacgtggcaagcaaaattacacatgtcggtgtgagactatagttagttgcgacgggtacgtcgttaaaagaatagctatcagtccaggcctgtatgggaagccttcaggctatgctgctacgatgcaccgcgagggattcttgtgctgcaaagtgacagacacattgaacggggagagggtctcttttcccgtgtgcacgtatgtgccagctacattgtgtgaccaaatgactggcatactggcaacagatgtcagtgcggacgacgcgcaaaaactgctggttgggctcaaccagcgtatagtcgtcaacggtcgcacccagagaaacaccaataccatgaaaaattaccttttgcccgtagtggcccaggcatttgctaggtgggcaaaggaatataaggaagatcaagaagatgaaaggccactaggactacgagatagacagttagtcatggggtgttgttgggcttttagaaggcacaagataacatctatttataagcgcccggatacccaaaccatcatcaaagtgaacagcgatttccactcattcgtgctgcccaggataggcagtaacacattggagatcgggctgagaacaagaatcaggaaaatgttagaggagcacaaggagccgtcacctctcattaccgccgaggacgtacaagaagctaagtgcgcagccgatgaggctaaggaggtgcgtgaagccgaggagttgcgcgcagctctaccacctttggcagctgatgttgaggagcccactctggaagccgatgtcgacttgatgttacaagaggctggggccggctcagtggagacacctcgtggcttgataaaggttaccagctacgatggcgaggacaagatcggctcttacgctgtgctttctccgcaggctgtactcaagagtgaaaaattatcttgcatccaccctctcgctgaacaagtcatagtgataacacactctggccgaaaagggcgttatgccgtggaaccataccatggtaaagtagtggtgccagagggacatgcaatacccgtccaggactttcaagctctgagtgaaagtgccaccattgtgtacaacgaacgtgagttcgtaaacaggtacctgcaccatattgccacacatggaggagcgctgaacactgatgaagaatattacaaaactgtcaagcccagcgagcacgacggcgaatacctgtacgacatcgacaggaaacagtgcgtcaagaaagaactagtcactgggctagggctcacaggcgagctggtggatcctcccttccatgaattcgcctacgagagtctgagaacacgaccagccgctccttaccaagtaccaaccataggggtgtatggcgtgccaggatcaggcaagtctggcatcattaaaagcgcagtcaccaaaaaagatctagtggtgagcgccaagaaagaaaactgtgcagaaattataagggacgtcaagaaaatgaaagggctggacgtcaatgccagaactgtggactcagtgctcttgaatggatgcaaacaccccgtagagaccctgtatattgacgaagcttttgcttgtcatgcaggtactctcagagcgctcatagccattataagacctaaaaaggcagtgctctgcggggatcccaaacagtgcggtttttttaacatgatgtgcctgaaagtgcattttaaccacgagatttgcacacaagtcttccacaaaagcatctctcgccgttgcactaaatctgtgacttcggtcgtctcaaccttgttttacgacaaaaaaatgagaacgacgaatccgaaagagactaagattgtgattgacactaccggcagtaccaaacctaagcaggacgatctcattctcacttgtttcagagggtgggtgaagcagttgcaaatagattacaaaggcaacgaaataatgacggcagctgcctctcaagggctgacccgtaaaggtgtgtatgccgttcggtacaaggtgaatgaaaatcctctgtacgcacccacctcagaacatgtgaacgtcctactgacccgcacggaggaccgcatcgtgtggaaaacactagccggcgacccatggataaaaacactgactgccaagtaccctgggaatttcactgccacgatagaggagtggcaagcagagcatgatgccatcatgaggcacatcttggagagaccggaccctaccgacgtcttccagaataaggcaaacgtgtgttgggccaaggctttagtgccggtgctgaagaccgctggcatagacatgaccactgaacaatggaacactgtggattattttgaaacggacaaagctcactcagcagagatagtattgaaccaactatgcgtgaggttctttggactcgatctggactccggtctattttctgcacccactgttccgttatccattaggaataatcactgggataactccccgtcgcctaacatgtacgggctgaataaagaagtggtccgtcagctctctcgcaggtacccacaactgcctcgggcagttgccactggaagagtctatgacatgaacactggtacactgcgcaattatgatccgcgcataaacctagtacctgtaaacagaagactgcctcatgctttagtcctccaccataatgaacacccacagagtgacttttcttcattcgtcagcaaattgaagggcagaactgtcctggtggtcggggaaaagttgtccgtcccaggcaaaatggttgactggttgtcagaccggcctgaggctaccttcagagctcggctggatttaggcatcccaggtgatgtgcccaaatatgacataatatttgttaatgtgaggaccccatataaataccatcactatcagcagtgtgaagaccatgccattaagcttagcatgttgaccaagaaagcttgtctgcatctgaatcccggcggaacctgtgtcagcataggttatggttacgctgacagggccagcgaaagcatcattggtgctatagcgcggcagttcaagttttcccgggtatgcaaaccgaaatcctcacttgaagagacggaagttctgtttgtattcattgggtacgatcgcaaggcccgtacgcacaatccttacaagctttcatcaaccttgaccaacatttatacaggttccagactccacgaagccggatgtgcaccctcatatcatgtggtgcgaggggatattgccacggccaccgaaggagtgattataaatgctgctaacagcaaaggacaacctggcggaggggtgtgcggagcgctgtataagaaattcccggaaagcttcgatttacagccgatcgaagtaggaaaagcgcgactggtcaaaggtgcagctaaacatatcattcatgccgtaggaccaaacttcaacaaagtttcggaggttgaaggtgacaaacagttggcagaggcttatgagtccatcgctaagattgtcaacgataacaattacaagtcagtagcgattccactgttgtccaccggcatcttttccgggaacaaagatcgactaacccaatcattgaaccatttgctgacagctttagacaccactgatgcagatgtagccatatactgcagggacaagaaatgggaaatgactctcaaggaagcagtggctaggagagaagcagtggaggagatatgcatatccgacgactcttcagtgacagaacctgatgcagagctggtgagggtgcatccgaagagttctttggctggaaggaagggctacagcacaagcgatggcaaaactttctcatatttggaagggaccaagtttcaccaggcggccaaggatatagcagaaattaatgccatgtggcccgttgcaacggaggccaatgagcaggtatgcatgtatatcctcggagaaagcatgagcagtattaggtcgaaatgccccgtcgaagagtcggaagcctccacaccacctagcacgctgccttgcttgtgcatccatgccatgactccagaaagagtacagcgcctaaaagcctcacgtccagaacaaattactgtgtgctcatcctttccattgccgaagtatagaatcactggtgtgcagaagatccaatgctcccagcctatattgttctcaccgaaagtgcctgcgtatattcatccaaggaagtatctcgtggaaacaccaccggtagacgagactccggagccatcggcagagaaccaatccacagaggggacacctgaacaaccaccacttataaccgaggatgagaccaggactagaacgcctgagccgatcatcatcgaagaggaagaagaggatagcataagtttgctgtcagatggcccgacccaccaggtgctgcaagtcgaggcagacattcacgggccgccctctgtatctagctcatcctggtccattcctcatgcatccgactttgatgtggacagtttatccatacttgacaccctggagggagctagcgtgaccagcggggcaacgtcagccgagactaactcttacttcgcaaagagtatggagtttctggcgcgaccggtgcctgcgcctcgaacagtattcaggaaccctccacatcccgctccgcgcacaagaacaccgtcacttgcacccagcagggcctgctcgagaaccagcctagtttccaccccgccaggcgtgaatagggtgatcactagagaggagctcgaggcgcttaccccgtcacgcactcctagcaggtcggtctcgagaaccagcctggtctccaacccgccaggcgtaaatagggtgattacaagagaggagtttgaggcgttcgtagcacaacaacaatgacggtttgatgcgggtgcatacatcttttcctccgacaccggtcaagggcatttacaacaaaaatcagtaaggcaaacggtgctatccgaagtggtgttggagaggaccgaattggagatttcgtatgccccgcgcctcgaccaagaaaaagaagaattactacgcaagaaattacagttaaatcccacacctgctaacagaagcagataccagtccaggaaggtggagaacatgaaagccataacagctagacgtattctgcaaggcctagggcattatttgaaggcagaaggaaaagtggagtgctaccgaaccctgcatcctgttcctttgtattcatctagtgtgaaccgtgccttttcaagccccaaggtcgcagtggaagcctgtaacgccatgttgaaagagaactttccgactgtggcttcttactgtattattccagagtacgatgcctatttggacatggttgacggagcttcatgctgcttagacactgccagtttttgccctgcaaagctgcgcagctttccaaagaaacactcctatttggaacccacaatacgatcggcagtgccttcagcgatccagaacacgctccagaacgtcctggcagctgccacaaaaagaaattgcaatgtcacgcaaatgagagaattgcccgtattggattcggcggcctttaatgtggaatgcttcaagaaatatgcgtgtaataatgaatattgggaaacgtttaaagaaaaccccatcaggcttactgaagaaaacgtggtaaattacattaccaaattaaaaggaccaaaagctgctgctctttttgcgaagacacataatttgaatatgttgcaggacataccaatggacaggtttgtaatggacttaaagagagacgtgaaagtgactccaggaacaaaacatactgaagaacggcccaaggtacaggtgatccaggctgccgatccgctagcaacagcgtatctgtgcggaatccaccgagagctggttaggagattaaatgcggtcctgcttccgaacattcatacactgtttgatatgtcggctgaagactttgacgctattatagccgagcacttccagcctggggattgtgttctggaaactgacatcgcgtcgtttgataaaagtgaggacgacgccatggctctgaccgcgttaatgattctggaagacttaggtgtggacgcagagctgttgacgctgattgaggcggctttcggcgaaatttcatcaatacatttgcccactaaaactaaatttaaattcggagccatgatgaaatctggaatgttcctcacactgtttgtgaacacagtcattaacattgtaatcgcaagcagagtgttgagagaacggctaaccggatcaccatgtgcagcattcattggagatgacaatatcgtgaaaggagtcaaatcggacaaattaatggcagacaggtgcgccacctggttgaatatggaagtcaagattatagatgctgtggtgggcgagaaagcgccttatttctgtggagggtttattttgtgtgactccgtgaccggcacagcgtgccgtgtggcagaccccctaaaaaggctgtttaagcttggcaaacctctggcagcagacgatgaacatgatgatgacaggagaagggcattgcatgaagagtcaacacgctggaaccgagtgggtattctttcagagctgtgcaaggcagtagaatcaaggtatgaaaccgtaggaacttccatcatagttatggccatgactactctagctagcagtgttaaatcattcagctacctgagaggggcccctataactctctacggctaacctgaatggactacgacatagtctagtccgccaagatgttcgtgttcctggtgctgctgcccctcgttagcagccagtgcgtgaatctgaccacccgcacccagctgccaccagcctacacaaacagcttcaccagaggagtgtattaccctgataaggtctttagatcctccgtcctgcattctacgcaggatctcttcttgccattcttcagcaacgtgacatggttccacgccatccacgtttctggcaccaacggcacaaagcgcttcgacaatcctgtgttgccgtttaacgacggcgtttacttcgccagcacagaaaagagcaacatcatccggggctggatcttcggcaccaccctggacagcaaaacccaaagcctgctcatcgtgaacaacgccaccaacgtggtgatcaaggtgtgcgagttccagttctgcaatgatccttttctgggcgtgtactatcacaagaacaacaagagctggatggaaagcgagttcagagtgtattctagcgccaacaactgcacctttgagtacgtgtcccagccctttcttatggacctggaaggcaagcagggcaacttcaagaatctgagagaattcgtgttcaagaacattgatggctacttcaagatctacagcaagcacacccctatcaacctggttcgggacctgccacaaggcttcagcgccctggaacctctggtggacctgcctatcggcatcaacatcacacggttccaaaccctgctggccctgcaccggagctacctgacccccggcgacagcagcagcggctggaccgccggcgctgccgcctattacgtgggctacctgcaacctagaaccttcctgctgaaatacaacgagaacggcacaatcaccgacgccgtggactgtgccctggaccccctgtctgagacaaagtgtaccctgaagtctttcaccgtggagaagggcatctaccagaccagcaacttccgggtgcagcctacagaatctatagtgcggttccctaacatcaccaacctgtgtccttttggcgaggtgttcaacgccactcggttcgcctctgtctacgcctggaaccggaaacggatctctaattgcgtggccgattacagcgtcctgtataactccgccagtttcagcacattcaagtgctacggcgtgtcacccaccaagctgaacgatctgtgcttcaccaatgtgtacgccgatagtttcgtgatccggggcgatgaggtgcggcagatcgcccctggacagacaggcaagatcgccgactacaactacaagctgcctgacgacttcacaggctgtgtgatcgcatggaacagcaacaacctggacagcaaggtgggcggaaactacaactacctgtacagactgttcagaaagtccaacctgaagcctttcgagagagatatatctaccgagatctaccaggccggcagcacaccctgtaatggagtggaaggctttaactgctacttccctctgcaaagctatggatttcaacctacaaatggggttggctaccagccttacagagtggtggtccttagcttcgagctgctccatgcccctgccaccgtgtgcggacctaagaagtccaccaacctggtgaaaaacaagtgcgtgaactttaattttaacggcctgaccggaacaggagtgctgacagaaagcaacaaaaagttcctgcctttccagcagttcggcagagacattgccgacaccacagatgctgttagagacccccagacgctggaaatcctggatatcaccccctgctcttttggcggcgtgagcgtgatcaccccaggcacaaacacaagcaaccaggtggctgtgctgtaccagggcgtgaactgtacagaggtccctgtggcaatccacgccgatcagctgacccctacatggcgggtgtactccactggatctaacgtgttccagacaagggccggatgcctcatcggcgctgagcacgtgaacaattcttacgagtgcgacatccctattggagcgggcatctgcgccagctaccagacacagaccaatagccctcgcagagccagaagcgtggcctcccagagcatcatcgcctacaccatgagcctgggagccgagaactctgtggcctacagcaacaacagcatcgctatccctaccaacttcaccatctctgtcaccaccgaaatcctgcccgtcagtatgaccaaaaccagcgtcgactgcaccatgtacatatgcggcgatagcaccgaatgcagcaacctgctgctgcagtatggctccttctgcacccaacttaacagagccctgactggcatcgccgtggagcaggacaagaatacccaggaggtgttcgcccaggtgaagcagatctacaagacacccccgatcaaggacttcggcggctttaatttctctcagatcctgccagacccatctaaaccctctaagcggagctttatcgaggacctgctgttcaacaaggtgactctggctgacgccggcttcatcaagcagtacggcgattgcctgggcgacattgctgctagagacctgatctgtgcccagaaattcaacggtcttactgtgctgcctcctctgctgacggatgagatgatcgcccagtacaccagcgccctgctggccggcaccatcacatccggctggacattcggcgccggcgcagccctgcagatcccttttgccatgcagatggcctaccggttcaacggaatcggagtgacacagaacgtgctctacgaaaatcagaagttgatcgccaaccagttcaacagcgccatcggcaagattcaggatagtctgagttccaccgccagcgccctgggaaagctgcaggacgtggtcaatcagaatgcccaagccctgaacaccctggtgaagcagctgagcagcaacttcggcgccatcagctctgtgctgaacgacatcctgagtagactggacaaggtggaagccgaagtgcagatcgacagattgatcaccggaagactgcaaagcctgcagacctacgtgacccagcagctgataagagctgctgaaatcagagccagcgctaatctggccgctaccaagatgagcgagtgcgttctgggccagtctaagagagtggacttctgcggaaaaggctaccacctgatgtcctttcctcagtctgccccccacggcgtggtgttcctgcacgtcacatacgtgcccgctcaagagaaaaacttcaccacggcccctgccatctgtcacgacggcaaggcccacttccccagagagggcgtgttcgtgagcaatggcacccactggtttgtgactcagagaaacttctacgagccacagattatcaccacagataacaccttcgtgtctggcaactgcgacgtggtgatcggcatcgtcaacaacacagtgtacgacccactgcaacctgagctggactcattcaaggaggaactggataagtacttcaagaatcacaccagccccgacgttgacctgggcgacatcagcggcattaacgcctctgtggtcaacatccagaaggaaatcgacagactgaatgaggtggccaagaatttgaacgagagcctgattgatctgcaggagctgggcaaatacgagcagtacatcaagtggccttggtacatctggctgggcttcatcgccgggctgatcgccatcgttatggtgacaatcatgctgtgttgcatgacaagctgttgtagctgcctgaaaggctgctgctcctgcggcagctgttgcaagtttgacgaagatgacagcgagcccgtgctgaaaggcgtcaagctgcactacacctgaggcgcgcccacccagcggccgcccgctacgccccaatgatccgaccagcaaaactcgatgtacttccgaggaactgatgtgcataatgcatcaggctggtacattagatccccgcttaccgcgggcaatatagcaacactaaaaactcgatgtacttccgaggaagcgcagtgcataatgctgcgcagtgttgccacataaccactatattaaccatttatctagcggacgccaaaaactcaatgtatttctgaggaagcgtggtgcataatgccacgcagcgtctgcataacttttattatttcttttattaatcaacaaaattttgtttttaacatttcaaaaaaaaaaaaaaaaaaaaaaaaaaaaaaaaaaaaagaagagcgtttaaacacgtgatatctggcctcatgggccttcctttcactgcccgctttccagtcgggaaacctgtcgtgccagctgcattaacatggtcatagctgtttccttgcgtattgggcgctctccgcttcctcgctcactgactcgctgcgctcggtcgttcgggtaaagcctggggtgcctaatgagcaaaaggccagcaaaaggccaggaaccgtaaaaaggccgcgttgctggcgtttttccataggctccgcccccctgacgagcatcacaaaaatcgacgctcaagtcagaggtggcgaaacccgacaggactataaagataccaggcgtttccccctggaagctccctcgtgcgctctcctgttccgaccctgccgcttaccggatacctgtccgcctttctcccttcgggaagcgtggcgctttctcatagctcacgctgtaggtatctcagttcggtgtaggtcgttcgctccaagctgggctgtgtgcacgaaccccccgttcagcccgaccgctgcgccttatccggtaactatcgtcttgagtccaacccggtaagacacgacttatcgccactggcagcagccactggtaacaggattagcagagcgaggtatgtaggcggtgctacagagttcttgaagtggtggcctaactacggctacactagaagaacagtatttggtatctgcgctctgctgaagccagttaccttcggaaaaagagttggtagctcttgatccggcaaacaaaccaccgctggtagcggtggtttttttgtttgcaggcagcagattacgcgcagaaaaaaaggatctcaagaagatcctttgatcttttctacggggtctgacgctcagtggaacgaaaactcacgttaagggattttggtcatgaatacacggtgcctgactgcgttagcaatttaactgtgataaactaccgcattaaagcttatcgatgataagctgtcaaacatgagaattcttagaaaaactcatcgagcatcaaatgaaactgcaatttattcatatcaggattatcaataccatatttttgaaaaagccgtttctgtaatgaaggagaaaactcaccgaggcagttccataggatggcaagatcctggtatcggtctgcgattccgactcgtccaacatcaatacaacctattaatttcccctcgtcaaaaataaggttatcaagtgagaaatcaccatgagtgacgactgaatccggtgagaatggcaaaagcttatgcatttctttccagacttgttcaacaggccagccattacgctcgtcatcaaaatcactcgcatcaaccaaaccgttattcattcgtgattgcgcctgagcgagacgaaatacgcgatcgctgttaaaaggacaattacaaacaggaatcgaatgcaaccggcgcaggaacactgccagcgcatcaacaatattttcacctgaatcaggatattcttctaatacctggaatgctgttttcccggggatcgcagtggtgagtaaccatgcatcatcaggagtacggataaaatgcttgatggtcggaagaggcataaattccgtcagccagtttagtctgaccatctcatctgtaacatcattggcaacgctacctttgccatgtttcagaaacaactctggcgcatcgggcttcccatacaatcgatagattgtcgcacctgattgcccgacattatcgcgagcccatttatacccatataaatcagcatccatgttggaatttaatcgcggcctcgagcaagacgtttcccgttgaatatggctcataacaccccttgtattactgtttatgtaagcagacagttttattgttcatgagcggatacatatttgaatgtatttagaaaaataaacaaataggggttccgcgcacatttccccgaaaagtgccacctaaattgtaagcgttaatattttgttaaaattcgcgttaaatttttgttaaatcagctcattttttaaccaataggccgaaatcggcaaaatcccttataaatcaaaagaatagaccgagatagggttgagtggccgctacagggcgctcccattcgccattcaggctgcgcaactgttgggaagggcgtttcggtgcgggcctcttcgctattacgccagctggcgaaagggggatgtgctgcaaggcgattaagttgggtaacgccagggttttcccagtcacacgcgtaatacgactcactatag

SEQ ID NO: 15 - DNA, 14014 bp, synthetic construct
  misc_feature 1..14014: note = Nucleotide sequence of construct Co49
  source 1..14014: mol_type = other DNA
ataggcggcgcatgagagaagcccagaccaattacctacccaaaatggagaaagttcacgttgacatcgaggaagacagcccattcctcagagctttgcagcggagcttcccgcagtttgaggtagaagccaagcaggtcactgataatgaccatgctaatgccagagcgttttcgcatctggcttcaaaactgatcgaaacggaggtggacccatccgacacgatccttgacattggaagtgcgcccgcccgcagaatgtattctaagcacaagtatcattgtatctgtccgatgagatgtgcggaagatccggacagattgtataagtatgcaactaagctgaagaaaaactgtaaggaaataactgataaggaattggacaagaaaatgaaggagctcgccgccgtcatgagcgaccctgacctggaaactgagactatgtgcctccacgacgacgagtcgtgtcgctacgaagggcaagtcgctgtttaccaggatgtatacgcggttgacggaccgacaagtctctatcaccaagccaataagggagttagagtcgcctactggataggctttgacaccaccccttttatgtttaagaacttggctggagcatatccatcatactctaccaactgggccgacgaaaccgtgttaacggctcgtaacataggcctatgcagctctgacgttatggagcggtcacgtagagggatgtccattcttagaaagaagtatttgaaaccatccaacaatgttctattctctgttggctcgaccatctaccacgagaagagggacttactgaggagctggcacctgccgtctgtatttcacttacgtggcaagcaaaattacacatgtcggtgtgagactatagttagttgcgacgggtacgtcgttaaaagaatagctatcagtccaggcctgtatgggaagccttcaggctatgctgctacgatgcaccgcgagggattcttgtgctgcaaagtgacagacacattgaacggggagagggtctcttttcccgtgtgcacgtatgtgccagctacattgtgtgaccaaatgactggcatactggcaacagatgtcagtgcggacgacgcgcaaaaactgctggttgggctcaaccagcgtatagtcgtcaacggtcgcacccagagaaacaccaataccatgaaaaattaccttttgcccgtagtggcccaggcatttgctaggtgggcaaaggaatataaggaagatcaagaagatgaaaggccactaggactacgagatagacagttagtcatggggtgttgttgggcttttagaaggcacaagataacatctatttataagcgcccggatacccaaaccatcatcaaagtgaacagcgatttccactcattcgtgctgcccaggataggcagtaacacattggagatcgggctgagaacaagaatcaggaaaatgttagaggagcacaaggagccgtcacctctcattaccgccgaggacgtacaagaagctaagtgcgcagccgatgaggctaaggaggtgcgtgaagccgaggagttgcgcgcagctctaccacctttggcagctgatgttgaggagcccactctggaagccgatgtcgacttgatgttacaagaggctggggccggctcagtggagacacctcgtggcttgataaaggttaccagctacgatggcgaggacaagatcggctcttacgctgtgctttctccgcaggctgtactcaagagtgaaaaattatcttgcatccaccctctcgctgaacaagtcatagtgataacacactctggccgaaaagggcgttatgccgtggaaccataccatggtaaagtagtggtgccagagggacatgcaatacccgtccaggactttcaagctctgagtgaaagtgccaccattgtgtacaacgaacgtgagttcgtaaacaggtacctgcaccatattgccacacatggaggagcgctgaacactgatgaagaatattacaaaactgtcaagcccagcgagcacgacggcgaatacctgtacgacatcgacaggaaacagtgcgtcaagaaagaactagtcactgggctagggctcacaggcgagctggtggatcctcccttccatgaattcgcctacgagagtctgagaacacgaccagccgctccttaccaagtaccaaccataggggtgtatggcgtgccaggatcaggcaagtctggcatcattaaaagcgcagtcaccaaaaaagatctagtggtgagcgccaagaaagaaaactgtgcagaaattataagggacgtcaagaaaatgaaagggctggacgtcaatgccagaactgtggactcagtgctcttgaatggatgcaaacaccccgtagagaccctgtatattgacgaagcttttgcttgtcatgcaggtactctcagagcgctcatagccattataagacctaaaaaggcagtgctctgcggggatcccaaacagtgcggtttttttaacatgatgtgcctgaaagtgcattttaaccacgagatttgcacacaagtcttccacaaaagcatctctcgccgttgcactaaatctgtgacttcggtcgtctcaaccttgttttacgacaaaaaaatgagaacgacgaatccgaaagagactaagattgtgattgacactaccggcagtaccaaacctaagcaggacgatctcattctcacttgtttcagagggtgggtgaagcagttgcaaatagattacaaaggcaacgaaataatgacggcagctgcctctcaagggctgacccgtaaaggtgtgtatgccgttcggtacaaggtgaatgaaaatcctctgtacgcacccacctcagaacatgtgaacgtcctactgacccgcacggaggaccgcatcgtgtggaaaacactagccggcgacccatggataaaaacactgactgccaagtaccctgggaatttcactgccacgatagaggagtggcaagcagagcatgatgccatcatgaggcacatcttggagagaccggaccctaccgacgtcttccagaataaggcaaacgtgtgttgggccaaggctttagtgccggtgctgaagaccgctggcatagacatgaccactgaacaatggaacactgtggattattttgaaacggacaaagctcactcagcagagatagtattgaaccaactatgcgtgaggttctttggactcgatctggactccggtctattttctgcacccactgttccgttatccattaggaataatcactgggataactccccgtcgcctaacatgtacgggctgaataaagaagtggtccgtcagctctctcgcaggtacccacaactgcctcgggcagttgccactggaagagtctatgacatgaacactggtacactgcgcaattatgatccgcgcataaacctagtacctgtaaacagaagactgcctcatgctttagtcctccaccataatgaacacccacagagtgacttttcttcattcgtcagcaaattgaagggcagaactgtcctggtggtcggggaaaagttgtccgtcccaggcaaaatggttgactggttgtcagaccggcctgaggctaccttcagagctcggctggatttaggcatcccaggtgatgtgcccaaatatgacataatatttgttaatgtgaggaccccatataaataccatcactatcagcagtgtgaagaccatgccattaagcttagcatgttgaccaagaaagcttgtctgcatctgaatcccggcggaacctgtgtcagcataggttatggttacgctgacagggccagcgaaagcatcattggtgctatagcgcggcagttcaagttttcccgggtatgcaaaccgaaatcctcacttgaagagacggaagttctgtttgtattcattgggtacgatcgcaaggcccgtacgcacaatccttacaagctttcatcaaccttgaccaacatttatacaggttccagactccacgaagccggatgtgcaccctcatatcatgtggtgcgaggggatattgccacggccaccgaaggagtgattataaatgctgctaacagcaaaggacaacctggcggaggggtgtgcggagcgctgtataagaaattcccggaaagcttcgatttacagccgatcgaagtaggaaaagcgcgactggtcaaaggtgcagctaaacatatcattcatgccgtaggaccaaacttcaacaaagtttcggaggttgaaggtgacaaacagttggcagaggcttatgagtccatcgctaagattgtcaacgataacaattacaagtcagtagcgattccactgttgtccaccggcatcttttccgggaacaaagatcgactaacccaatcattgaaccatttgctgacagctttagacaccactgatgcagatgtagccatatactgcagggacaagaaatgggaaatgactctcaaggaagcagtggctaggagagaagcagtggaggagatatgcatatccgacgactcttcagtgacagaacctgatgcagagctggtgagggtgcatccgaagagttctttggctggaaggaagggctacagcacaagcgatggcaaaactttctcatatttggaagggaccaagtttcaccaggcggccaaggatatagcagaaattaatgccatgtggcccgttgcaacggaggccaatgagcaggtatgcatgtatatcctcggagaaagcatgagcagtattaggtcgaaatgccccgtcgaagagtcggaagcctccacaccacctagcacgctgccttgcttgtgcatccatgccatgactccagaaagagtacagcgcctaaaagcctcacgtccagaacaaattactgtgtgctcatcctttccattgccgaagtatagaatcactggtgtgcagaagatccaatgctcccagcctatattgttctcaccgaaagtgcctgcgtatattcatccaaggaagtatctcgtggaaacaccaccggtagacgagactccggagccatcggcagagaaccaatccacagaggggacacctgaacaaccaccacttataaccgaggatgagaccaggactagaacgcctgagccgatcatcatcgaagaggaagaagaggatagcataagtttgctgtcagatggcccgacccaccaggtgctgcaagtcgaggcagacattcacgggccgccctctgtatctagctcatcctggtccattcctcatgcatccgactttgatgtggacagtttatccatacttgacaccctggagggagctagcgtgaccagcggggcaacgtcagccgagactaactcttacttcgcaaagagtatggagtttctggcgcgaccggtgcctgcgcctcgaacagtattcaggaaccctccacatcccgctccgcgcacaagaacaccgtcacttgcacccagcagggcctgctcgagaaccagcctagtttccaccccgccaggcgtgaatagggtgatcactagagaggagctcgaggcgcttaccccgtcacgcactcctagcaggtcggtctcgagaaccagcctggtctccaacccgccaggcgtaaatagggtgattacaagagaggagtttgaggcgttcgtagcacaacaacaatgacggtttgatgcgggtgcatacatcttttcctccgacaccggtcaagggcatttacaacaaaaatcagtaaggcaaacggtgctatccgaagtggtgttggagaggaccgaattggagatttcgtatgccccgcgcctcgaccaagaaaaagaagaattactacgcaagaaattacagttaaatcccacacctgctaacagaagcagataccagtccaggaaggtggagaacatgaaagccataacagctagacgtattctgcaaggcctagggcattatttgaaggcagaaggaaaagtggagtgctaccgaaccctgcatcctgttcctttgtattcatctagtgtgaaccgtgccttttcaagccccaaggtcgcagtggaagcctgtaacgccatgttgaaagagaactttccgactgtggcttcttactgtattattccagagtacgatgcctatttggacatggttgacggagcttcatgctgcttagacactgccagtttttgccctgcaaagctgcgcagctttccaaagaaacactcctatttggaacccacaatacgatcggcagtgccttcagcgatccagaacacgctccagaacgtcctggcagctgccacaaaaagaaattgcaatgtcacgcaaatgagagaattgcccgtattggattcggcggcctttaatgtggaatgcttcaagaaatatgcgtgtaataatgaatattgggaaacgtttaaagaaaaccccatcaggcttactgaagaaaacgtggtaaattacattaccaaattaaaaggaccaaaagctgctgctctttttgcgaagacacataatttgaatatgttgcaggacataccaatggacaggtttgtaatggacttaaagagagacgtgaaagtgactccaggaacaaaacatactgaagaacggcccaaggtacaggtgatccaggctgccgatccgctagcaacagcgtatctgtgcggaatccaccgagagctggttaggagattaaatgcggtcctgcttccgaacattcatacactgtttgatatgtcggctgaagactttgacgctattatagccgagcacttccagcctggggattgtgttctggaaactgacatcgcgtcgtttgataaaagtgaggacgacgccatggctctgaccgcgttaatgattctggaagacttaggtgtggacgcagagctgttgacgctgattgaggcggctttcggcgaaatttcatcaatacatttgcccactaaaactaaatttaaattcggagccatgatgaaatctggaatgttcctcacactgtttgtgaacacagtcattaacattgtaatcgcaagcagagtgttgagagaacggctaaccggatcaccatgtgcagcattcattggagatgacaatatcgtgaaaggagtcaaatcggacaaattaatggcagacaggtgcgccacctggttgaatatggaagtcaagattatagatgctgtggtgggcgagaaagcgccttatttctgtggagggtttattttgtgtgactccgtgaccggcacagcgtgccgtgtggcagaccccctaaaaaggctgtttaagcttggcaaacctctggcagcagacgatgaacatgatgatgacaggagaagggcattgcatgaagagtcaacacgctggaaccgagtgggtattctttcagagctgtgcaaggcagtagaatcaaggtatgaaaccgtaggaacttccatcatagttatggccatgactactctagctagcagtgttaaatcattcagctacctgagaggggcccctataactctctacggctaacctgaatggactacgacatagtctagtccgccaagatgttcgtgttcctggtgctgctgcccctcgttagcagccagtgcgtgaatctgaccacccgcacccagctgccaccagcctacacaaacagcttcaccagaggagtgtattaccctgataaggtctttagatcctccgtcctgcattctacgcaggatctcttcttgccattcttcagcaacgtgacatggttccacgccatccacgtttctggcaccaacggcacaaagcgcttcgacaatcctgtgttgccgtttaacgacggcgtttacttcgccagcacagaaaagagcaacatcatccggggctggatcttcggcaccaccctggacagcaaaacccaaagcctgctcatcgtgaacaacgccaccaacgtggtgatcaaggtgtgcgagttccagttctgcaatgatccttttctgggcgtgtactatcacaagaacaacaagagctggatggaaagcgagttcagagtgtattctagcgccaacaactgcacctttgagtacgtgtcccagccctttcttatggacctggaaggcaagcagggcaacttcaagaatctgagagaattcgtgttcaagaacattgatggctacttcaagatctacagcaagcacacccctatcaacctggttcgggacctgccacaaggcttcagcgccctggaacctctggtggacctgcctatcggcatcaacatcacacggttccaaaccctgctggccctgcaccggagctacctgacccccggcgacagcagcagcggctggaccgccggcgctgccgcctattacgtgggctacctgcaacctagaaccttcctgctgaaatacaacgagaacggcacaatcaccgacgccgtggactgtgccctggaccccctgtctgagacaaagtgtaccctgaagtctttcaccgtggagaagggcatctaccagaccagcaacttccgggtgcagcctacagaatctatagtgcggttccctaacatcaccaacctgtgtccttttggcgaggtgttcaacgccactcggttcgcctctgtctacgcctggaaccggaaacggatctctaattgcgtggccgattacagcgtcctgtataactccgccagtttcagcacattcaagtgctacggcgtgtcacccaccaagctgaacgatctgtgcttcaccaatgtgtacgccgatagtttcgtgatccggggcgatgaggtgcggcagatcgcccctggacagacaggcaagatcgccgactacaactacaagctgcctgacgacttcacaggctgtgtgatcgcatggaacagcaacaacctggacagcaaggtgggcggaaactacaactacctgtacagactgttcagaaagtccaacctgaagcctttcgagagagatatatctaccgagatctaccaggccggcagcacaccctgtaatggagtggaaggctttaactgctacttccctctgcaaagctatggatttcaacctacaaatggggttggctaccagccttacagagtggtggtccttagcttcgagctgctccatgcccctgccaccgtgtgcggacctaagaagtccaccaacctggtgaaaaacaagtgcgtgaactttaattttaacggcctgaccggaacaggagtgctgacagaaagcaacaaaaagttcctgcctttccagcagttcggcagagacattgccgacaccacagatgctgttagagacccccagacgctggaaatcctggatatcaccccctgctcttttggcggcgtgagcgtgatcaccccaggcacaaacacaagcaaccaggtggctgtgctgtaccagggcgtgaactgtacagaggtccctgtggcaatccacgccgatcagctgacccctacatggcgggtgtactccactggatctaacgtgttccagacaagggccggatgcctcatcggcgctgagcacgtgaacaattcttacgagtgcgacatccctattggagcgggcatctgcgccagctaccagacacagaccaatagccctcagcaagccgctagcgtggcctcccagagcatcatcgcctacaccatgagcctgggagccgagaactctgtggcctacagcaacaacagcatcgctatccctaccaacttcaccatctctgtcaccaccgaaatcctgcccgtcagtatgaccaaaaccagcgtcgactgcaccatgtacatatgcggcgatagcaccgaatgcagcaacctgctgctgcagtatggctccttctgcacccaacttaacagagccctgactggcatcgccgtggagcaggacaagaatacccaggaggtgttcgcccaggtgaagcagatctacaagacacccccgatcaaggacttcggcggctttaatttctctcagatcctgccagacccatctaaaccctctaagcggagctttatcgaggacctgctgttcaacaaggtgactctggctgacgccggcttcatcaagcagtacggcgattgcctgggcgacattgctgctagagacctgatctgtgcccagaaattcaacggtcttactgtgctgcctcctctgctgacggatgagatgatcgcccagtacaccagcgccctgctggccggcaccatcacatccggctggacattcggcgccggcgcagccctgcagatcccttttgccatgcagatggcctaccggttcaacggaatcggagtgacacagaacgtgctctacgaaaatcagaagttgatcgccaaccagttcaacagcgccatcggcaagattcaggatagtctgagttccaccgccagcgccctgggaaagctgcaggacgtggtcaatcagaatgcccaagccctgaacaccctggtgaagcagctgagcagcaacttcggcgccatcagctctgtgctgaacgacatcctgagtagactggacaaggtggaagccgaagtgcagatcgacagattgatcaccggaagactgcaaagcctgcagacctacgtgacccagcagctgataagagctgctgaaatcagagccagcgctaatctggccgctaccaagatgagcgagtgcgttctgggccagtctaagagagtggacttctgcggaaaaggctaccacctgatgtcctttcctcagtctgccccccacggcgtggtgttcctgcacgtcacatacgtgcccgctcaagagaaaaacttcaccacggcccctgccatctgtcacgacggcaaggcccacttccccagagagggcgtgttcgtgagcaatggcacccactggtttgtgactcagagaaacttctacgagccacagattatcaccacagataacaccttcgtgtctggcaactgcgacgtggtgatcggcatcgtcaacaacacagtgtacgacccactgcaacctgagctggactcattcaaggaggaactggataagtacttcaagaatcacaccagccccgacgttgacctgggcgacatcagcggcattaacgcctctgtggtcaacatccagaaggaaatcgacagactgaatgaggtggccaagaatttgaacgagagcctgattgatctgcaggagctgggcaaatacgagcagtacatcaagtggccttggtacatctggctgggcttcatcgccgggctgatcgccatcgttatggtgacaatcatgctgtgttgcatgacaagctgttgtagctgcctgaaaggctgctgctcctgcggcagctgttgcaagtttgacgaagatgacagcgagcccgtgctgaaaggcgtcaagctgcactacacctgaggcgcgcccacccagcggccgcccgctacgccccaatgatccgaccagcaaaactcgatgtacttccgaggaactgatgtgcataatgcatcaggctggtacattagatccccgcttaccgcgggcaatatagcaacactaaaaactcgatgtacttccgaggaagcgcagtgcataatgctgcgcagtgttgccacataaccactatattaaccatttatctagcggacgccaaaaactcaatgtatttctgaggaagcgtggtgcataatgccacgcagcgtctgcataacttttattatttcttttattaatcaacaaaattttgtttttaacatttcaaaaaaaaaaaaaaaaaaaaaaaaaaaaaaaaaaaaagaagagcgtttaaacacgtgatatctggcctcatgggccttcctttcactgcccgctttccagtcgggaaacctgtcgtgccagctgcattaacatggtcatagctgtttccttgcgtattgggcgctctccgcttcctcgctcactgactcgctgcgctcggtcgttcgggtaaagcctggggtgcctaatgagcaaaaggccagcaaaaggccaggaaccgtaaaaaggccgcgttgctggcgtttttccataggctccgcccccctgacgagcatcacaaaaatcgacgctcaagtcagaggtggcgaaacccgacaggactataaagataccaggcgtttccccctggaagctccctcgtgcgctctcctgttccgaccctgccgcttaccggatacctgtccgcctttctcccttcgggaagcgtggcgctttctcatagctcacgctgtaggtatctcagttcggtgtaggtcgttcgctccaagctgggctgtgtgcacgaaccccccgttcagcccgaccgctgcgccttatccggtaactatcgtcttgagtccaacccggtaagacacgacttatcgccactggcagcagccactggtaacaggattagcagagcgaggtatgtaggcggtgctacagagttcttgaagtggtggcctaactacggctacactagaagaacagtatttggtatctgcgctctgctgaagccagttaccttcggaaaaagagttggtagctcttgatccggcaaacaaaccaccgctggtagcggtggtttttttgtttgcaggcagcagattacgcgcagaaaaaaaggatctcaagaagatcctttgatcttttctacggggtctgacgctcagtggaacgaaaactcacgttaagggattttggtcatgaatacacggtgcctgactgcgttagcaatttaactgtgataaactaccgcattaaagcttatcgatgataagctgtcaaacatgagaattcttagaaaaactcatcgagcatcaaatgaaactgcaatttattcatatcaggattatcaataccatatttttgaaaaagccgtttctgtaatgaaggagaaaactcaccgaggcagttccataggatggcaagatcctggtatcggtctgcgattccgactcgtccaacatcaatacaacctattaatttcccctcgtcaaaaataaggttatcaagtgagaaatcaccatgagtgacgactgaatccggtgagaatggcaaaagcttatgcatttctttccagacttgttcaacaggccagccattacgctcgtcatcaaaatcactcgcatcaaccaaaccgttattcattcgtgattgcgcctgagcgagacgaaatacgcgatcgctgttaaaaggacaattacaaacaggaatcgaatgcaaccggcgcaggaacactgccagcgcatcaacaatattttcacctgaatcaggatattcttctaatacctggaatgctgttttcccggggatcgcagtggtgagtaaccatgcatcatcaggagtacggataaaatgcttgatggtcggaagaggcataaattccgtcagccagtttagtctgaccatctcatctgtaacatcattggcaacgctacctttgccatgtttcagaaacaactctggcgcatcgggcttcccatacaatcgatagattgtcgcacctgattgcccgacattatcgcgagcccatttatacccatataaatcagcatccatgttggaatttaatcgcggcctcgagcaagacgtttcccgttgaatatggctcataacaccccttgtattactgtttatgtaagcagacagttttattgttcatgagcggatacatatttgaatgtatttagaaaaataaacaaataggggttccgcgcacatttccccgaaaagtgccacctaaattgtaagcgttaatattttgttaaaattcgcgttaaatttttgttaaatcagctcattttttaaccaataggccgaaatcggcaaaatcccttataaatcaaaagaatagaccgagatagggttgagtggccgctacagggcgctcccattcgccattcaggctgcgcaactgttgggaagggcgtttcggtgcgggcctcttcgctattacgccagctggcgaaagggggatgtgctgcaaggcgattaagttgggtaacgccagggttttcccagtcacacgcgtaatacgactcactatag

SEQ ID NO: 16 - DNA, 14014 bp, synthetic construct
  misc_feature 1..14014: note = Nucleotide sequence of construct Co58
  source 1..14014: mol_type = other DNA
ataggcggcgcatgagagaagcccagaccaattacctacccaaaatggagaaagttcacgttgacatcgaggaagacagcccattcctcagagctttgcagcggagcttcccgcagtttgaggtagaagccaagcaggtcactgataatgaccatgctaatgccagagcgttttcgcatctggcttcaaaactgatcgaaacggaggtggacccatccgacacgatccttgacattggaagtgcgcccgcccgcagaatgtattctaagcacaagtatcattgtatctgtccgatgagatgtgcggaagatccggacagattgtataagtatgcaactaagctgaagaaaaactgtaaggaaataactgataaggaattggacaagaaaatgaaggagctcgccgccgtcatgagcgaccctgacctggaaactgagactatgtgcctccacgacgacgagtcgtgtcgctacgaagggcaagtcgctgtttaccaggatgtatacgcggttgacggaccgacaagtctctatcaccaagccaataagggagttagagtcgcctactggataggctttgacaccaccccttttatgtttaagaacttggctggagcatatccatcatactctaccaactgggccgacgaaaccgtgttaacggctcgtaacataggcctatgcagctctgacgttatggagcggtcacgtagagggatgtccattcttagaaagaagtatttgaaaccatccaacaatgttctattctctgttggctcgaccatctaccacgagaagagggacttactgaggagctggcacctgccgtctgtatttcacttacgtggcaagcaaaattacacatgtcggtgtgagactatagttagttgcgacgggtacgtcgttaaaagaatagctatcagtccaggcctgtatgggaagccttcaggctatgctgctacgatgcaccgcgagggattcttgtgctgcaaagtgacagacacattgaacggggagagggtctcttttcccgtgtgcacgtatgtgccagctacattgtgtgaccaaatgactggcatactggcaacagatgtcagtgcggacgacgcgcaaaaactgctggttgggctcaaccagcgtatagtcgtcaacggtcgcacccagagaaacaccaataccatgaaaaattaccttttgcccgtagtggcccaggcatttgctaggtgggcaaaggaatataaggaagatcaagaagatgaaaggccactaggactacgagatagacagttagtcatggggtgttgttgggcttttagaaggcacaagataacatctatttataagcgcccggatacccaaaccatcatcaaagtgaacagcgatttccactcattcgtgctgcccaggataggcagtaacacattggagatcgggctgagaacaagaatcaggaaaatgttagaggagcacaaggagccgtcacctctcattaccgccgaggacgtacaagaagctaagtgcgcagccgatgaggctaaggaggtgcgtgaagccgaggagttgcgcgcagctctaccacctttggcagctgatgttgaggagcccactctggaagccgatgtcgacttgatgttacaagaggctggggccggctcagtggagacacctcgtggcttgataaaggttaccagctacgatggcgaggacaagatcggctcttacgctgtgctttctccgcaggctgtactcaagagtgaaaaattatcttgcatccaccctctcgctgaacaagtcatagtgataacacactctggccgaaaagggcgttatgccgtggaaccataccatggtaaagtagtggtgccagagggacatgcaatacccgtccaggactttcaagctctgagtgaaagtgccaccattgtgtacaacgaacgtgagttcgtaaacaggtacctgcaccatattgccacacatggaggagcgctgaacactgatgaagaatattacaaaactgtcaagcccagcgagcacgacggcgaatacctgtacgacatcgacaggaaacagtgcgtcaagaaagaactagtcactgggctagggctcacaggcgagctggtggatcctcccttccatgaattcgcctacgagagtctgagaacacgaccagccgctccttaccaagtaccaaccataggggtgtatggcgtgccaggatcaggcaagtctggcatcattaaaagcgcagtcaccaaaaaagatctagtggtgagcgccaagaaagaaaactgtgcagaaattataagggacgtcaagaaaatgaaagggctggacgtcaatgccagaactgtggactcagtgctcttgaatggatgcaaacaccccgtagagaccctgtatattgacgaagcttttgcttgtcatgcaggtactctcagagcgctcatagccattataagacctaaaaaggcagtgctctgcggggatcccaaacagtgcggtttttttaacatgatgtgcctgaaagtgcattttaaccacgagatttgcacacaagtcttccacaaaagcatctctcgccgttgcactaaatctgtgacttcggtcgtctcaaccttgttttacgacaaaaaaatgagaacgacgaatccgaaagagactaagattgtgattgacactaccggcagtaccaaacctaagcaggacgatctcattctcacttgtttcagagggtgggtgaagcagttgcaaatagattacaaaggcaacgaaataatgacggcagctgcctctcaagggctgacccgtaaaggtgtgtatgccgttcggtacaaggtgaatgaaaatcctctgtacgcacccacctcagaacatgtgaacgtcctactgacccgcacggaggaccgcatcgtgtggaaaacactagccggcgacccatggataaaaacactgactgccaagtaccctgggaatttcactgccacgatagaggagtggcaagcagagcatgatgccatcatgaggcacatcttggagagaccggaccctaccgacgtcttccagaataaggcaaacgtgtgttgggccaaggctttagtgccggtgctgaagaccgctggcatagacatgaccactgaacaatggaacactgtggattattttgaaacggacaaagctcactcagcagagatagtattgaaccaactatgcgtgaggttctttggactcgatctggactccggtctattttctgcacccactgttccgttatccattaggaataatcactgggataactccccgtcgcctaacatgtacgggctgaataaagaagtggtccgtcagctctctcgcaggtacccacaactgcctcgggcagttgccactggaagagtctatgacatgaacactggtacactgcgcaattatgatccgcgcataaacctagtacctgtaaacagaagactgcctcatgctttagtcctccaccataatgaacacccacagagtgacttttcttcattcgtcagcaaattgaagggcagaactgtcctggtggtcggggaaaagttgtccgtcccaggcaaaatggttgactggttgtcagaccggcctgaggctaccttcagagctcggctggatttaggcatcccaggtgatgtgcccaaatatgacataatatttgttaatgtgaggaccccatataaataccatcactatcagcagtgtgaagaccatgccattaagcttagcatgttgaccaagaaagcttgtctgcatctgaatcccggcggaacctgtgtcagcataggttatggttacgctgacagggccagcgaaagcatcattggtgctatagcgcggcagttcaagttttcccgggtatgcaaaccgaaatcctcacttgaagagacggaagttctgtttgtattcattgggtacgatcgcaaggcccgtacgcacaatccttacaagctttcatcaaccttgaccaacatttatacaggttccagactccacgaagccggatgtgcaccctcatatcatgtggtgcgaggggatattgccacggccaccgaaggagtgattataaatgctgctaacagcaaaggacaacctggcggaggggtgtgcggagcgctgtataagaaattcccggaaagcttcgatttacagccgatcgaagtaggaaaagcgcgactggtcaaaggtgcagctaaacatatcattcatgccgtaggaccaaacttcaacaaagtttcggaggttgaaggtgacaaacagttggcagaggcttatgagtccatcgctaagattgtcaacgataacaattacaagtcagtagcgattccactgttgtccaccggcatcttttccgggaacaaagatcgactaacccaatcattgaaccatttgctgacagctttagacaccactgatgcagatgtagccatatactgcagggacaagaaatgggaaatgactctcaaggaagcagtggctaggagagaagcagtggaggagatatgcatatccgacgactcttcagtgacagaacctgatgcagagctggtgagggtgcatccgaagagttctttggctggaaggaagggctacagcacaagcgatggcaaaactttctcatatttggaagggaccaagtttcaccaggcggccaaggatatagcagaaattaatgccatgtggcccgttgcaacggaggccaatgagcaggtatgcatgtatatcctcggagaaagcatgagcagtattaggtcgaaatgccccgtcgaagagtcggaagcctccacaccacctagcacgctgccttgcttgtgcatccatgccatgactccagaaagagtacagcgcctaaaagcctcacgtccagaacaaattactgtgtgctcatcctttccattgccgaagtatagaatcactggtgtgcagaagatccaatgctcccagcctatattgttctcaccgaaagtgcctgcgtatattcatccaaggaagtatctcgtggaaacaccaccggtagacgagactccggagccatcggcagagaaccaatccacagaggggacacctgaacaaccaccacttataaccgaggatgagaccaggactagaacgcctgagccgatcatcatcgaagaggaagaagaggatagcataagtttgctgtcagatggcccgacccaccaggtgctgcaagtcgaggcagacattcacgggccgccctctgtatctagctcatcctggtccattcctcatgcatccgactttgatgtggacagtttatccatacttgacaccctggagggagctagcgtgaccagcggggcaacgtcagccgagactaactcttacttcgcaaagagtatggagtttctggcgcgaccggtgcctgcgcctcgaacagtattcaggaaccctccacatcccgctccgcgcacaagaacaccgtcacttgcacccagcagggcctgctcgagaaccagcctagtttccaccccgccaggcgtgaatagggtgatcactagagaggagctcgaggcgcttaccccgtcacgcactcctagcaggtcggtctcgagaaccagcctggtctccaacccgccaggcgtaaatagggtgattacaagagaggagtttgaggcgttcgtagcacaacaacaatgacggtttgatgcgggtgcatacatcttttcctccgacaccggtcaagggcatttacaacaaaaatcagtaaggcaaacggtgctatccgaagtggtgttggagaggaccgaattggagatttcgtatgccccgcgcctcgaccaagaaaaagaagaattactacgcaagaaattacagttaaatcccacacctgctaacagaagcagataccagtccaggaaggtggagaacatgaaagccataacagctagacgtattctgcaaggcctagggcattatttgaaggcagaaggaaaagtggagtgctaccgaaccctgcatcctgttcctttgtattcatctagtgtgaaccgtgccttttcaagccccaaggtcgcagtggaagcctgtaacgccatgttgaaagagaactttccgactgtggcttcttactgtattattccagagtacgatgcctatttggacatggttgacggagcttcatgctgcttagacactgccagtttttgccctgcaaagctgcgcagctttccaaagaaacactcctatttggaacccacaatacgatcggcagtgccttcagcgatccagaacacgctccagaacgtcctggcagctgccacaaaaagaaattgcaatgtcacgcaaatgagagaattgcccgtattggattcggcggcctttaatgtggaatgcttcaagaaatatgcgtgtaataatgaatattgggaaacgtttaaagaaaaccccatcaggcttactgaagaaaacgtggtaaattacattaccaaattaaaaggaccaaaagctgctgctctttttgcgaagacacataatttgaatatgttgcaggacataccaatggacaggtttgtaatggacttaaagagagacgtgaaagtgactccaggaacaaaacatactgaagaacggcccaaggtacaggtgatccaggctgccgatccgctagcaacagcgtatctgtgcggaatccaccgagagctggttaggagattaaatgcggtcctgcttccgaacattcatacactgtttgatatgtcggctgaagactttgacgctattatagccgagcacttccagcctggggattgtgttctggaaactgacatcgcgtcgtttgataaaagtgaggacgacgccatggctctgaccgcgttaatgattctggaagacttaggtgtggacgcagagctgttgacgctgattgaggcggctttcggcgaaatttcatcaatacatttgcccactaaaactaaatttaaattcggagccatgatgaaatctggaatgttcctcacactgtttgtgaacacagtcattaacattgtaatcgcaagcagagtgttgagagaacggctaaccggatcaccatgtgcagcattcattggagatgacaatatcgtgaaaggagtcaaatcggacaaattaatggcagacaggtgcgccacctggttgaatatggaagtcaagattatagatgctgtggtgggcgagaaagcgccttatttctgtggagggtttattttgtgtgactccgtgaccggcacagcgtgccgtgtggcagaccccctaaaaaggctgtttaagcttggcaaacctctggcagcagacgatgaacatgatgatgacaggagaagggcattgcatgaagagtcaacacgctggaaccgagtgggtattctttcagagctgtgcaaggcagtagaatcaaggtatgaaaccgtaggaacttccatcatagttatggccatgactactctagctagcagtgttaaatcattcagctacctgagaggggcccctataactctctacggctaacctgaatggactacgacatagtctagtccgccaagatgttcgtgttcctggtgctgctgcccctcgttagcagccagtgcgtgaatctgaccacccgcacccagctgccaccagcctacacaaacagcttcaccagaggagtgtattaccctgataaggtctttagatcctccgtcctgcattctacgcaggatctcttcttgccattcttcagcaacgtgacatggttccacgccatccacgtttctggcaccaacggcacaaagcgcttcgacaatcctgtgttgccgtttaacgacggcgtttacttcgccagcacagaaaagagcaacatcatccggggctggatcttcggcaccaccctggacagcaaaacccaaagcctgctcatcgtgaacaacgccaccaacgtggtgatcaaggtgtgcgagttccagttctgcaatgatccttttctgggcgtgtactatcacaagaacaacaagagctggatggaaagcgagttcagagtgtattctagcgccaacaactgcacctttgagtacgtgtcccagccctttcttatggacctggaaggcaagcagggcaacttcaagaatctgagagaattcgtgttcaagaacattgatggctacttcaagatctacagcaagcacacccctatcaacctggttcgggacctgccacaaggcttcagcgccctggaacctctggtggacctgcctatcggcatcaacatcacacggttccaaaccctgctggccctgcaccggagctacctgacccccggcgacagcagcagcggctggaccgccggcgctgccgcctattacgtgggctacctgcaacctagaaccttcctgctgaaatacaacgagaacggcacaatcaccgacgccgtggactgtgccctggaccccctgtctgagacaaagtgtaccctgaagtctttcaccgtggagaagggcatctaccagaccagcaacttccgggtgcagcctacagaatctatagtgcggttccctaacatcaccaacctgtgtccttttggcgaggtgttcaacgccactcggttcgcctctgtctacgcctggaaccggaaacggatctctaattgcgtggccgattacagcgtcctgtataactccgccagtttcagcacattcaagtgctacggcgtgtcacccaccaagctgaacgatctgtgcttcaccaatgtgtacgccgatagtttcgtgatccggggcgatgaggtgcggcagatcgcccctggacagacaggcaagatcgccgactacaactacaagctgcctgacgacttcacaggctgtgtgatcgcatggaacagcaacaacctggacagcaaggtgggcggaaactacaactacctgtacagactgttcagaaagtccaacctgaagcctttcgagagagatatatctaccgagatctaccaggccggcagcacaccctgtaatggagtggaaggctttaactgctacttccctctgcaaagctatggatttcaacctacaaatggggttggctaccagccttacagagtggtggtccttagcttcgagctgctccatgcccctgccaccgtgtgcggacctaagaagtccaccaacctggtgaaaaacaagtgcgtgaactttaattttaacggcctgaccggaacaggagtgctgacagaaagcaacaaaaagttcctgcctttccagcagttcggcagagacattgccgacaccacagatgctgttagagacccccagacgctggaaatcctggatatcaccccctgctcttttggcggcgtgagcgtgatcaccccaggcacaaacacaagcaaccaggtggctgtgctgtaccaggacgtgaactgtacagaggtccctgtggcaatccacgccgatcagctgacccctacatggcgggtgtactccactggatctaacgtgttccagacaagggccggatgcctcatcggcgctgagcacgtgaacaattcttacgagtgcgacatccctattggagcgggcatctgcgccagctaccagacacagaccaatagccctcagcaagccgctagcgtggcctcccagagcatcatcgcctacaccatgagcctgggagccgagaactctgtggcctacagcaacaacagcatcgctatccctaccaacttcaccatctctgtcaccaccgaaatcctgcccgtcagtatgaccaaaaccagcgtcgactgcaccatgtacatatgcggcgatagcaccgaatgcagcaacctgctgctgcagtatggctccttctgcacccaacttaacagagccctgactggcatcgccgtggagcaggacaagaatacccaggaggtgttcgcccaggtgaagcagatctacaagacacccccgatcaaggacttcggcggctttaatttctctcagatcctgccagacccatctaaaccctctaagaacagctttatcgaggacctgctgttcaacaaggtgactctggctgacgccggcttcatcaagcagtacggcgattgcctgggcgacattgctgctagagacctgatctgtgcccagaaattcaacggtcttactgtgctgcctcctctgctgacggatgagatgatcgcccagtacaccagcgccctgctggccggcaccatcacatccggctggacattcggcgccggcgcagccctgcagatcccttttgccatgcagatggcctaccggttcaacggaatcggagtgacacagaacgtgctctacgaaaatcagaagttgatcgccaaccagttcaacagcgccatcggcaagattcaggatagtctgagttccaccgccagcgccctgggaaagctgcaggacgtggtcaatcagaatgcccaagccctgaacaccctggtgaagcagctgagcagcaacttcggcgccatcagctctgtgctgaacgacatcctgagtagactggacaaggtggaagccgaagtgcagatcgacagattgatcaccggaagactgcaaagcctgcagacctacgtgacccagcagctgataagagctgctgaaatcagagccagcgctaatctggccgctaccaagatgagcgagtgcgttctgggccagtctaagagagtggacttctgcggaaaaggctaccacctgatgtcctttcctcagtctgccccccacggcgtggtgttcctgcacgtcacatacgtgcccgctcaagagaaaaacttcaccacggcccctgccatctgtcacgacggcaaggcccacttccccagagagggcgtgttcgtgagcaatggcacccactggtttgtgactcagagaaacttctacgagccacagattatcaccacagataacaccttcgtgtctggcaactgcgacgtggtgatcggcatcgtcaacaacacagtgtacgacccactgcaacctgagctggactcattcaaggaggaactggataagtacttcaagaatcacaccagccccgacgttgacctgggcgacatcagcggcattaacgcctctgtggtcaacatccagaaggaaatcgacagactgaatgaggtggccaagaatttgaacgagagcctgattgatctgcaggagctgggcaaatacgagcagtacatcaagtggccttggtacatctggctgggcttcatcgccgggctgatcgccatcgttatggtgacaatcatgctgtgttgcatgacaagctgttgtagctgcctgaaaggctgctgctcctgcggcagctgttgcaagtttgacgaagatgacagcgagcccgtgctgaaaggcgtcaagctgcactacacctgaggcgcgcccacccagcggccgcccgctacgccccaatgatccgaccagcaaaactcgatgtacttccgaggaactgatgtgcataatgcatcaggctggtacattagatccccgcttaccgcgggcaatatagcaacactaaaaactcgatgtacttccgaggaagcgcagtgcataatgctgcgcagtgttgccacataaccactatattaaccatttatctagcggacgccaaaaactcaatgtatttctgaggaagcgtggtgcataatgccacgcagcgtctgcataacttttattatttcttttattaatcaacaaaattttgtttttaacatttcaaaaaaaaaaaaaaaaaaaaaaaaaaaaaaaaaaaaagaagagcgtttaaacacgtgatatctggcctcatgggccttcctttcactgcccgctttccagtcgggaaacctgtcgtgccagctgcattaacatggtcatagctgtttccttgcgtattgggcgctctccgcttcctcgctcactgactcgctgcgctcggtcgttcgggtaaagcctggggtgcctaatgagcaaaaggccagcaaaaggccaggaaccgtaaaaaggccgcgttgctggcgtttttccataggctccgcccccctgacgagcatcacaaaaatcgacgctcaagtcagaggtggcgaaacccgacaggactataaagataccaggcgtttccccctggaagctccctcgtgcgctctcctgttccgaccctgccgcttaccggatacctgtccgcctttctcccttcgggaagcgtggcgctttctcatagctcacgctgtaggtatctcagttcggtgtaggtcgttcgctccaagctgggctgtgtgcacgaaccccccgttcagcccgaccgctgcgccttatccggtaactatcgtcttgagtccaacccggtaagacacgacttatcgccactggcagcagccactggtaacaggattagcagagcgaggtatgtaggcggtgctacagagttcttgaagtggtggcctaactacggctacactagaagaacagtatttggtatctgcgctctgctgaagccagttaccttcggaaaaagagttggtagctcttgatccggcaaacaaaccaccgctggtagcggtggtttttttgtttgcaggcagcagattacgcgcagaaaaaaaggatctcaagaagatcctttgatcttttctacggggtctgacgctcagtggaacgaaaactcacgttaagggattttggtcatgaatacacggtgcctgactgcgttagcaatttaactgtgataaactaccgcattaaagcttatcgatgataagctgtcaaacatgagaattcttagaaaaactcatcgagcatcaaatgaaactgcaatttattcatatcaggattatcaataccatatttttgaaaaagccgtttctgtaatgaaggagaaaactcaccgaggcagttccataggatggcaagatcctggtatcggtctgcgattccgactcgtccaacatcaatacaacctattaatttcccctcgtcaaaaataaggttatcaagtgagaaatcaccatgagtgacgactgaatccggtgagaatggcaaaagcttatgcatttctttccagacttgttcaacaggccagccattacgctcgtcatcaaaatcactcgcatcaaccaaaccgttattcattcgtgattgcgcctgagcgagacgaaatacgcgatcgctgttaaaaggacaattacaaacaggaatcgaatgcaaccggcgcaggaacactgccagcgcatcaacaatattttcacctgaatcaggatattcttctaatacctggaatgctgttttcccggggatcgcagtggtgagtaaccatgcatcatcaggagtacggataaaatgcttgatggtcggaagaggcataaattccgtcagccagtttagtctgaccatctcatctgtaacatcattggcaacgctacctttgccatgtttcagaaacaactctggcgcatcgggcttcccatacaatcgatagattgtcgcacctgattgcccgacattatcgcgagcccatttatacccatataaatcagcatccatgttggaatttaatcgcggcctcgagcaagacgtttcccgttgaatatggctcataacaccccttgtattactgtttatgtaagcagacagttttattgttcatgagcggatacatatttgaatgtatttagaaaaataaacaaataggggttccgcgcacatttccccgaaaagtgccacctaaattgtaagcgttaatattttgttaaaattcgcgttaaatttttgttaaatcagctcattttttaaccaataggccgaaatcggcaaaatcccttataaatcaaaagaatagaccgagatagggttgagtggccgctacagggcgctcccattcgccattcaggctgcgcaactgttgggaagggcgtttcggtgcgggcctcttcgctattacgccagctggcgaaagggggatgtgctgcaaggcgattaagttgggtaacgccagggttttcccagtcacacgcgtaatacgactcactatag

SEQ ID NO: 17 - DNA, 14014 bp, synthetic construct
  misc_feature 1..14014: note = Nucleotide sequence of construct Co59
  source 1..14014: mol_type = other DNA
ataggcggcgcatgagagaagcccagaccaattacctacccaaaatggagaaagttcacgttgacatcgaggaagacagcccattcctcagagctttgcagcggagcttcccgcagtttgaggtagaagccaagcaggtcactgataatgaccatgctaatgccagagcgttttcgcatctggcttcaaaactgatcgaaacggaggtggacccatccgacacgatccttgacattggaagtgcgcccgcccgcagaatgtattctaagcacaagtatcattgtatctgtccgatgagatgtgcggaagatccggacagattgtataagtatgcaactaagctgaagaaaaactgtaaggaaataactgataaggaattggacaagaaaatgaaggagctcgccgccgtcatgagcgaccctgacctggaaactgagactatgtgcctccacgacgacgagtcgtgtcgctacgaagggcaagtcgctgtttaccaggatgtatacgcggttgacggaccgacaagtctctatcaccaagccaataagggagttagagtcgcctactggataggctttgacaccaccccttttatgtttaagaacttggctggagcatatccatcatactctaccaactgggccgacgaaaccgtgttaacggctcgtaacataggcctatgcagctctgacgttatggagcggtcacgtagagggatgtccattcttagaaagaagtatttgaaaccatccaacaatgttctattctctgttggctcgaccatctaccacgagaagagggacttactgaggagctggcacctgccgtctgtatttcacttacgtggcaagcaaaattacacatgtcggtgtgagactatagttagttgcgacgggtacgtcgttaaaagaatagctatcagtccaggcctgtatgggaagccttcaggctatgctgctacgatgcaccgcgagggattcttgtgctgcaaagtgacagacacattgaacggggagagggtctcttttcccgtgtgcacgtatgtgccagctacattgtgtgaccaaatgactggcatactggcaacagatgtcagtgcggacgacgcgcaaaaactgctggttgggctcaaccagcgtatagtcgtcaacggtcgcacccagagaaacaccaataccatgaaaaattaccttttgcccgtagtggcccaggcatttgctaggtgggcaaaggaatataaggaagatcaagaagatgaaaggccactaggactacgagatagacagttagtcatggggtgttgttgggcttttagaaggcacaagataacatctatttataagcgcccggatacccaaaccatcatcaaagtgaacagcgatttccactcattcgtgctgcccaggataggcagtaacacattggagatcgggctgagaacaagaatcaggaaaatgttagaggagcacaaggagccgtcacctctcattaccgccgaggacgtacaagaagctaagtgcgcagccgatgaggctaaggaggtgcgtgaagccgaggagttgcgcgcagctctaccacctttggcagctgatgttgaggagcccactctggaagccgatgtcgacttgatgttacaagaggctggggccggctcagtggagacacctcgtggcttgataaaggttaccagctacgatggcgaggacaagatcggctcttacgctgtgctttctccgcaggctgtactcaagagtgaaaaattatcttgcatccaccctctcgctgaacaagtcatagtgataacacactctggccgaaaagggcgttatgccgtggaaccataccatggtaaagtagtggtgccagagggacatgcaatacccgtccaggactttcaagctctgagtgaaagtgccaccattgtgtacaacgaacgtgagttcgtaaacaggtacctgcaccatattgccacacatggaggagcgctgaacactgatgaagaatattacaaaactgtcaagcccagcgagcacgacggcgaatacctgtacgacatcgacaggaaacagtgcgtcaagaaagaactagtcactgggctagggctcacaggcgagctggtggatcctcccttccatgaattcgcctacgagagtctgagaacacgaccagccgctccttaccaagtaccaaccataggggtgtatggcgtgccaggatcaggcaagtctggcatcattaaaagcgcagtcaccaaaaaagatctagtggtgagcgccaagaaagaaaactgtgcagaaattataagggacgtcaagaaaatgaaagggctggacgtcaatgccagaactgtggactcagtgctcttgaatggatgcaaacaccccgtagagaccctgtatattgacgaagcttttgcttgtcatgcaggtactctcagagcgctcatagccattataagacctaaaaaggcagtgctctgcggggatcccaaacagtgcggtttttttaacatgatgtgcctgaaagtgcattttaaccacgagatttgcacacaagtcttccacaaaagcatctctcgccgttgcactaaatctgtgacttcggtcgtctcaaccttgttttacgacaaaaaaatgagaacgacgaatccgaaagagactaagattgtgattgacactaccggcagtaccaaacctaagcaggacgatctcattctcacttgtttcagagggtgggtgaagcagttgcaaatagattacaaaggcaacgaaataatgacggcagctgcctctcaagggctgacccgtaaaggtgtgtatgccgttcggtacaaggtgaatgaaaatcctctgtacgcacccacctcagaacatgtgaacgtcctactgacccgcacggaggaccgcatcgtgtggaaaacactagccggcgacccatggataaaaacactgactgccaagtaccctgggaatttcactgccacgatagaggagtggcaagcagagcatgatgccatcatgaggcacatcttggagagaccggaccctaccgacgtcttccagaataaggcaaacgtgtgttgggccaaggctttagtgccggtgctgaagaccgctggcatagacatgaccactgaacaatggaacactgtggattattttgaaacggacaaagctcactcagcagagatagtattgaaccaactatgcgtgaggttctttggactcgatctggactccggtctattttctgcacccactgttccgttatccattaggaataatcactgggataactccccgtcgcctaacatgtacgggctgaataaagaagtggtccgtcagctctctcgcaggtacccacaactgcctcgggcagttgccactggaagagtctatgacatgaacactggtacactgcgcaattatgatccgcgcataaacctagtacctgtaaacagaagactgcctcatgctttagtcctccaccataatgaacacccacagagtgacttttcttcattcgtcagcaaattgaagggcagaactgtcctggtggtcggggaaaagttgtccgtcccaggcaaaatggttgactggttgtcagaccggcctgaggctaccttcagagctcggctggatttaggcatcccaggtgatgtgcccaaatatgacataatatttgttaatgtgaggaccccatataaataccatcactatcagcagtgtgaagaccatgccattaagcttagcatgttgaccaagaaagcttgtctgcatctgaatcccggcggaacctgtgtcagcataggttatggttacgctgacagggccagcgaaagcatcattggtgctatagcgcggcagttcaagttttcccgggtatgcaaaccgaaatcctcacttgaagagacggaagttctgtttgtattcattgggtacgatcgcaaggcccgtacgcacaatccttacaagctttcatcaaccttgaccaacatttatacaggttccagactccacgaagccggatgtgcaccctcatatcatgtggtgcgaggggatattgccacggccaccgaaggagtgattataaatgctgctaacagcaaaggacaacctggcggaggggtgtgcggagcgctgtataagaaattcccggaaagcttcgatttacagccgatcgaagtaggaaaagcgcgactggtcaaaggtgcagctaaacatatcattcatgccgtaggaccaaacttcaacaaagtttcggaggttgaaggtgacaaacagttggcagaggcttatgagtccatcgctaagattgtcaacgataacaattacaagtcagtagcgattccactgttgtccaccggcatcttttccgggaacaaagatcgactaacccaatcattgaaccatttgctgacagctttagacaccactgatgcagatgtagccatatactgcagggacaagaaatgggaaatgactctcaaggaagcagtggctaggagagaagcagtggaggagatatgcatatccgacgactcttcagtgacagaacctgatgcagagctggtgagggtgcatccgaagagttctttggctggaaggaagggctacagcacaagcgatggcaaaactttctcatatttggaagggaccaagtttcaccaggcggccaaggatatagcagaaattaatgccatgtggcccgttgcaacggaggccaatgagcaggtatgcatgtatatcctcggagaaagcatgagcagtattaggtcgaaatgccccgtcgaagagtcggaagcctccacaccacctagcacgctgccttgcttgtgcatccatgccatgactccagaaagagtacagcgcctaaaagcctcacgtccagaacaaattactgtgtgctcatcctttccattgccgaagtatagaatcactggtgtgcagaagatccaatgctcccagcctatattgttctcaccgaaagtgcctgcgtatattcatccaaggaagtatctcgtggaaacaccaccggtagacgagactccggagccatcggcagagaaccaatccacagaggggacacctgaacaaccaccacttataaccgaggatgagaccaggactagaacgcctgagccgatcatcatcgaagaggaagaagaggatagcataagtttgctgtcagatggcccgacccaccaggtgctgcaagtcgaggcagacattcacgggccgccctctgtatctagctcatcctggtccattcctcatgcatccgactttgatgtggacagtttatccatacttgacaccctggagggagctagcgtgaccagcggggcaacgtcagccgagactaactcttacttcgcaaagagtatggagtttctggcgcgaccggtgcctgcgcctcgaacagtattcaggaaccctccacatcccgctccgcgcacaagaacaccgtcacttgcacccagcagggcctgctcgagaaccagcctagtttccaccccgccaggcgtgaatagggtgatcactagagaggagctcgaggcgcttaccccgtcacgcactcctagcaggtcggtctcgagaaccagcctggtctccaacccgccaggcgtaaatagggtgattacaagagaggagtttgaggcgttcgtagcacaacaacaatgacggtttgatgcgggtgcatacatcttttcctccgacaccggtcaagggcatttacaacaaaaatcagtaaggcaaacggtgctatccgaagtggtgttggagaggaccgaattggagatttcgtatgccccgcgcctcgaccaagaaaaagaagaattactacgcaagaaattacagttaaatcccacacctgctaacagaagcagataccagtccaggaaggtggagaacatgaaagccataacagctagacgtattctgcaaggcctagggcattatttgaaggcagaaggaaaagtggagtgctaccgaaccctgcatcctgttcctttgtattcatctagtgtgaaccgtgccttttcaagccccaaggtcgcagtggaagcctgtaacgccatgttgaaagagaactttccgactgtggcttcttactgtattattccagagtacgatgcctatttggacatggttgacggagcttcatgctgcttagacactgccagtttttgccctgcaaagctgcgcagctttccaaagaaacactcctatttggaacccacaatacgatcggcagtgccttcagcgatccagaacacgctccagaacgtcctggcagctgccacaaaaagaaattgcaatgtcacgcaaatgagagaattgcccgtattggattcggcggcctttaatgtggaatgcttcaagaaatatgcgtgtaataatgaatattgggaaacgtttaaagaaaaccccatcaggcttactgaagaaaacgtggtaaattacattaccaaattaaaaggaccaaaagctgctgctctttttgcgaagacacataatttgaatatgttgcaggacataccaatggacaggtttgtaatggacttaaagagagacgtgaaagtgactccaggaacaaaacatactgaagaacggcccaaggtacaggtgatccaggctgccgatccgctagcaacagcgtatctgtgcggaatccaccgagagctggttaggagattaaatgcggtcctgcttccgaacattcatacactgtttgatatgtcggctgaagactttgacgctattatagccgagcacttccagcctggggattgtgttctggaaactgacatcgcgtcgtttgataaaagtgaggacgacgccatggctctgaccgcgttaatgattctggaagacttaggtgtggacgcagagctgttgacgctgattgaggcggctttcggcgaaatttcatcaatacatttgcccactaaaactaaatttaaattcggagccatgatgaaatctggaatgttcctcacactgtttgtgaacacagtcattaacattgtaatcgcaagcagagtgttgagagaacggctaaccggatcaccatgtgcagcattcattggagatgacaatatcgtgaaaggagtcaaatcggacaaattaatggcagacaggtgcgccacctggttgaatatggaagtcaagattatagatgctgtggtgggcgagaaagcgccttatttctgtggagggtttattttgtgtgactccgtgaccggcacagcgtgccgtgtggcagaccccctaaaaaggctgtttaagcttggcaaacctctggcagcagacgatgaacatgatgatgacaggagaagggcattgcatgaagagtcaacacgctggaaccgagtgggtattctttcagagctgtgcaaggcagtagaatcaaggtatgaaaccgtaggaacttccatcatagttatggccatgactactctagctagcagtgttaaatcattcagctacctgagaggggcccctataactctctacggctaacctgaatggactacgacatagtctagtccgccaagatgttcgtgttcctggtgctgctgcccctcgttagcagccagtgcgtgaatctgaccacccgcacccagctgccaccagcctacacaaacagcttcaccagaggagtgtattaccctgataaggtctttagatcctccgtcctgcattctacgcaggatctcttcttgccattcttcagcaacgtgacatggttccacgccatccacgtttctggcaccaacggcacaaagcgcttcgacaatcctgtgttgccgtttaacgacggcgtttacttcgccagcacagaaaagagcaacatcatccggggctggatcttcggcaccaccctggacagcaaaacccaaagcctgctcatcgtgaacaacgccaccaacgtggtgatcaaggtgtgcgagttccagttctgcaatgatccttttctgggcgtgtactatcacaagaacaacaagagctggatggaaagcgagttcagagtgtattctagcgccaacaactgcacctttgagtacgtgtcccagccctttcttatggacctggaaggcaagcagggcaacttcaagaatctgagagaattcgtgttcaagaacattgatggctacttcaagatctacagcaagcacacccctatcaacctggttcgggacctgccacaaggcttcagcgccctggaacctctggtggacctgcctatcggcatcaacatcacacggttccaaaccctgctggccctgcaccggagctacctgacccccggcgacagcagcagcggctggaccgccggcgctgccgcctattacgtgggctacctgcaacctagaaccttcctgctgaaatacaacgagaacggcacaatcaccgacgccgtggactgtgccctggaccccctgtctgagacaaagtgtaccctgaagtctttcaccgtggagaagggcatctaccagaccagcaacttccgggtgcagcctacagaatctatagtgcggttccctaacatcaccaacctgtgtccttttggcgaggtgttcaacgccactcggttcgcctctgtctacgcctggaaccggaaacggatctctaattgcgtggccgattacagcgtcctgtataactccgccagtttcagcacattcaagtgctacggcgtgtcacccaccaagctgaacgatctgtgcttcaccaatgtgtacgccgatagtttcgtgatccggggcgatgaggtgcggcagatcgcccctggacagacaggcaagatcgccgactacaactacaagctgcctgacgacttcacaggctgtgtgatcgcatggaacagcaacaacctggacagcaaggtgggcggaaactacaactacctgtacagactgttcagaaagtccaacctgaagcctttcgagagagatatatctaccgagatctaccaggccggcagcacaccctgtaatggagtggaaggctttaactgctacttccctctgcaaagctatggatttcaacctacaaatggggttggctaccagccttacagagtggtggtccttagcttcgagctgctccatgcccctgccaccgtgtgcggacctaagaagtccaccaacctggtgaaaaacaagtgcgtgaactttaattttaacggcctgaccggaacaggagtgctgacagaaagcaacaaaaagttcctgcctttccagcagttcggcagagacattgccgacaccacagatgctgttagagacccccagacgctggaaatcctggatatcaccccctgctcttttggcggcgtgagcgtgatcaccccaggcacaaacacaagcaaccaggtggctgtgctgtaccagggcgtgaactgtacagaggtccctgtggcaatccacgccgatcagctgacccctacatggcgggtgtactccactggatctaacgtgttccagacaagggccggatgcctcatcggcgctgagcacgtgaacaattcttacgagtgcgacatccctattggagcgggcatctgcgccagctaccagacacagaccaatagccctcagcaagccgctagcgtggcctcccagagcatcatcgcctacaccatgagcctgggagccgagaactctgtggcctacagcaacaacagcatcgctatccctaccaacttcaccatctctgtcaccaccgaaatcctgcccgtcagtatgaccaaaaccagcgtcgactgcaccatgtacatatgcggcgatagcaccgaatgcagcaacctgctgctgcagtatggctccttctgcacccaacttaacagagccctgactggcatcgccgtggagcaggacaagaatacccaggaggtgttcgcccaggtgaagcagatctacaagacacccccgatcaaggacttcggcggctttaatttctctcagatcctgccagacccatctaaaccctctaagaacagctttatcgaggacctgctgttcaacaaggtgactctggctgacgccggcttcatcaagcagtacggcgattgcctgggcgacattgctgctagagacctgatctgtgcccagaaattcaacggtcttactgtgctgcctcctctgctgacggatgagatgatcgcccagtacaccagcgccctgctggccggcaccatcacatccggctggacattcggcgccggcgcagccctgcagatcccttttgccatgcagatggcctaccggttcaacggaatcggagtgacacagaacgtgctctacgaaaatcagaagttgatcgccaaccagttcaacagcgccatcggcaagattcaggatagtctgagttccaccgccagcgccctgggaaagctgcaggacgtggtcaatcagaatgcccaagccctgaacaccctggtgaagcagctgagcagcaacttcggcgccatcagctctgtgctgaacgacatcctgagtagactggacaaggtggaagccgaagtgcagatcgacagattgatcaccggaagactgcaaagcctgcagacctacgtgacccagcagctgataagagctgctgaaatcagagccagcgctaatctggccgctaccaagatgagcgagtgcgttctgggccagtctaagagagtggacttctgcggaaaaggctaccacctgatgtcctttcctcagtctgccccccacggcgtggtgttcctgcacgtcacatacgtgcccgctcaagagaaaaacttcaccacggcccctgccatctgtcacgacggcaaggcccacttccccagagagggcgtgttcgtgagcaatggcacccactggtttgtgactcagagaaacttctacgagccacagattatcaccacagataacaccttcgtgtctggcaactgcgacgtggtgatcggcatcgtcaacaacacagtgtacgacccactgcaacctgagctggactcattcaaggaggaactggataagtacttcaagaatcacaccagccccgacgttgacctgggcgacatcagcggcattaacgcctctgtggtcaacatccagaaggaaatcgacagactgaatgaggtggccaagaatttgaacgagagcctgattgatctgcaggagctgggcaaatacgagcagtacatcaagtggccttggtacatctggctgggcttcatcgccgggctgatcgccatcgttatggtgacaatcatgctgtgttgcatgacaagctgttgtagctgcctgaaaggctgctgctcctgcggcagctgttgcaagtttgacgaagatgacagcgagcccgtgctgaaaggcgtcaagctgcactacacctgaggcgcgcccacccagcggccgcccgctacgccccaatgatccgaccagcaaaactcgatgtacttccgaggaactgatgtgcataatgcatcaggctggtacattagatccccgcttaccgcgggcaatatagcaacactaaaaactcgatgtacttccgaggaagcgcagtgcataatgctgcgcagtgttgccacataaccactatattaaccatttatctagcggacgccaaaaactcaatgtatttctgaggaagcgtggtgcataatgccacgcagcgtctgcataacttttattatttcttttattaatcaacaaaattttgtttttaacatttcaaaaaaaaaaaaaaaaaaaaaaaaaaaaaaaaaaaaagaagagcgtttaaacacgtgatatctggcctcatgggccttcctttcactgcccgctttccagtcgggaaacctgtcgtgccagctgcattaacatggtcatagctgtttccttgcgtattgggcgctctccgcttcctcgctcactgactcgctgcgctcggtcgttcgggtaaagcctggggtgcctaatgagcaaaaggccagcaaaaggccaggaaccgtaaaaaggccgcgttgctggcgtttttccataggctccgcccccctgacgagcatcacaaaaatcgacgctcaagtcagaggtggcgaaacccgacaggactataaagataccaggcgtttccccctggaagctccctcgtgcgctctcctgttccgaccctgccgcttaccggatacctgtccgcctttctcccttcgggaagcgtggcgctttctcatagctcacgctgtaggtatctcagttcggtgtaggtcgttcgctccaagctgggctgtgtgcacgaaccccccgttcagcccgaccgctgcgccttatccggtaactatcgtcttgagtccaacccggtaagacacgacttatcgccactggcagcagccactggtaacaggattagcagagcgaggtatgtaggcggtgctacagagttcttgaagtggtggcctaactacggctacactagaagaacagtatttggtatctgcgctctgctgaagccagttaccttcggaaaaagagttggtagctcttgatccggcaaacaaaccaccgctggtagcggtggtttttttgtttgcaggcagcagattacgcgcagaaaaaaaggatctcaagaagatcctttgatcttttctacggggtctgacgctcagtggaacgaaaactcacgttaagggattttggtcatgaatacacggtgcctgactgcgttagcaatttaactgtgataaactaccgcattaaagcttatcgatgataagctgtcaaacatgagaattcttagaaaaactcatcgagcatcaaatgaaactgcaatttattcatatcaggattatcaataccatatttttgaaaaagccgtttctgtaatgaaggagaaaactcaccgaggcagttccataggatggcaagatcctggtatcggtctgcgattccgactcgtccaacatcaatacaacctattaatttcccctcgtcaaaaataaggttatcaagtgagaaatcaccatgagtgacgactgaatccggtgagaatggcaaaagcttatgcatttctttccagacttgttcaacaggccagccattacgctcgtcatcaaaatcactcgcatcaaccaaaccgttattcattcgtgattgcgcctgagcgagacgaaatacgcgatcgctgttaaaaggacaattacaaacaggaatcgaatgcaaccggcgcaggaacactgccagcgcatcaacaatattttcacctgaatcaggatattcttctaatacctggaatgctgttttcccggggatcgcagtggtgagtaaccatgcatcatcaggagtacggataaaatgcttgatggtcggaagaggcataaattccgtcagccagtttagtctgaccatctcatctgtaacatcattggcaacgctacctttgccatgtttcagaaacaactctggcgcatcgggcttcccatacaatcgatagattgtcgcacctgattgcccgacattatcgcgagcccatttatacccatataaatcagcatccatgttggaatttaatcgcggcctcgagcaagacgtttcccgttgaatatggctcataacaccccttgtattactgtttatgtaagcagacagttttattgttcatgagcggatacatatttgaatgtatttagaaaaataaacaaataggggttccgcgcacatttccccgaaaagtgccacctaaattgtaagcgttaatattttgttaaaattcgcgttaaatttttgttaaatcagctcattttttaaccaataggccgaaatcggcaaaatcccttataaatcaaaagaatagaccgagatagggttgagtggccgctacagggcgctcccattcgccattcaggctgcgcaactgttgggaagggcgtttcggtgcgggcctcttcgctattacgccagctggcgaaagggggatgtgctgcaaggcgattaagttgggtaacgccagggttttcccagtcacacgcgtaatacgactcactatag

SEQ ID NO: 18 - protein, 1273 aa, synthetic construct
  REGION 1..1273: note = Amino acid sequence of SARS-CoV-2 spike (S) protein full length wt (cleavable)
MFVFLVLLPLVSSQCVNLTTRTQLPPAYTNSFTRGVYYPDKVFRSSVLHSTQDLFLPFFSNVTWFHAIHVSGTNGTKRFDNPVLPFNDGVYFASTEKSNIIRGWIFGTTLDSKTQSLLIVNNATNVVIKVCEFQFCNDPFLGVYYHKNNKSWMESEFRVYSSANNCTFEYVSQPFLMDLEGKQGNFKNLREFVFKNIDGYFKIYSKHTPINLVRDLPQGFSALEPLVDLPIGINITRFQTLLALHRSYLTPGDSSSGWTAGAAAYYVGYLQPRTFLLKYNENGTITDAVDCALDPLSETKCTLKSFTVEKGIYQTSNFRVQPTESIVRFPNITNLCPFGEVFNATRFASVYAWNRKRISNCVADYSVLYNSASFSTFKCYGVSPTKLNDLCFTNVYADSFVIRGDEVRQIAPGQTGKIADYNYKLPDDFTGCVIAWNSNNLDSKVGGNYNYLYRLFRKSNLKPFERDISTEIYQAGSTPCNGVEGFNCYFPLQSYGFQPTNGVGYQPYRVVVLSFELLHAPATVCGPKKSTNLVKNKCVNFNFNGLTGTGVLTESNKKFLPFQQFGRDIADTTDAVRDPQTLEILDITPCSFGGVSVITPGTNTSNQVAVLYQDVNCTEVPVAIHADQLTPTWRVYSTGSNVFQTRAGCLIGAEHVNNSYECDIPIGAGICASYQTQTNSPRRARSVASQSIIAYTMSLGAENSVAYSNNSIAIPTNFTISVTTEILPVSMTKTSVDCTMYICGDSTECSNLLLQYGSFCTQLNRALTGIAVEQDKNTQEVFAQVKQIYKTPPIKDFGGFNFSQILPDPSKPSKRSFIEDLLFNKVTLADAGFIKQYGDCLGDIAARDLICAQKFNGLTVLPPLLTDEMIAQYTSALLAGTITSGWTFGAGAALQIPFAMQMAYRFNGIGVTQNVLYENQKLIANQFNSAIGKIQDSLSSTASALGKLQDVVNQNAQALNTLVKQLSSNFGAISSVLNDILSRLDKVEAEVQIDRLITGRLQSLQTYVTQQLIRAAEIRASANLAATKMSECVLGQSKRVDFCGKGYHLMSFPQSAPHGVVFLHVTYVPAQEKNFTTAPAICHDGKAHFPREGVFVSNGTHWFVTQRNFYEPQIITTDNTFVSGNCDVVIGIVNNTVYDPLQPELDSFKEELDKYFKNHTSPDVDLGDISGINASVVNIQKEIDRLNEVAKNLNESLIDLQELGKYEQYIKWPWYIWLGFIAGLIAIVMVTIMLCCMTSCCSCLKGCCSCGSCCKFDEDDSEPVLKGVKLHYT

SEQ ID NO: 19 - DNA, 3813 bp, synthetic construct
  misc_feature 1..3813: note = Nucleotide sequence of SARS-CoV-2 spike (S) protein uncleavable (RRAR-QQAA; del69-70; delY144; N501Y; D614G)
  source 1..3813: mol_type = other DNA
atgttcgtgttcctggtgctgctgcccctcgttagcagccagtgcgtgaatctgaccacccgcacccagctgccaccagcctacacaaacagcttcaccagaggagtgtattaccctgataaggtctttagatcctccgtcctgcattctacgcaggatctcttcttgccattcttcagcaacgtgacatggttccacgccatctctggcaccaacggcacaaagcgcttcgacaatcctgtgttgccgtttaacgacggcgtttacttcgccagcacagaaaagagcaacatcatccggggctggatcttcggcaccaccctggacagcaaaacccaaagcctgctcatcgtgaacaacgccaccaacgtggtgatcaaggtgtgcgagttccagttctgcaatgatccttttctgggcgtgtatcacaagaacaacaagagctggatggaaagcgagttcagagtgtattctagcgccaacaactgcacctttgagtacgtgtcccagccctttcttatggacctggaaggcaagcagggcaacttcaagaatctgagagaattcgtgttcaagaacattgatggctacttcaagatctacagcaagcacacccctatcaacctggttcgggacctgccacaaggcttcagcgccctggaacctctggtggacctgcctatcggcatcaacatcacacggttccaaaccctgctggccctgcaccggagctacctgacccccggcgacagcagcagcggctggaccgccggcgctgccgcctattacgtgggctacctgcaacctagaaccttcctgctgaaatacaacgagaacggcacaatcaccgacgccgtggactgtgccctggaccccctgtctgagacaaagtgtaccctgaagtctttcaccgtggagaagggcatctaccagaccagcaacttccgggtgcagcctacagaatctatagtgcggttccctaacatcaccaacctgtgtccttttggcgaggtgttcaacgccactcggttcgcctctgtctacgcctggaaccggaaacggatctctaattgcgtggccgattacagcgtcctgtataactccgccagtttcagcacattcaagtgctacggcgtgtcacccaccaagctgaacgatctgtgcttcaccaatgtgtacgccgatagtttcgtgatccggggcgatgaggtgcggcagatcgcccctggacagacaggcaagatcgccgactacaactacaagctgcctgacgacttcacaggctgtgtgatcgcatggaacagcaacaacctggacagcaaggtgggcggaaactacaactacctgtacagactgttcagaaagtccaacctgaagcctttcgagagagatatatctaccgagatctaccaggccggcagcacaccctgtaatggagtggaaggctttaactgctacttccctctgcaaagctatggatttcaacctacatatggggttggctaccagccttacagagtggtggtccttagcttcgagctgctccatgcccctgccaccgtgtgcggacctaagaagtccaccaacctggtgaaaaacaagtgcgtgaactttaattttaacggcctgaccggaacaggagtgctgacagaaagcaacaaaaagttcctgcctttccagcagttcggcagagacattgccgacaccacagatgctgttagagacccccagacgctggaaatcctggatatcaccccctgctcttttggcggcgtgagcgtgatcaccccaggcacaaacacaagcaaccaggtggctgtgctgtaccagggcgtgaactgtacagaggtccctgtggcaatccacgccgatcagctgacccctacatggcgggtgtactccactggatctaacgtgttccagacaagggccggatgcctcatcggcgctgagcacgtgaacaattcttacgagtgcgacatccctattggagcgggcatctgcgccagctaccagacacagaccaatagccctcagcaagccgctagcgtggcctcccagagcatcatcgcctacaccatgagcctgggagccgagaactctgtggcctacagcaacaacagcatcgctatccctaccaacttcaccatctctgtcaccaccgaaatcctgcccgtcagtatgaccaaaaccagcgtcgactgcaccatgtacatatgcggcgatagcaccgaatgcagcaacctgctgctgcagtatggctccttctgcacccaacttaacagagccctgactggcatcgccgtggagcaggacaagaatacccaggaggtgttcgcccaggtgaagcagatctacaagacacccccgatcaaggacttcggcggctttaatttctctcagatcctgccagacccatctaaaccctctaagcggagctttatcgaggacctgctgttcaacaaggtgactctggctgacgccggcttcatcaagcagtacggcgattgcctgggcgacattgctgctagagacctgatctgtgcccagaaattcaacggtcttactgtgctgcctcctctgctgacggatgagatgatcgcccagtacaccagcgccctgctggccggcaccatcacatccggctggacattcggcgccggcgcagccctgcagatcccttttgccatgcagatggcctaccggttcaacggaatcggagtgacacagaacgtgctctacgaaaatcagaagttgatcgccaaccagttcaacagcgccatcggcaagattcaggatagtctgagttccaccgccagcgccctgggaaagctgcaggacgtggtcaatcagaatgcccaagccctgaacaccctggtgaagcagctgagcagcaacttcggcgccatcagctctgtgctgaacgacatcctgagtagactggacaaggtggaagccgaagtgcagatcgacagattgatcaccggaagactgcaaagcctgcagacctacgtgacccagcagctgataagagctgctgaaatcagagccagcgctaatctggccgctaccaagatgagcgagtgcgttctgggccagtctaagagagtggacttctgcggaaaaggctaccacctgatgtcctttcctcagtctgccccccacggcgtggtgttcctgcacgtcacatacgtgcccgctcaagagaaaaacttcaccacggcccctgccatctgtcacgacggcaaggcccacttccccagagagggcgtgttcgtgagcaatggcacccactggtttgtgactcagagaaacttctacgagccacagattatcaccacagataacaccttcgtgtctggcaactgcgacgtggtgatcggcatcgtcaacaacacagtgtacgacccactgcaacctgagctggactcattcaaggaggaactggataagtacttcaagaatcacaccagccccgacgttgacctgggcgacatcagcggcattaacgcctctgtggtcaacatccagaaggaaatcgacagactgaatgaggtggccaagaatttgaacgagagcctgattgatctgcaggagctgggcaaatacgagcagtacatcaagtggccttggtacatctggctgggcttcatcgccgggctgatcgccatcgttatggtgacaatcatgctgtgttgcatgacaagctgttgtagctgcctgaaaggctgctgctcctgcggcagctgttgcaagtttgacgaagatgacagcgagcccgtgctgaaaggcgtcaagctgcactacacctga

SEQ ID NO: 20 - DNA, 3813 bp, synthetic construct
  misc_feature 1..3813: note = Nucleotide sequence of SARS-CoV-2 spike (S) protein uncleavable (RRAR-QQAA; del242-244; K417N; E484K; N501Y; D614G)
  source 1..3813: mol_type = other DNA
atgttcgtgttcctggtgctgctgcccctcgttagcagccagtgcgtgaatctgaccacccgcacccagctgccaccagcctacacaaacagcttcaccagaggagtgtattaccctgataaggtctttagatcctccgtcctgcattctacgcaggatctcttcttgccattcttcagcaacgtgacatggttccacgccatccacgtttctggcaccaacggcacaaagcgcttcgacaatcctgtgttgccgtttaacgacggcgtttacttcgccagcacagaaaagagcaacatcatccggggctggatcttcggcaccaccctggacagcaaaacccaaagcctgctcatcgtgaacaacgccaccaacgtggtgatcaaggtgtgcgagttccagttctgcaatgatccttttctgggcgtgtactatcacaagaacaacaagagctggatggaaagcgagttcagagtgtattctagcgccaacaactgcacctttgagtacgtgtcccagccctttcttatggacctggaaggcaagcagggcaacttcaagaatctgagagaattcgtgttcaagaacattgatggctacttcaagatctacagcaagcacacccctatcaacctggttcgggacctgccacaaggcttcagcgccctggaacctctggtggacctgcctatcggcatcaacatcacacggttccaaaccctgcaccggagctacctgacccccggcgacagcagcagcggctggaccgccggcgctgccgcctattacgtgggctacctgcaacctagaaccttcctgctgaaatacaacgagaacggcacaatcaccgacgccgtggactgtgccctggaccccctgtctgagacaaagtgtaccctgaagtctttcaccgtggagaagggcatctaccagaccagcaacttccgggtgcagcctacagaatctatagtgcggttccctaacatcaccaacctgtgtccttttggcgaggtgttcaacgccactcggttcgcctctgtctacgcctggaaccggaaacggatctctaattgcgtggccgattacagcgtcctgtataactccgccagtttcagcacattcaagtgctacggcgtgtcacccaccaagctgaacgatctgtgcttcaccaatgtgtacgccgatagtttcgtgatccggggcgatgaggtgcggcagatcgcccctggacagacaggcaacatcgccgactacaactacaagctgcctgacgacttcacaggctgtgtgatcgcatggaacagcaacaacctggacagcaaggtgggcggaaactacaactacctgtacagactgttcagaaagtccaacctgaagcctttcgagagagatatatctaccgagatctaccaggccggcagcacaccctgtaatggagtgaaaggctttaactgctacttccctctgcaaagctatggatttcaacctacatatggggttggctaccagccttacagagtggtggtccttagcttcgagctgctccatgcccctgccaccgtgtgcggacctaagaagtccaccaacctggtgaaaaacaagtgcgtgaactttaattttaacggcctgaccggaacaggagtgctgacagaaagcaacaaaaagttcctgcctttccagcagttcggcagagacattgccgacaccacagatgctgttagagacccccagacgctggaaatcctggatatcaccccctgctcttttggcggcgtgagcgtgatcaccccaggcacaaacacaagcaaccaggtggctgtgctgtaccagggcgtgaactgtacagaggtccctgtggcaatccacgccgatcagctgacccctacatggcgggtgtactccactggatctaacgtgttccagacaagggccggatgcctcatcggcgctgagcacgtgaacaattcttacgagtgcgacatccctattggagcgggcatctgcgccagctaccagacacagaccaatagccctcagcaagccgctagcgtggcctcccagagcatcatcgcctacaccatgagcctgggagccgagaactctgtggcctacagcaacaacagcatcgctatccctaccaacttcaccatctctgtcaccaccgaaatcctgcccgtcagtatgaccaaaaccagcgtcgactgcaccatgtacatatgcggcgatagcaccgaatgcagcaacctgctgctgcagtatggctccttctgcacccaacttaacagagccctgactggcatcgccgtggagcaggacaagaatacccaggaggtgttcgcccaggtgaagcagatctacaagacacccccgatcaaggacttcggcggctttaatttctctcagatcctgccagacccatctaaaccctctaagcggagctttatcgaggacctgctgttcaacaaggtgactctggctgacgccggcttcatcaagcagtacggcgattgcctgggcgacattgctgctagagacctgatctgtgcccagaaattcaacggtcttactgtgctgcctcctctgctgacggatgagatgatcgcccagtacaccagcgccctgctggccggcaccatcacatccggctggacattcggcgccggcgcagccctgcagatcccttttgccatgcagatggcctaccggttcaacggaatcggagtgacacagaacgtgctctacgaaaatcagaagttgatcgccaaccagttcaacagcgccatcggcaagattcaggatagtctgagttccaccgccagcgccctgggaaagctgcaggacgtggtcaatcagaatgcccaagccctgaacaccctggtgaagcagctgagcagcaacttcggcgccatcagctctgtgctgaacgacatcctgagtagactggacaaggtggaagccgaagtgcagatcgacagattgatcaccggaagactgcaaagcctgcagacctacgtgacccagcagctgataagagctgctgaaatcagagccagcgctaatctggccgctaccaagatgagcgagtgcgttctgggccagtctaagagagtggacttctgcggaaaaggctaccacctgatgtcctttcctcagtctgccccccacggcgtggtgttcctgcacgtcacatacgtgcccgctcaagagaaaaacttcaccacggcccctgccatctgtcacgacggcaaggcccacttccccagagagggcgtgttcgtgagcaatggcacccactggtttgtgactcagagaaacttctacgagccacagattatcaccacagataacaccttcgtgtctggcaactgcgacgtggtgatcggcatcgtcaacaacacagtgtacgacccactgcaacctgagctggactcattcaaggaggaactggataagtacttcaagaatcacaccagccccgacgttgacctgggcgacatcagcggcattaacgcctctgtggtcaacatccagaaggaaatcgacagactgaatgaggtggccaagaatttgaacgagagcctgattgatctgcaggagctgggcaaatacgagcagtacatcaagtggccttggtacatctggctgggcttcatcgccgggctgatcgccatcgttatggtgacaatcatgctgtgttgcatgacaagctgttgtagctgcctgaaaggctgctgctcctgcggcagctgttgcaagtttgacgaagatgacagcgagcccgtgctgaaaggcgtcaagctgcactacacctga

SEQ ID NO: 21 - DNA, 3804 bp, synthetic construct
  misc_feature 1..3804: note = Nucleotide sequence of SARS-CoV-2 spike (S) protein uncleavable (RRAR-QQAA; del69-70; del242-244; K417N; E484K; N501Y; D614G)
  source 1..3804: mol_type = other DNA
atgttcgtgttcctggtgctgctgcccctcgttagcagccagtgcgtgaatctgaccacccgcacccagctgccaccagcctacacaaacagcttcaccagaggagtgtattaccctgataaggtctttagatcctccgtcctgcattctacgcaggatctcttcttgccattcttcagcaacgtgacatggttccacgccatctctggcaccaacggcacaaagcgcttcgacaatcctgtgttgccgtttaacgacggcgtttacttcgccagcacagaaaagagcaacatcatccggggctggatcttcggcaccaccctggacagcaaaacccaaagcctgctcatcgtgaacaacgccaccaacgtggtgatcaaggtgtgcgagttccagttctgcaatgatccttttctgggcgtgtatcacaagaacaacaagagctggatggaaagcgagttcagagtgtattctagcgccaacaactgcacctttgagtacgtgtcccagccctttcttatggacctggaaggcaagcagggcaacttcaagaatctgagagaattcgtgttcaagaacattgatggctacttcaagatctacagcaagcacacccctatcaacctggttcgggacctgccacaaggcttcagcgccctggaacctctggtggacctgcctatcggcatcaacatcacacggttccaaaccctgcaccggagctacctgacccccggcgacagcagcagcggctggaccgccggcgctgccgcctattacgtgggctacctgcaacctagaaccttcctgctgaaatacaacgagaacggcacaatcaccgacgccgtggactgtgccctggaccccctgtctgagacaaagtgtaccctgaagtctttcaccgtggagaagggcatctaccagaccagcaacttccgggtgcagcctacagaatctatagtgcggttccctaacatcaccaacctgtgtccttttggcgaggtgttcaacgccactcggttcgcctctgtctacgcctggaaccggaaacggatctctaattgcgtggccgattacagcgtcctgtataactccgccagtttcagcacattcaagtgctacggcgtgtcacccaccaagctgaacgatctgtgcttcaccaatgtgtacgccgatagtttcgtgatccggggcgatgaggtgcggcagatcgcccctggacagacaggcaacatcgccgactacaactacaagctgcctgacgacttcacaggctgtgtgatcgcatggaacagcaacaacctggacagcaaggtgggcggaaactacaactacctgtacagactgttcagaaagtccaacctgaagcctttcgagagagatatatctaccgagatctaccaggccggcagcacaccctgtaatggagtgaaaggctttaactgctacttccctctgcaaagctatggatttcaacctacatatggggttggctaccagccttacagagtggtggtccttagcttcgagctgctccatgcccctgccaccgtgtgcggacctaagaagtccaccaacctggtgaaaaacaagtgcgtgaactttaattttaacggcctgaccggaacaggagtgctgacagaaagcaacaaaaagttcctgcctttccagcagttcggcagagacattgccgacaccacagatgctgttagagacccccagacgctggaaatcctggatatcaccccctgctcttttggcggcgtgagcgtgatcaccccaggcacaaacacaagcaaccaggtggctgtgctgtaccagggcgtgaactgtacagaggtccctgtggcaatccacgccgatcagctgacccctacatggcgggtgtactccactggatctaacgtgttccagacaagggccggatgcctcatcggcgctgagcacgtgaacaattcttacgagtgcgacatccctattggagcgggcatctgcgccagctaccagacacagaccaatagccctcagcaagccgctagcgtggcctcccagagcatcatcgcctacaccatgagcctgggagccgagaactctgtggcctacagcaacaacagcatcgctatccctaccaacttcaccatctctgtcaccaccgaaatcctgcccgtcagtatgaccaaaaccagcgtcgactgcaccatgtacatatgcggcgatagcaccgaatgcagcaacctgctgctgcagtatggctccttctgcacccaacttaacagagccctgactggcatcgccgtggagcaggacaagaatacccaggaggtgttcgcccaggtgaagcagatctacaagacacccccgatcaaggacttcggcggctttaatttctctcagatcctgccagacccatctaaaccctctaagcggagctttatcgaggacctgctgttcaacaaggtgactctggctgacgccggcttcatcaagcagtacggcgattgcctgggcgacattgctgctagagacctgatctgtgcccagaaattcaacggtcttactgtgctgcctcctctgctgacggatgagatgatcgcccagtacaccagcgccctgctggccggcaccatcacatccggctggacattcggcgccggcgcagccctgcagatcccttttgccatgcagatggcctaccggttcaacggaatcggagtgacacagaacgtgctctacgaaaatcagaagttgatcgccaaccagttcaacagcgccatcggcaagattcaggatagtctgagttccaccgccagcgccctgggaaagctgcaggacgtggtcaatcagaatgcccaagccctgaacaccctggtgaagcagctgagcagcaacttcggcgccatcagctctgtgctgaacgacatcctgagtagactggacaaggtggaagccgaagtgcagatcgacagattgatcaccggaagactgcaaagcctgcagacctacgtgacccagcagctgataagagctgctgaaatcagagccagcgctaatctggccgctaccaagatgagcgagtgcgttctgggccagtctaagagagtggacttctgcggaaaaggctaccacctgatgtcctttcctcagtctgccccccacggcgtggtgttcctgcacgtcacatacgtgcccgctcaagagaaaaacttcaccacggcccctgccatctgtcacgacggcaaggcccacttccccagagagggcgtgttcgtgagcaatggcacccactggtttgtgactcagagaaacttctacgagccacagattatcaccacagataacaccttcgtgtctggcaactgcgacgtggtgatcggcatcgtcaacaacacagtgtacgacccactgcaacctgagctggactcattcaaggaggaactggataagtacttcaagaatcacaccagccccgacgttgacctgggcgacatcagcggcattaacgcctctgtggtcaacatccagaaggaaatcgacagactgaatgaggtggccaagaatttgaacgagagcctgattgatctgcaggagctgggcaaatacgagcagtacatcaagtggccttggtacatctggctgggcttcatcgccgggctgatcgccatcgttatggtgacaatcatgctgtgttgcatgacaagctgttgtagctgcctgaaaggctgctgctcctgcggcagctgttgcaagtttgacgaagatgacagcgagcccgtgctgaaaggcgtcaagctgcactacacctga

SEQ ID NO: 22 - DNA, 3813 bp, synthetic construct
  misc_feature 1..3813: note = Nucleotide sequence of SARS-CoV-2 spike (S) protein uncleavable (RRAR-QQAA; del69-70; delY144; N501Y; A570D; D614G; P680H; T716I)
  source 1..3813: mol_type = other DNA
atgttcgtgttcctggtgctgctgcccctcgttagcagccagtgcgtgaatctgaccacccgcacccagctgccaccagcctacacaaacagcttcaccagaggagtgtattaccctgataaggtctttagatcctccgtcctgcattctacgcaggatctcttcttgccattcttcagcaacgtgacatggttccacgccatctctggcaccaacggcacaaagcgcttcgacaatcctgtgttgccgtttaacgacggcgtttacttcgccagcacagaaaagagcaacatcatccggggctggatcttcggcaccaccctggacagcaaaacccaaagcctgctcatcgtgaacaacgccaccaacgtggtgatcaaggtgtgcgagttccagttctgcaatgatccttttctgggcgtgtatcacaagaacaacaagagctggatggaaagcgagttcagagtgtattctagcgccaacaactgcacctttgagtacgtgtcccagccctttcttatggacctggaaggcaagcagggcaacttcaagaatctgagagaattcgtgttcaagaacattgatggctacttcaagatctacagcaagcacacccctatcaacctggttcgggacctgccacaaggcttcagcgccctggaacctctggtggacctgcctatcggcatcaacatcacacggttccaaaccctgctggccctgcaccggagctacctgacccccggcgacagcagcagcggctggaccgccggcgctgccgcctattacgtgggctacctgcaacctagaaccttcctgctgaaatacaacgagaacggcacaatcaccgacgccgtggactgtgccctggaccccctgtctgagacaaagtgtaccctgaagtctttcaccgtggagaagggcatctaccagaccagcaacttccgggtgcagcctacagaatctatagtgcggttccctaacatcaccaacctgtgtccttttggcgaggtgttcaacgccactcggttcgcctctgtctacgcctggaaccggaaacggatctctaattgcgtggccgattacagcgtcctgtataactccgccagtttcagcacattcaagtgctacggcgtgtcacccaccaagctgaacgatctgtgcttcaccaatgtgtacgccgatagtttcgtgatccggggcgatgaggtgcggcagatcgcccctggacagacaggcaagatcgccgactacaactacaagctgcctgacgacttcacaggctgtgtgatcgcatggaacagcaacaacctggacagcaaggtgggcggaaactacaactacctgtacagactgttcagaaagtccaacctgaagcctttcgagagagatatatctaccgagatctaccaggccggcagcacaccctgtaatggagtggaaggctttaactgctacttccctctgcaaagctatggatttcaacctacatatggggttggctaccagccttacagagtggtggtccttagcttcgagctgctccatgcccctgccaccgtgtgcggacctaagaagtccaccaacctggtgaaaaacaagtgcgtgaactttaattttaacggcctgaccggaacaggagtgctgacagaaagcaacaaaaagttcctgcctttccagcagttcggcagagacattgacgacaccacagatgctgttagagacccccagacgctggaaatcctggatatcaccccctgctcttttggcggcgtgagcgtgatcaccccaggcacaaacacaagcaaccaggtggctgtgctgtaccagggcgtgaactgtacagaggtccctgtggcaatccacgccgatcagctgacccctacatggcgggtgtactccactggatctaacgtgttccagacaagggccggatgcctcatcggcgctgagcacgtgaacaattcttacgagtgcgacatccctattggagcgggcatctgcgccagctaccagacacagaccaatagccatcagcaagccgctagcgtggcctcccagagcatcatcgcctacaccatgagcctgggagccgagaactctgtggcctacagcaacaacagcatcgctatccctatcaacttcaccatctctgtcaccaccgaaatcctgcccgtcagtatgaccaaaaccagcgtcgactgcaccatgtacatatgcggcgatagcaccgaatgcagcaacctgctgctgcagtatggctccttctgcacccaacttaacagagccctgactggcatcgccgtggagcaggacaagaatacccaggaggtgttcgcccaggtgaagcagatctacaagacacccccgatcaaggacttcggcggctttaatttctctcagatcctgccagacccatctaaaccctctaagcggagctttatcgaggacctgctgttcaacaaggtgactctggctgacgccggcttcatcaagcagtacggcgattgcctgggcgacattgctgctagagacctgatctgtgcccagaaattcaacggtcttactgtgctgcctcctctgctgacggatgagatgatcgcccagtacaccagcgccctgctggccggcaccatcacatccggctggacattcggcgccggcgcagccctgcagatcccttttgccatgcagatggcctaccggttcaacggaatcggagtgacacagaacgtgctctacgaaaatcagaagttgatcgccaaccagttcaacagcgccatcggcaagattcaggatagtctgagttccaccgccagcgccctgggaaagctgcaggacgtggtcaatcagaatgcccaagccctgaacaccctggtgaagcagctgagcagcaacttcggcgccatcagctctgtgctgaacgacatcctggctagactggacaaggtggaagccgaagtgcagatcgacagattgatcaccggaagactgcaaagcctgcagacctacgtgacccagcagctgataagagctgctgaaatcagagccagcgctaatctggccgctaccaagatgagcgagtgcgttctgggccagtctaagagagtggacttctgcggaaaaggctaccacctgatgtcctttcctcagtctgccccccacggcgtggtgttcctgcacgtcacatacgtgcccgctcaagagaaaaacttcaccacggcccctgccatctgtcacgacggcaaggcccacttccccagagagggcgtgttcgtgagcaatggcacccactggtttgtgactcagagaaacttctacgagccacagattatcaccacacataacaccttcgtgtctggcaactgcgacgtggtgatcggcatcgtcaacaacacagtgtacgacccactgcaacctgagctggactcattcaaggaggaactggataagtacttcaagaatcacaccagccccgacgttgacctgggcgacatcagcggcattaacgcctctgtggtcaacatccagaaggaaatcgacagactgaatgaggtggccaagaatttgaacgagagcctgattgatctgcaggagctgggcaaatacgagcagtacatcaagtggccttggtacatctggctgggcttcatcgccgggctgatcgccatcgttatggtgacaatcatgctgtgttgcatgacaagctgttgtagctgcctgaaaggctgctgctcctgcggcagctgttgcaagtttgacgaagatgacagcgagcccgtgctgaaaggcgtcaagctgcactacacctga

SEQ ID NO: 23 - DNA, 3813 bp, synthetic construct
  misc_feature 1..3813: note = Nucleotide sequence of SARS-CoV-2 spike (S) protein uncleavable (RRAR-QQAA; L18F; D80A; D215G; ?242-244; K417N; E484K; N501Y; D614G; A701V)
  source 1..3813: mol_type = other DNA
atgttcgtgttcctggtgctgctgcccctcgttagcagccagtgcgtgaatttcaccacccgcacccagctgccaccagcctacacaaacagcttcaccagaggagtgtattaccctgataaggtctttagatcctccgtcctgcattctacgcaggatctcttcttgccattcttcagcaacgtgacatggttccacgccatccacgtttctggcaccaacggcacaaagcgcttcgccaatcctgtgttgccgtttaacgacggcgtttacttcgccagcacagaaaagagcaacatcatccggggctggatcttcggcaccaccctggacagcaaaacccaaagcctgctcatcgtgaacaacgccaccaacgtggtgatcaaggtgtgcgagttccagttctgcaatgatccttttctgggcgtgtactatcacaagaacaacaagagctggatggaaagcgagttcagagtgtattctagcgccaacaactgcacctttgagtacgtgtcccagccctttcttatggacctggaaggcaagcagggcaacttcaagaatctgagagaattcgtgttcaagaacattgatggctacttcaagatctacagcaagcacacccctatcaacctggttcggggcctgccacaaggcttcagcgccctggaacctctggtggacctgcctatcggcatcaacatcacacggttccaaaccctgcaccggagctacctgacccccggcgacagcagcagcggctggaccgccggcgctgccgcctattacgtgggctacctgcaacctagaaccttcctgctgaaatacaacgagaacggcacaatcaccgacgccgtggactgtgccctggaccccctgtctgagacaaagtgtaccctgaagtctttcaccgtggagaagggcatctaccagaccagcaacttccgggtgcagcctacagaatctatagtgcggttccctaacatcaccaacctgtgtccttttggcgaggtgttcaacgccactcggttcgcctctgtctacgcctggaaccggaaacggatctctaattgcgtggccgattacagcgtcctgtataactccgccagtttcagcacattcaagtgctacggcgtgtcacccaccaagctgaacgatctgtgcttcaccaatgtgtacgccgatagtttcgtgatccggggcgatgaggtgcggcagatcgcccctggacagacaggcaatatcgccgactacaactacaagctgcctgacgacttcacaggctgtgtgatcgcatggaacagcaacaacctggacagcaaggtgggcggaaactacaactacctgtacagactgttcagaaagtccaacctgaagcctttcgagagagatatatctaccgagatctaccaggccggcagcacaccctgtaatggagtgaaaggctttaactgctacttccctctgcaaagctatggatttcaacctacatatggggttggctaccagccttacagagtggtggtccttagcttcgagctgctccatgcccctgccaccgtgtgcggacctaagaagtccaccaacctggtgaaaaacaagtgcgtgaactttaattttaacggcctgaccggaacaggagtgctgacagaaagcaacaaaaagttcctgcctttccagcagttcggcagagacattgccgacaccacagatgctgttagagacccccagacgctggaaatcctggatatcaccccctgctcttttggcggcgtgagcgtgatcaccccaggcacaaacacaagcaaccaggtggctgtgctgtaccagggcgtgaactgtacagaggtccctgtggcaatccacgccgatcagctgacccctacatggcgggtgtactccactggatctaacgtgttccagacaagggccggatgcctcatcggcgctgagcacgtgaacaattcttacgagtgcgacatccctattggagcgggcatctgcgccagctaccagacacagaccaatagccctcagcaagccgctagcgtggcctcccagagcatcatcgcctacaccatgagcctgggagtcgagaactctgtggcctacagcaacaacagcatcgctatccctaccaacttcaccatctctgtcaccaccgaaatcctgcccgtcagtatgaccaaaaccagcgtcgactgcaccatgtacatatgcggcgatagcaccgaatgcagcaacctgctgctgcagtatggctccttctgcacccaacttaacagagccctgactggcatcgccgtggagcaggacaagaatacccaggaggtgttcgcccaggtgaagcagatctacaagacacccccgatcaaggacttcggcggctttaatttctctcagatcctgccagacccatctaaaccctctaagcggagctttatcgaggacctgctgttcaacaaggtgactctggctgacgccggcttcatcaagcagtacggcgattgcctgggcgacattgctgctagagacctgatctgtgcccagaaattcaacggtcttactgtgctgcctcctctgctgacggatgagatgatcgcccagtacaccagcgccctgctggccggcaccatcacatccggctggacattcggcgccggcgcagccctgcagatcccttttgccatgcagatggcctaccggttcaacggaatcggagtgacacagaacgtgctctacgaaaatcagaagttgatcgccaaccagttcaacagcgccatcggcaagattcaggatagtctgagttccaccgccagcgccctgggaaagctgcaggacgtggtcaatcagaatgcccaagccctgaacaccctggtgaagcagctgagcagcaacttcggcgccatcagctctgtgctgaacgacatcctgagtagactggacaaggtggaagccgaagtgcagatcgacagattgatcaccggaagactgcaaagcctgcagacctacgtgacccagcagctgataagagctgctgaaatcagagccagcgctaatctggccgctaccaagatgagcgagtgcgttctgggccagtctaagagagtggacttctgcggaaaaggctaccacctgatgtcctttcctcagtctgccccccacggcgtggtgttcctgcacgtcacatacgtgcccgctcaagagaaaaacttcaccacggcccctgccatctgtcacgacggcaaggcccacttccccagagagggcgtgttcgtgagcaatggcacccactggtttgtgactcagagaaacttctacgagccacagattatcaccacagataacaccttcgtgtctggcaactgcgacgtggtgatcggcatcgtcaacaacacagtgtacgacccactgcaacctgagctggactcattcaaggaggaactggataagtacttcaagaatcacaccagccccgacgttgacctgggcgacatcagcggcattaacgcctctgtggtcaacatccagaaggaaatcgacagactgaatgaggtggccaagaatttgaacgagagcctgattgatctgcaggagctgggcaaatacgagcagtacatcaagtggccttggtacatctggctgggcttcatcgccgggctgatcgccatcgttatggtgacaatcatgctgtgttgcatgacaagctgttgtagctgcctgaaaggctgctgctcctgcggcagctgttgcaagtttgacgaagatgacagcgagcccgtgctgaaaggcgtcaagctgcactacacctga

SEQ ID NO: 24 - DNA, 14005 bp, synthetic construct
  misc_feature 1..14005: note = Nucleotide sequence of construct Co77
  source 1..14005: mol_type = other DNA
ataggcggcgcatgagagaagcccagaccaattacctacccaaaatggagaaagttcacgttgacatcgaggaagacagcccattcctcagagctttgcagcggagcttcccgcagtttgaggtagaagccaagcaggtcactgataatgaccatgctaatgccagagcgttttcgcatctggcttcaaaactgatcgaaacggaggtggacccatccgacacgatccttgacattggaagtgcgcccgcccgcagaatgtattctaagcacaagtatcattgtatctgtccgatgagatgtgcggaagatccggacagattgtataagtatgcaactaagctgaagaaaaactgtaaggaaataactgataaggaattggacaagaaaatgaaggagctcgccgccgtcatgagcgaccctgacctggaaactgagactatgtgcctccacgacgacgagtcgtgtcgctacgaagggcaagtcgctgtttaccaggatgtatacgcggttgacggaccgacaagtctctatcaccaagccaataagggagttagagtcgcctactggataggctttgacaccaccccttttatgtttaagaacttggctggagcatatccatcatactctaccaactgggccgacgaaaccgtgttaacggctcgtaacataggcctatgcagctctgacgttatggagcggtcacgtagagggatgtccattcttagaaagaagtatttgaaaccatccaacaatgttctattctctgttggctcgaccatctaccacgagaagagggacttactgaggagctggcacctgccgtctgtatttcacttacgtggcaagcaaaattacacatgtcggtgtgagactatagttagttgcgacgggtacgtcgttaaaagaatagctatcagtccaggcctgtatgggaagccttcaggctatgctgctacgatgcaccgcgagggattcttgtgctgcaaagtgacagacacattgaacggggagagggtctcttttcccgtgtgcacgtatgtgccagctacattgtgtgaccaaatgactggcatactggcaacagatgtcagtgcggacgacgcgcaaaaactgctggttgggctcaaccagcgtatagtcgtcaacggtcgcacccagagaaacaccaataccatgaaaaattaccttttgcccgtagtggcccaggcatttgctaggtgggcaaaggaatataaggaagatcaagaagatgaaaggccactaggactacgagatagacagttagtcatggggtgttgttgggcttttagaaggcacaagataacatctatttataagcgcccggatacccaaaccatcatcaaagtgaacagcgatttccactcattcgtgctgcccaggataggcagtaacacattggagatcgggctgagaacaagaatcaggaaaatgttagaggagcacaaggagccgtcacctctcattaccgccgaggacgtacaagaagctaagtgcgcagccgatgaggctaaggaggtgcgtgaagccgaggagttgcgcgcagctctaccacctttggcagctgatgttgaggagcccactctggaagccgatgtcgacttgatgttacaagaggctggggccggctcagtggagacacctcgtggcttgataaaggttaccagctacgatggcgaggacaagatcggctcttacgctgtgctttctccgcaggctgtactcaagagtgaaaaattatcttgcatccaccctctcgctgaacaagtcatagtgataacacactctggccgaaaagggcgttatgccgtggaaccataccatggtaaagtagtggtgccagagggacatgcaatacccgtccaggactttcaagctctgagtgaaagtgccaccattgtgtacaacgaacgtgagttcgtaaacaggtacctgcaccatattgccacacatggaggagcgctgaacactgatgaagaatattacaaaactgtcaagcccagcgagcacgacggcgaatacctgtacgacatcgacaggaaacagtgcgtcaagaaagaactagtcactgggctagggctcacaggcgagctggtggatcctcccttccatgaattcgcctacgagagtctgagaacacgaccagccgctccttaccaagtaccaaccataggggtgtatggcgtgccaggatcaggcaagtctggcatcattaaaagcgcagtcaccaaaaaagatctagtggtgagcgccaagaaagaaaactgtgcagaaattataagggacgtcaagaaaatgaaagggctggacgtcaatgccagaactgtggactcagtgctcttgaatggatgcaaacaccccgtagagaccctgtatattgacgaagcttttgcttgtcatgcaggtactctcagagcgctcatagccattataagacctaaaaaggcagtgctctgcggggatcccaaacagtgcggtttttttaacatgatgtgcctgaaagtgcattttaaccacgagatttgcacacaagtcttccacaaaagcatctctcgccgttgcactaaatctgtgacttcggtcgtctcaaccttgttttacgacaaaaaaatgagaacgacgaatccgaaagagactaagattgtgattgacactaccggcagtaccaaacctaagcaggacgatctcattctcacttgtttcagagggtgggtgaagcagttgcaaatagattacaaaggcaacgaaataatgacggcagctgcctctcaagggctgacccgtaaaggtgtgtatgccgttcggtacaaggtgaatgaaaatcctctgtacgcacccacctcagaacatgtgaacgtcctactgacccgcacggaggaccgcatcgtgtggaaaacactagccggcgacccatggataaaaacactgactgccaagtaccctgggaatttcactgccacgatagaggagtggcaagcagagcatgatgccatcatgaggcacatcttggagagaccggaccctaccgacgtcttccagaataaggcaaacgtgtgttgggccaaggctttagtgccggtgctgaagaccgctggcatagacatgaccactgaacaatggaacactgtggattattttgaaacggacaaagctcactcagcagagatagtattgaaccaactatgcgtgaggttctttggactcgatctggactccggtctattttctgcacccactgttccgttatccattaggaataatcactgggataactccccgtcgcctaacatgtacgggctgaataaagaagtggtccgtcagctctctcgcaggtacccacaactgcctcgggcagttgccactggaagagtctatgacatgaacactggtacactgcgcaattatgatccgcgcataaacctagtacctgtaaacagaagactgcctcatgctttagtcctccaccataatgaacacccacagagtgacttttcttcattcgtcagcaaattgaagggcagaactgtcctggtggtcggggaaaagttgtccgtcccaggcaaaatggttgactggttgtcagaccggcctgaggctaccttcagagctcggctggatttaggcatcccaggtgatgtgcccaaatatgacataatatttgttaatgtgaggaccccatataaataccatcactatcagcagtgtgaagaccatgccattaagcttagcatgttgaccaagaaagcttgtctgcatctgaatcccggcggaacctgtgtcagcataggttatggttacgctgacagggccagcgaaagcatcattggtgctatagcgcggcagttcaagttttcccgggtatgcaaaccgaaatcctcacttgaagagacggaagttctgtttgtattcattgggtacgatcgcaaggcccgtacgcacaatccttacaagctttcatcaaccttgaccaacatttatacaggttccagactccacgaagccggatgtgcaccctcatatcatgtggtgcgaggggatattgccacggccaccgaaggagtgattataaatgctgctaacagcaaaggacaacctggcggaggggtgtgcggagcgctgtataagaaattcccggaaagcttcgatttacagccgatcgaagtaggaaaagcgcgactggtcaaaggtgcagctaaacatatcattcatgccgtaggaccaaacttcaacaaagtttcggaggttgaaggtgacaaacagttggcagaggcttatgagtccatcgctaagattgtcaacgataacaattacaagtcagtagcgattccactgttgtccaccggcatcttttccgggaacaaagatcgactaacccaatcattgaaccatttgctgacagctttagacaccactgatgcagatgtagccatatactgcagggacaagaaatgggaaatgactctcaaggaagcagtggctaggagagaagcagtggaggagatatgcatatccgacgactcttcagtgacagaacctgatgcagagctggtgagggtgcatccgaagagttctttggctggaaggaagggctacagcacaagcgatggcaaaactttctcatatttggaagggaccaagtttcaccaggcggccaaggatatagcagaaattaatgccatgtggcccgttgcaacggaggccaatgagcaggtatgcatgtatatcctcggagaaagcatgagcagtattaggtcgaaatgccccgtcgaagagtcggaagcctccacaccacctagcacgctgccttgcttgtgcatccatgccatgactccagaaagagtacagcgcctaaaagcctcacgtccagaacaaattactgtgtgctcatcctttccattgccgaagtatagaatcactggtgtgcagaagatccaatgctcccagcctatattgttctcaccgaaagtgcctgcgtatattcatccaaggaagtatctcgtggaaacaccaccggtagacgagactccggagccatcggcagagaaccaatccacagaggggacacctgaacaaccaccacttataaccgaggatgagaccaggactagaacgcctgagccgatcatcatcgaagaggaagaagaggatagcataagtttgctgtcagatggcccgacccaccaggtgctgcaagtcgaggcagacattcacgggccgccctctgtatctagctcatcctggtccattcctcatgcatccgactttgatgtggacagtttatccatacttgacaccctggagggagctagcgtgaccagcggggcaacgtcagccgagactaactcttacttcgcaaagagtatggagtttctggcgcgaccggtgcctgcgcctcgaacagtattcaggaaccctccacatcccgctccgcgcacaagaacaccgtcacttgcacccagcagggcctgctcgagaaccagcctagtttccaccccgccaggcgtgaatagggtgatcactagagaggagctcgaggcgcttaccccgtcacgcactcctagcaggtcggtctcgagaaccagcctggtctccaacccgccaggcgtaaatagggtgattacaagagaggagtttgaggcgttcgtagcacaacaacaatgacggtttgatgcgggtgcatacatcttttcctccgacaccggtcaagggcatttacaacaaaaatcagtaaggcaaacggtgctatccgaagtggtgttggagaggaccgaattggagatttcgtatgccccgcgcctcgaccaagaaaaagaagaattactacgcaagaaattacagttaaatcccacacctgctaacagaagcagataccagtccaggaaggtggagaacatgaaagccataacagctagacgtattctgcaaggcctagggcattatttgaaggcagaaggaaaagtggagtgctaccgaaccctgcatcctgttcctttgtattcatctagtgtgaaccgtgccttttcaagccccaaggtcgcagtggaagcctgtaacgccatgttgaaagagaactttccgactgtggcttcttactgtattattccagagtacgatgcctatttggacatggttgacggagcttcatgctgcttagacactgccagtttttgccctgcaaagctgcgcagctttccaaagaaacactcctatttggaacccacaatacgatcggcagtgccttcagcgatccagaacacgctccagaacgtcctggcagctgccacaaaaagaaattgcaatgtcacgcaaatgagagaattgcccgtattggattcggcggcctttaatgtggaatgcttcaagaaatatgcgtgtaataatgaatattgggaaacgtttaaagaaaaccccatcaggcttactgaagaaaacgtggtaaattacattaccaaattaaaaggaccaaaagctgctgctctttttgcgaagacacataatttgaatatgttgcaggacataccaatggacaggtttgtaatggacttaaagagagacgtgaaagtgactccaggaacaaaacatactgaagaacggcccaaggtacaggtgatccaggctgccgatccgctagcaacagcgtatctgtgcggaatccaccgagagctggttaggagattaaatgcggtcctgcttccgaacattcatacactgtttgatatgtcggctgaagactttgacgctattatagccgagcacttccagcctggggattgtgttctggaaactgacatcgcgtcgtttgataaaagtgaggacgacgccatggctctgaccgcgttaatgattctggaagacttaggtgtggacgcagagctgttgacgctgattgaggcggctttcggcgaaatttcatcaatacatttgcccactaaaactaaatttaaattcggagccatgatgaaatctggaatgttcctcacactgtttgtgaacacagtcattaacattgtaatcgcaagcagagtgttgagagaacggctaaccggatcaccatgtgcagcattcattggagatgacaatatcgtgaaaggagtcaaatcggacaaattaatggcagacaggtgcgccacctggttgaatatggaagtcaagattatagatgctgtggtgggcgagaaagcgccttatttctgtggagggtttattttgtgtgactccgtgaccggcacagcgtgccgtgtggcagaccccctaaaaaggctgtttaagcttggcaaacctctggcagcagacgatgaacatgatgatgacaggagaagggcattgcatgaagagtcaacacgctggaaccgagtgggtattctttcagagctgtgcaaggcagtagaatcaaggtatgaaaccgtaggaacttccatcatagttatggccatgactactctagctagcagtgttaaatcattcagctacctgagaggggcccctataactctctacggctaacctgaatggactacgacatagtctagtccgccaagatgttcgtgttcctggtgctgctgcccctcgttagcagccagtgcgtgaatctgaccacccgcacccagctgccaccagcctacacaaacagcttcaccagaggagtgtattaccctgataaggtctttagatcctccgtcctgcattctacgcaggatctcttcttgccattcttcagcaacgtgacatggttccacgccatctctggcaccaacggcacaaagcgcttcgacaatcctgtgttgccgtttaacgacggcgtttacttcgccagcacagaaaagagcaacatcatccggggctggatcttcggcaccaccctggacagcaaaacccaaagcctgctcatcgtgaacaacgccaccaacgtggtgatcaaggtgtgcgagttccagttctgcaatgatccttttctgggcgtgtatcacaagaacaacaagagctggatggaaagcgagttcagagtgtattctagcgccaacaactgcacctttgagtacgtgtcccagccctttcttatggacctggaaggcaagcagggcaacttcaagaatctgagagaattcgtgttcaagaacattgatggctacttcaagatctacagcaagcacacccctatcaacctggttcgggacctgccacaaggcttcagcgccctggaacctctggtggacctgcctatcggcatcaacatcacacggttccaaaccctgctggccctgcaccggagctacctgacccccggcgacagcagcagcggctggaccgccggcgctgccgcctattacgtgggctacctgcaacctagaaccttcctgctgaaatacaacgagaacggcacaatcaccgacgccgtggactgtgccctggaccccctgtctgagacaaagtgtaccctgaagtctttcaccgtggagaagggcatctaccagaccagcaacttccgggtgcagcctacagaatctatagtgcggttccctaacatcaccaacctgtgtccttttggcgaggtgttcaacgccactcggttcgcctctgtctacgcctggaaccggaaacggatctctaattgcgtggccgattacagcgtcctgtataactccgccagtttcagcacattcaagtgctacggcgtgtcacccaccaagctgaacgatctgtgcttcaccaatgtgtacgccgatagtttcgtgatccggggcgatgaggtgcggcagatcgcccctggacagacaggcaagatcgccgactacaactacaagctgcctgacgacttcacaggctgtgtgatcgcatggaacagcaacaacctggacagcaaggtgggcggaaactacaactacctgtacagactgttcagaaagtccaacctgaagcctttcgagagagatatatctaccgagatctaccaggccggcagcacaccctgtaatggagtggaaggctttaactgctacttccctctgcaaagctatggatttcaacctacatatggggttggctaccagccttacagagtggtggtccttagcttcgagctgctccatgcccctgccaccgtgtgcggacctaagaagtccaccaacctggtgaaaaacaagtgcgtgaactttaattttaacggcctgaccggaacaggagtgctgacagaaagcaacaaaaagttcctgcctttccagcagttcggcagagacattgccgacaccacagatgctgttagagacccccagacgctggaaatcctggatatcaccccctgctcttttggcggcgtgagcgtgatcaccccaggcacaaacacaagcaaccaggtggctgtgctgtaccagggcgtgaactgtacagaggtccctgtggcaatccacgccgatcagctgacccctacatggcgggtgtactccactggatctaacgtgttccagacaagggccggatgcctcatcggcgctgagcacgtgaacaattcttacgagtgcgacatccctattggagcgggcatctgcgccagctaccagacacagaccaatagccctcagcaagccgctagcgtggcctcccagagcatcatcgcctacaccatgagcctgggagccgagaactctgtggcctacagcaacaacagcatcgctatccctaccaacttcaccatctctgtcaccaccgaaatcctgcccgtcagtatgaccaaaaccagcgtcgactgcaccatgtacatatgcggcgatagcaccgaatgcagcaacctgctgctgcagtatggctccttctgcacccaacttaacagagccctgactggcatcgccgtggagcaggacaagaatacccaggaggtgttcgcccaggtgaagcagatctacaagacacccccgatcaaggacttcggcggctttaatttctctcagatcctgccagacccatctaaaccctctaagcggagctttatcgaggacctgctgttcaacaaggtgactctggctgacgccggcttcatcaagcagtacggcgattgcctgggcgacattgctgctagagacctgatctgtgcccagaaattcaacggtcttactgtgctgcctcctctgctgacggatgagatgatcgcccagtacaccagcgccctgctggccggcaccatcacatccggctggacattcggcgccggcgcagccctgcagatcccttttgccatgcagatggcctaccggttcaacggaatcggagtgacacagaacgtgctctacgaaaatcagaagttgatcgccaaccagttcaacagcgccatcggcaagattcaggatagtctgagttccaccgccagcgccctgggaaagctgcaggacgtggtcaatcagaatgcccaagccctgaacaccctggtgaagcagctgagcagcaacttcggcgccatcagctctgtgctgaacgacatcctgagtagactggacaaggtggaagccgaagtgcagatcgacagattgatcaccggaagactgcaaagcctgcagacctacgtgacccagcagctgataagagctgctgaaatcagagccagcgctaatctggccgctaccaagatgagcgagtgcgttctgggccagtctaagagagtggacttctgcggaaaaggctaccacctgatgtcctttcctcagtctgccccccacggcgtggtgttcctgcacgtcacatacgtgcccgctcaagagaaaaacttcaccacggcccctgccatctgtcacgacggcaaggcccacttccccagagagggcgtgttcgtgagcaatggcacccactggtttgtgactcagagaaacttctacgagccacagattatcaccacagataacaccttcgtgtctggcaactgcgacgtggtgatcggcatcgtcaacaacacagtgtacgacccactgcaacctgagctggactcattcaaggaggaactggataagtacttcaagaatcacaccagccccgacgttgacctgggcgacatcagcggcattaacgcctctgtggtcaacatccagaaggaaatcgacagactgaatgaggtggccaagaatttgaacgagagcctgattgatctgcaggagctgggcaaatacgagcagtacatcaagtggccttggtacatctggctgggcttcatcgccgggctgatcgccatcgttatggtgacaatcatgctgtgttgcatgacaagctgttgtagctgcctgaaaggctgctgctcctgcggcagctgttgcaagtttgacgaagatgacagcgagcccgtgctgaaaggcgtcaagctgcactacacctgaggcgcgcccacccagcggccgcccgctacgccccaatgatccgaccagcaaaactcgatgtacttccgaggaactgatgtgcataatgcatcaggctggtacattagatccccgcttaccgcgggcaatatagcaacactaaaaactcgatgtacttccgaggaagcgcagtgcataatgctgcgcagtgttgccacataaccactatattaaccatttatctagcggacgccaaaaactcaatgtatttctgaggaagcgtggtgcataatgccacgcagcgtctgcataacttttattatttcttttattaatcaacaaaattttgtttttaacatttcaaaaaaaaaaaaaaaaaaaaaaaaaaaaaaaaaaaaagaagagcgtttaaacacgtgatatctggcctcatgggccttcctttcactgcccgctttccagtcgggaaacctgtcgtgccagctgcattaacatggtcatagctgtttccttgcgtattgggcgctctccgcttcctcgctcactgactcgctgcgctcggtcgttcgggtaaagcctggggtgcctaatgagcaaaaggccagcaaaaggccaggaaccgtaaaaaggccgcgttgctggcgtttttccataggctccgcccccctgacgagcatcacaaaaatcgacgctcaagtcagaggtggcgaaacccgacaggactataaagataccaggcgtttccccctggaagctccctcgtgcgctctcctgttccgaccctgccgcttaccggatacctgtccgcctttctcccttcgggaagcgtggcgctttctcatagctcacgctgtaggtatctcagttcggtgtaggtcgttcgctccaagctgggctgtgtgcacgaaccccccgttcagcccgaccgctgcgccttatccggtaactatcgtcttgagtccaacccggtaagacacgacttatcgccactggcagcagccactggtaacaggattagcagagcgaggtatgtaggcggtgctacagagttcttgaagtggtggcctaactacggctacactagaagaacagtatttggtatctgcgctctgctgaagccagttaccttcggaaaaagagttggtagctcttgatccggcaaacaaaccaccgctggtagcggtggtttttttgtttgcaggcagcagattacgcgcagaaaaaaaggatctcaagaagatcctttgatcttttctacggggtctgacgctcagtggaacgaaaactcacgttaagggattttggtcatgaatacacggtgcctgactgcgttagcaatttaactgtgataaactaccgcattaaagcttatcgatgataagctgtcaaacatgagaattcttagaaaaactcatcgagcatcaaatgaaactgcaatttattcatatcaggattatcaataccatatttttgaaaaagccgtttctgtaatgaaggagaaaactcaccgaggcagttccataggatggcaagatcctggtatcggtctgcgattccgactcgtccaacatcaatacaacctattaatttcccctcgtcaaaaataaggttatcaagtgagaaatcaccatgagtgacgactgaatccggtgagaatggcaaaagcttatgcatttctttccagacttgttcaacaggccagccattacgctcgtcatcaaaatcactcgcatcaaccaaaccgttattcattcgtgattgcgcctgagcgagacgaaatacgcgatcgctgttaaaaggacaattacaaacaggaatcgaatgcaaccggcgcaggaacactgccagcgcatcaacaatattttcacctgaatcaggatattcttctaatacctggaatgctgttttcccggggatcgcagtggtgagtaaccatgcatcatcaggagtacggataaaatgcttgatggtcggaagaggcataaattccgtcagccagtttagtctgaccatctcatctgtaacatcattggcaacgctacctttgccatgtttcagaaacaactctggcgcatcgggcttcccatacaatcgatagattgtcgcacctgattgcccgacattatcgcgagcccatttatacccatataaatcagcatccatgttggaatttaatcgcggcctcgagcaagacgtttcccgttgaatatggctcataacaccccttgtattactgtttatgtaagcagacagttttattgttcatgagcggatacatatttgaatgtatttagaaaaataaacaaataggggttccgcgcacatttccccgaaaagtgccacctaaattgtaagcgttaatattttgttaaaattcgcgttaaatttttgttaaatcagctcattttttaaccaataggccgaaatcggcaaaatcccttataaatcaaaagaatagaccgagatagggttgagtggccgctacagggcgctcccattcgccattcaggctgcgcaactgttgggaagggcgtttcggtgcgggcctcttcgctattacgccagctggcgaaagggggatgtgctgcaaggcgattaagttgggtaacgccagggttttcccagtcacacgcgtaatacgactcactatag

SEQ ID NO: 25 - DNA, 14005 bp, synthetic construct
  misc_feature 1..14005: note = Nucleotide sequence of construct Co78
  source 1..14005: mol_type = other DNA
ataggcggcgcatgagagaagcccagaccaattacctacccaaaatggagaaagttcacgttgacatcgaggaagacagcccattcctcagagctttgcagcggagcttcccgcagtttgaggtagaagccaagcaggtcactgataatgaccatgctaatgccagagcgttttcgcatctggcttcaaaactgatcgaaacggaggtggacccatccgacacgatccttgacattggaagtgcgcccgcccgcagaatgtattctaagcacaagtatcattgtatctgtccgatgagatgtgcggaagatccggacagattgtataagtatgcaactaagctgaagaaaaactgtaaggaaataactgataaggaattggacaagaaaatgaaggagctcgccgccgtcatgagcgaccctgacctggaaactgagactatgtgcctccacgacgacgagtcgtgtcgctacgaagggcaagtcgctgtttaccaggatgtatacgcggttgacggaccgacaagtctctatcaccaagccaataagggagttagagtcgcctactggataggctttgacaccaccccttttatgtttaagaacttggctggagcatatccatcatactctaccaactgggccgacgaaaccgtgttaacggctcgtaacataggcctatgcagctctgacgttatggagcggtcacgtagagggatgtccattcttagaaagaagtatttgaaaccatccaacaatgttctattctctgttggctcgaccatctaccacgagaagagggacttactgaggagctggcacctgccgtctgtatttcacttacgtggcaagcaaaattacacatgtcggtgtgagactatagttagttgcgacgggtacgtcgttaaaagaatagctatcagtccaggcctgtatgggaagccttcaggctatgctgctacgatgcaccgcgagggattcttgtgctgcaaagtgacagacacattgaacggggagagggtctcttttcccgtgtgcacgtatgtgccagctacattgtgtgaccaaatgactggcatactggcaacagatgtcagtgcggacgacgcgcaaaaactgctggttgggctcaaccagcgtatagtcgtcaacggtcgcacccagagaaacaccaataccatgaaaaattaccttttgcccgtagtggcccaggcatttgctaggtgggcaaaggaatataaggaagatcaagaagatgaaaggccactaggactacgagatagacagttagtcatggggtgttgttgggcttttagaaggcacaagataacatctatttataagcgcccggatacccaaaccatcatcaaagtgaacagcgatttccactcattcgtgctgcccaggataggcagtaacacattggagatcgggctgagaacaagaatcaggaaaatgttagaggagcacaaggagccgtcacctctcattaccgccgaggacgtacaagaagctaagtgcgcagccgatgaggctaaggaggtgcgtgaagccgaggagttgcgcgcagctctaccacctttggcagctgatgttgaggagcccactctggaagccgatgtcgacttgatgttacaagaggctggggccggctcagtggagacacctcgtggcttgataaaggttaccagctacgatggcgaggacaagatcggctcttacgctgtgctttctccgcaggctgtactcaagagtgaaaaattatcttgcatccaccctctcgctgaacaagtcatagtgataacacactctggccgaaaagggcgttatgccgtggaaccataccatggtaaagtagtggtgccagagggacatgcaatacccgtccaggactttcaagctctgagtgaaagtgccaccattgtgtacaacgaacgtgagttcgtaaacaggtacctgcaccatattgccacacatggaggagcgctgaacactgatgaagaatattacaaaactgtcaagcccagcgagcacgacggcgaatacctgtacgacatcgacaggaaacagtgcgtcaagaaagaactagtcactgggctagggctcacaggcgagctggtggatcctcccttccatgaattcgcctacgagagtctgagaacacgaccagccgctccttaccaagtaccaaccataggggtgtatggcgtgccaggatcaggcaagtctggcatcattaaaagcgcagtcaccaaaaaagatctagtggtgagcgccaagaaagaaaactgtgcagaaattataagggacgtcaagaaaatgaaagggctggacgtcaatgccagaactgtggactcagtgctcttgaatggatgcaaacaccccgtagagaccctgtatattgacgaagcttttgcttgtcatgcaggtactctcagagcgctcatagccattataagacctaaaaaggcagtgctctgcggggatcccaaacagtgcggtttttttaacatgatgtgcctgaaagtgcattttaaccacgagatttgcacacaagtcttccacaaaagcatctctcgccgttgcactaaatctgtgacttcggtcgtctcaaccttgttttacgacaaaaaaatgagaacgacgaatccgaaagagactaagattgtgattgacactaccggcagtaccaaacctaagcaggacgatctcattctcacttgtttcagagggtgggtgaagcagttgcaaatagattacaaaggcaacgaaataatgacggcagctgcctctcaagggctgacccgtaaaggtgtgtatgccgttcggtacaaggtgaatgaaaatcctctgtacgcacccacctcagaacatgtgaacgtcctactgacccgcacggaggaccgcatcgtgtggaaaacactagccggcgacccatggataaaaacactgactgccaagtaccctgggaatttcactgccacgatagaggagtggcaagcagagcatgatgccatcatgaggcacatcttggagagaccggaccctaccgacgtcttccagaataaggcaaacgtgtgttgggccaaggctttagtgccggtgctgaagaccgctggcatagacatgaccactgaacaatggaacactgtggattattttgaaacggacaaagctcactcagcagagatagtattgaaccaactatgcgtgaggttctttggactcgatctggactccggtctattttctgcacccactgttccgttatccattaggaataatcactgggataactccccgtcgcctaacatgtacgggctgaataaagaagtggtccgtcagctctctcgcaggtacccacaactgcctcgggcagttgccactggaagagtctatgacatgaacactggtacactgcgcaattatgatccgcgcataaacctagtacctgtaaacagaagactgcctcatgctttagtcctccaccataatgaacacccacagagtgacttttcttcattcgtcagcaaattgaagggcagaactgtcctggtggtcggggaaaagttgtccgtcccaggcaaaatggttgactggttgtcagaccggcctgaggctaccttcagagctcggctggatttaggcatcccaggtgatgtgcccaaatatgacataatatttgttaatgtgaggaccccatataaataccatcactatcagcagtgtgaagaccatgccattaagcttagcatgttgaccaagaaagcttgtctgcatctgaatcccggcggaacctgtgtcagcataggttatggttacgctgacagggccagcgaaagcatcattggtgctatagcgcggcagttcaagttttcccgggtatgcaaaccgaaatcctcacttgaagagacggaagttctgtttgtattcattgggtacgatcgcaaggcccgtacgcacaatccttacaagctttcatcaaccttgaccaacatttatacaggttccagactccacgaagccggatgtgcaccctcatatcatgtggtgcgaggggatattgccacggccaccgaaggagtgattataaatgctgctaacagcaaaggacaacctggcggaggggtgtgcggagcgctgtataagaaattcccggaaagcttcgatttacagccgatcgaagtaggaaaagcgcgactggtcaaaggtgcagctaaacatatcattcatgccgtaggaccaaacttcaacaaagtttcggaggttgaaggtgacaaacagttggcagaggcttatgagtccatcgctaagattgtcaacgataacaattacaagtcagtagcgattccactgttgtccaccggcatcttttccgggaacaaagatcgactaacccaatcattgaaccatttgctgacagctttagacaccactgatgcagatgtagccatatactgcagggacaagaaatgggaaatgactctcaaggaagcagtggctaggagagaagcagtggaggagatatgcatatccgacgactcttcagtgacagaacctgatgcagagctggtgagggtgcatccgaagagttctttggctggaaggaagggctacagcacaagcgatggcaaaactttctcatatttggaagggaccaagtttcaccaggcggccaaggatatagcagaaattaatgccatgtggcccgttgcaacggaggccaatgagcaggtatgcatgtatatcctcggagaaagcatgagcagtattaggtcgaaatgccccgtcgaagagtcggaagcctccacaccacctagcacgctgccttgcttgtgcatccatgccatgactccagaaagagtacagcgcctaaaagcctcacgtccagaacaaattactgtgtgctcatcctttccattgccgaagtatagaatcactggtgtgcagaagatccaatgctcccagcctatattgttctcaccgaaagtgcctgcgtatattcatccaaggaagtatctcgtggaaacaccaccggtagacgagactccggagccatcggcagagaaccaatccacagaggggacacctgaacaaccaccacttataaccgaggatgagaccaggactagaacgcctgagccgatcatcatcgaagaggaagaagaggatagcataagtttgctgtcagatggcccgacccaccaggtgctgcaagtcgaggcagacattcacgggccgccctctgtatctagctcatcctggtccattcctcatgcatccgactttgatgtggacagtttatccatacttgacaccctggagggagctagcgtgaccagcggggcaacgtcagccgagactaactcttacttcgcaaagagtatggagtttctggcgcgaccggtgcctgcgcctcgaacagtattcaggaaccctccacatcccgctccgcgcacaagaacaccgtcacttgcacccagcagggcctgctcgagaaccagcctagtttccaccccgccaggcgtgaatagggtgatcactagagaggagctcgaggcgcttaccccgtcacgcactcctagcaggtcggtctcgagaaccagcctggtctccaacccgccaggcgtaaatagggtgattacaagagaggagtttgaggcgttcgtagcacaacaacaatgacggtttgatgcgggtgcatacatcttttcctccgacaccggtcaagggcatttacaacaaaaatcagtaaggcaaacggtgctatccgaagtggtgttggagaggaccgaattggagatttcgtatgccccgcgcctcgaccaagaaaaagaagaattactacgcaagaaattacagttaaatcccacacctgctaacagaagcagataccagtccaggaaggtggagaacatgaaagccataacagctagacgtattctgcaaggcctagggcattatttgaaggcagaaggaaaagtggagtgctaccgaaccctgcatcctgttcctttgtattcatctagtgtgaaccgtgccttttcaagccccaaggtcgcagtggaagcctgtaacgccatgttgaaagagaactttccgactgtggcttcttactgtattattccagagtacgatgcctatttggacatggttgacggagcttcatgctgcttagacactgccagtttttgccctgcaaagctgcgcagctttccaaagaaacactcctatttggaacccacaatacgatcggcagtgccttcagcgatccagaacacgctccagaacgtcctggcagctgccacaaaaagaaattgcaatgtcacgcaaatgagagaattgcccgtattggattcggcggcctttaatgtggaatgcttcaagaaatatgcgtgtaataatgaatattgggaaacgtttaaagaaaaccccatcaggcttactgaagaaaacgtggtaaattacattaccaaattaaaaggaccaaaagctgctgctctttttgcgaagacacataatttgaatatgttgcaggacataccaatggacaggtttgtaatggacttaaagagagacgtgaaagtgactccaggaacaaaacatactgaagaacggcccaaggtacaggtgatccaggctgccgatccgctagcaacagcgtatctgtgcggaatccaccgagagctggttaggagattaaatgcggtcctgcttccgaacattcatacactgtttgatatgtcggctgaagactttgacgctattatagccgagcacttccagcctggggattgtgttctggaaactgacatcgcgtcgtttgataaaagtgaggacgacgccatggctctgaccgcgttaatgattctggaagacttaggtgtggacgcagagctgttgacgctgattgaggcggctttcggcgaaatttcatcaatacatttgcccactaaaactaaatttaaattcggagccatgatgaaatctggaatgttcctcacactgtttgtgaacacagtcattaacattgtaatcgcaagcagagtgttgagagaacggctaaccggatcaccatgtgcagcattcattggagatgacaatatcgtgaaaggagtcaaatcggacaaattaatggcagacaggtgcgccacctggttgaatatggaagtcaagattatagatgctgtggtgggcgagaaagcgccttatttctgtggagggtttattttgtgtgactccgtgaccggcacagcgtgccgtgtggcagaccccctaaaaaggctgtttaagcttggcaaacctctggcagcagacgatgaacatgatgatgacaggagaagggcattgcatgaagagtcaacacgctggaaccgagtgggtattctttcagagctgtgcaaggcagtagaatcaaggtatgaaaccgtaggaacttccatcatagttatggccatgactactctagctagcagtgttaaatcattcagctacctgagaggggcccctataactctctacggctaacctgaatggactacgacatagtctagtccgccaagatgttcgtgttcctggtgctgctgcccctcgttagcagccagtgcgtgaatctgaccacccgcacccagctgccaccagcctacacaaacagcttcaccagaggagtgtattaccctgataaggtctttagatcctccgtcctgcattctacgcaggatctcttcttgccattcttcagcaacgtgacatggttccacgccatccacgtttctggcaccaacggcacaaagcgcttcgacaatcctgtgttgccgtttaacgacggcgtttacttcgccagcacagaaaagagcaacatcatccggggctggatcttcggcaccaccctggacagcaaaacccaaagcctgctcatcgtgaacaacgccaccaacgtggtgatcaaggtgtgcgagttccagttctgcaatgatccttttctgggcgtgtactatcacaagaacaacaagagctggatggaaagcgagttcagagtgtattctagcgccaacaactgcacctttgagtacgtgtcccagccctttcttatggacctggaaggcaagcagggcaacttcaagaatctgagagaattcgtgttcaagaacattgatggctacttcaagatctacagcaagcacacccctatcaacctggttcgggacctgccacaaggcttcagcgccctggaacctctggtggacctgcctatcggcatcaacatcacacggttccaaaccctgcaccggagctacctgacccccggcgacagcagcagcggctggaccgccggcgctgccgcctattacgtgggctacctgcaacctagaaccttcctgctgaaatacaacgagaacggcacaatcaccgacgccgtggactgtgccctggaccccctgtctgagacaaagtgtaccctgaagtctttcaccgtggagaagggcatctaccagaccagcaacttccgggtgcagcctacagaatctatagtgcggttccctaacatcaccaacctgtgtccttttggcgaggtgttcaacgccactcggttcgcctctgtctacgcctggaaccggaaacggatctctaattgcgtggccgattacagcgtcctgtataactccgccagtttcagcacattcaagtgctacggcgtgtcacccaccaagctgaacgatctgtgcttcaccaatgtgtacgccgatagtttcgtgatccggggcgatgaggtgcggcagatcgcccctggacagacaggcaacatcgccgactacaactacaagctgcctgacgacttcacaggctgtgtgatcgcatggaacagcaacaacctggacagcaaggtgggcggaaactacaactacctgtacagactgttcagaaagtccaacctgaagcctttcgagagagatatatctaccgagatctaccaggccggcagcacaccctgtaatggagtgaaaggctttaactgctacttccctctgcaaagctatggatttcaacctacatatggggttggctaccagccttacagagtggtggtccttagcttcgagctgctccatgcccctgccaccgtgtgcggacctaagaagtccaccaacctggtgaaaaacaagtgcgtgaactttaattttaacggcctgaccggaacaggagtgctgacagaaagcaacaaaaagttcctgcctttccagcagttcggcagagacattgccgacaccacagatgctgttagagacccccagacgctggaaatcctggatatcaccccctgctcttttggcggcgtgagcgtgatcaccccaggcacaaacacaagcaaccaggtggctgtgctgtaccagggcgtgaactgtacagaggtccctgtggcaatccacgccgatcagctgacccctacatggcgggtgtactccactggatctaacgtgttccagacaagggccggatgcctcatcggcgctgagcacgtgaacaattcttacgagtgcgacatccctattggagcgggcatctgcgccagctaccagacacagaccaatagccctcagcaagccgctagcgtggcctcccagagcatcatcgcctacaccatgagcctgggagccgagaactctgtggcctacagcaacaacagcatcgctatccctaccaacttcaccatctctgtcaccaccgaaatcctgcccgtcagtatgaccaaaaccagcgtcgactgcaccatgtacatatgcggcgatagcaccgaatgcagcaacctgctgctgcagtatggctccttctgcacccaacttaacagagccctgactggcatcgccgtggagcaggacaagaatacccaggaggtgttcgcccaggtgaagcagatctacaagacacccccgatcaaggacttcggcggctttaatttctctcagatcctgccagacccatctaaaccctctaagcggagctttatcgaggacctgctgttcaacaaggtgactctggctgacgccggcttcatcaagcagtacggcgattgcctgggcgacattgctgctagagacctgatctgtgcccagaaattcaacggtcttactgtgctgcctcctctgctgacggatgagatgatcgcccagtacaccagcgccctgctggccggcaccatcacatccggctggacattcggcgccggcgcagccctgcagatcccttttgccatgcagatggcctaccggttcaacggaatcggagtgacacagaacgtgctctacgaaaatcagaagttgatcgccaaccagttcaacagcgccatcggcaagattcaggatagtctgagttccaccgccagcgccctgggaaagctgcaggacgtggtcaatcagaatgcccaagccctgaacaccctggtgaagcagctgagcagcaacttcggcgccatcagctctgtgctgaacgacatcctgagtagactggacaaggtggaagccgaagtgcagatcgacagattgatcaccggaagactgcaaagcctgcagacctacgtgacccagcagctgataagagctgctgaaatcagagccagcgctaatctggccgctaccaagatgagcgagtgcgttctgggccagtctaagagagtggacttctgcggaaaaggctaccacctgatgtcctttcctcagtctgccccccacggcgtggtgttcctgcacgtcacatacgtgcccgctcaagagaaaaacttcaccacggcccctgccatctgtcacgacggcaaggcccacttccccagagagggcgtgttcgtgagcaatggcacccactggtttgtgactcagagaaacttctacgagccacagattatcaccacagataacaccttcgtgtctggcaactgcgacgtggtgatcggcatcgtcaacaacacagtgtacgacccactgcaacctgagctggactcattcaaggaggaactggataagtacttcaagaatcacaccagccccgacgttgacctgggcgacatcagcggcattaacgcctctgtggtcaacatccagaaggaaatcgacagactgaatgaggtggccaagaatttgaacgagagcctgattgatctgcaggagctgggcaaatacgagcagtacatcaagtggccttggtacatctggctgggcttcatcgccgggctgatcgccatcgttatggtgacaatcatgctgtgttgcatgacaagctgttgtagctgcctgaaaggctgctgctcctgcggcagctgttgcaagtttgacgaagatgacagcgagcccgtgctgaaaggcgtcaagctgcactacacctgaggcgcgcccacccagcggccgcccgctacgccccaatgatccgaccagcaaaactcgatgtacttccgaggaactgatgtgcataatgcatcaggctggtacattagatccccgcttaccgcgggcaatatagcaacactaaaaactcgatgtacttccgaggaagcgcagtgcataatgctgcgcagtgttgccacataaccactatattaaccatttatctagcggacgccaaaaactcaatgtatttctgaggaagcgtggtgcataatgccacgcagcgtctgcataacttttattatttcttttattaatcaacaaaattttgtttttaacatttcaaaaaaaaaaaaaaaaaaaaaaaaaaaaaaaaaaaaagaagagcgtttaaacacgtgatatctggcctcatgggccttcctttcactgcccgctttccagtcgggaaacctgtcgtgccagctgcattaacatggtcatagctgtttccttgcgtattgggcgctctccgcttcctcgctcactgactcgctgcgctcggtcgttcgggtaaagcctggggtgcctaatgagcaaaaggccagcaaaaggccaggaaccgtaaaaaggccgcgttgctggcgtttttccataggctccgcccccctgacgagcatcacaaaaatcgacgctcaagtcagaggtggcgaaacccgacaggactataaagataccaggcgtttccccctggaagctccctcgtgcgctctcctgttccgaccctgccgcttaccggatacctgtccgcctttctcccttcgggaagcgtggcgctttctcatagctcacgctgtaggtatctcagttcggtgtaggtcgttcgctccaagctgggctgtgtgcacgaaccccccgttcagcccgaccgctgcgccttatccggtaactatcgtcttgagtccaacccggtaagacacgacttatcgccactggcagcagccactggtaacaggattagcagagcgaggtatgtaggcggtgctacagagttcttgaagtggtggcctaactacggctacactagaagaacagtatttggtatctgcgctctgctgaagccagttaccttcggaaaaagagttggtagctcttgatccggcaaacaaaccaccgctggtagcggtggtttttttgtttgcaggcagcagattacgcgcagaaaaaaaggatctcaagaagatcctttgatcttttctacggggtctgacgctcagtggaacgaaaactcacgttaagggattttggtcatgaatacacggtgcctgactgcgttagcaatttaactgtgataaactaccgcattaaagcttatcgatgataagctgtcaaacatgagaattcttagaaaaactcatcgagcatcaaatgaaactgcaatttattcatatcaggattatcaataccatatttttgaaaaagccgtttctgtaatgaaggagaaaactcaccgaggcagttccataggatggcaagatcctggtatcggtctgcgattccgactcgtccaacatcaatacaacctattaatttcccctcgtcaaaaataaggttatcaagtgagaaatcaccatgagtgacgactgaatccggtgagaatggcaaaagcttatgcatttctttccagacttgttcaacaggccagccattacgctcgtcatcaaaatcactcgcatcaaccaaaccgttattcattcgtgattgcgcctgagcgagacgaaatacgcgatcgctgttaaaaggacaattacaaacaggaatcgaatgcaaccggcgcaggaacactgccagcgcatcaacaatattttcacctgaatcaggatattcttctaatacctggaatgctgttttcccggggatcgcagtggtgagtaaccatgcatcatcaggagtacggataaaatgcttgatggtcggaagaggcataaattccgtcagccagtttagtctgaccatctcatctgtaacatcattggcaacgctacctttgccatgtttcagaaacaactctggcgcatcgggcttcccatacaatcgatagattgtcgcacctgattgcccgacattatcgcgagcccatttatacccatataaatcagcatccatgttggaatttaatcgcggcctcgagcaagacgtttcccgttgaatatggctcataacaccccttgtattactgtttatgtaagcagacagttttattgttcatgagcggatacatatttgaatgtatttagaaaaataaacaaataggggttccgcgcacatttccccgaaaagtgccacctaaattgtaagcgttaatattttgttaaaattcgcgttaaatttttgttaaatcagctcattttttaaccaataggccgaaatcggcaaaatcccttataaatcaaaagaatagaccgagatagggttgagtggccgctacagggcgctcccattcgccattcaggctgcgcaactgttgggaagggcgtttcggtgcgggcctcttcgctattacgccagctggcgaaagggggatgtgctgcaaggcgattaagttgggtaacgccagggttttcccagtcacacgcgtaatacgactcactatag

SEQ ID NO: 26 - DNA, 13996 bp, synthetic construct
  misc_feature 1..13996: note = Nucleotide sequence of construct Co79
  source 1..13996: mol_type = other DNA
ataggcggcgcatgagagaagcccagaccaattacctacccaaaatggagaaagttcacgttgacatcgaggaagacagcccattcctcagagctttgcagcggagcttcccgcagtttgaggtagaagccaagcaggtcactgataatgaccatgctaatgccagagcgttttcgcatctggcttcaaaactgatcgaaacggaggtggacccatccgacacgatccttgacattggaagtgcgcccgcccgcagaatgtattctaagcacaagtatcattgtatctgtccgatgagatgtgcggaagatccggacagattgtataagtatgcaactaagctgaagaaaaactgtaaggaaataactgataaggaattggacaagaaaatgaaggagctcgccgccgtcatgagcgaccctgacctggaaactgagactatgtgcctccacgacgacgagtcgtgtcgctacgaagggcaagtcgctgtttaccaggatgtatacgcggttgacggaccgacaagtctctatcaccaagccaataagggagttagagtcgcctactggataggctttgacaccaccccttttatgtttaagaacttggctggagcatatccatcatactctaccaactgggccgacgaaaccgtgttaacggctcgtaacataggcctatgcagctctgacgttatggagcggtcacgtagagggatgtccattcttagaaagaagtatttgaaaccatccaacaatgttctattctctgttggctcgaccatctaccacgagaagagggacttactgaggagctggcacctgccgtctgtatttcacttacgtggcaagcaaaattacacatgtcggtgtgagactatagttagttgcgacgggtacgtcgttaaaagaatagctatcagtccaggcctgtatgggaagccttcaggctatgctgctacgatgcaccgcgagggattcttgtgctgcaaagtgacagacacattgaacggggagagggtctcttttcccgtgtgcacgtatgtgccagctacattgtgtgaccaaatgactggcatactggcaacagatgtcagtgcggacgacgcgcaaaaactgctggttgggctcaaccagcgtatagtcgtcaacggtcgcacccagagaaacaccaataccatgaaaaattaccttttgcccgtagtggcccaggcatttgctaggtgggcaaaggaatataaggaagatcaagaagatgaaaggccactaggactacgagatagacagttagtcatggggtgttgttgggcttttagaaggcacaagataacatctatttataagcgcccggatacccaaaccatcatcaaagtgaacagcgatttccactcattcgtgctgcccaggataggcagtaacacattggagatcgggctgagaacaagaatcaggaaaatgttagaggagcacaaggagccgtcacctctcattaccgccgaggacgtacaagaagctaagtgcgcagccgatgaggctaaggaggtgcgtgaagccgaggagttgcgcgcagctctaccacctttggcagctgatgttgaggagcccactctggaagccgatgtcgacttgatgttacaagaggctggggccggctcagtggagacacctcgtggcttgataaaggttaccagctacgatggcgaggacaagatcggctcttacgctgtgctttctccgcaggctgtactcaagagtgaaaaattatcttgcatccaccctctcgctgaacaagtcatagtgataacacactctggccgaaaagggcgttatgccgtggaaccataccatggtaaagtagtggtgccagagggacatgcaatacccgtccaggactttcaagctctgagtgaaagtgccaccattgtgtacaacgaacgtgagttcgtaaacaggtacctgcaccatattgccacacatggaggagcgctgaacactgatgaagaatattacaaaactgtcaagcccagcgagcacgacggcgaatacctgtacgacatcgacaggaaacagtgcgtcaagaaagaactagtcactgggctagggctcacaggcgagctggtggatcctcccttccatgaattcgcctacgagagtctgagaacacgaccagccgctccttaccaagtaccaaccataggggtgtatggcgtgccaggatcaggcaagtctggcatcattaaaagcgcagtcaccaaaaaagatctagtggtgagcgccaagaaagaaaactgtgcagaaattataagggacgtcaagaaaatgaaagggctggacgtcaatgccagaactgtggactcagtgctcttgaatggatgcaaacaccccgtagagaccctgtatattgacgaagcttttgcttgtcatgcaggtactctcagagcgctcatagccattataagacctaaaaaggcagtgctctgcggggatcccaaacagtgcggtttttttaacatgatgtgcctgaaagtgcattttaaccacgagatttgcacacaagtcttccacaaaagcatctctcgccgttgcactaaatctgtgacttcggtcgtctcaaccttgttttacgacaaaaaaatgagaacgacgaatccgaaagagactaagattgtgattgacactaccggcagtaccaaacctaagcaggacgatctcattctcacttgtttcagagggtgggtgaagcagttgcaaatagattacaaaggcaacgaaataatgacggcagctgcctctcaagggctgacccgtaaaggtgtgtatgccgttcggtacaaggtgaatgaaaatcctctgtacgcacccacctcagaacatgtgaacgtcctactgacccgcacggaggaccgcatcgtgtggaaaacactagccggcgacccatggataaaaacactgactgccaagtaccctgggaatttcactgccacgatagaggagtggcaagcagagcatgatgccatcatgaggcacatcttggagagaccggaccctaccgacgtcttccagaataaggcaaacgtgtgttgggccaaggctttagtgccggtgctgaagaccgctggcatagacatgaccactgaacaatggaacactgtggattattttgaaacggacaaagctcactcagcagagatagtattgaaccaactatgcgtgaggttctttggactcgatctggactccggtctattttctgcacccactgttccgttatccattaggaataatcactgggataactccccgtcgcctaacatgtacgggctgaataaagaagtggtccgtcagctctctcgcaggtacccacaactgcctcgggcagttgccactggaagagtctatgacatgaacactggtacactgcgcaattatgatccgcgcataaacctagtacctgtaaacagaagactgcctcatgctttagtcctccaccataatgaacacccacagagtgacttttcttcattcgtcagcaaattgaagggcagaactgtcctggtggtcggggaaaagttgtccgtcccaggcaaaatggttgactggttgtcagaccggcctgaggctaccttcagagctcggctggatttaggcatcccaggtgatgtgcccaaatatgacataatatttgttaatgtgaggaccccatataaataccatcactatcagcagtgtgaagaccatgccattaagcttagcatgttgaccaagaaagcttgtctgcatctgaatcccggcggaacctgtgtcagcataggttatggttacgctgacagggccagcgaaagcatcattggtgctatagcgcggcagttcaagttttcccgggtatgcaaaccgaaatcctcacttgaagagacggaagttctgtttgtattcattgggtacgatcgcaaggcccgtacgcacaatccttacaagctttcatcaaccttgaccaacatttatacaggttccagactccacgaagccggatgtgcaccctcatatcatgtggtgcgaggggatattgccacggccaccgaaggagtgattataaatgctgctaacagcaaaggacaacctggcggaggggtgtgcggagcgctgtataagaaattcccggaaagcttcgatttacagccgatcgaagtaggaaaagcgcgactggtcaaaggtgcagctaaacatatcattcatgccgtaggaccaaacttcaacaaagtttcggaggttgaaggtgacaaacagttggcagaggcttatgagtccatcgctaagattgtcaacgataacaattacaagtcagtagcgattccactgttgtccaccggcatcttttccgggaacaaagatcgactaacccaatcattgaaccatttgctgacagctttagacaccactgatgcagatgtagccatatactgcagggacaagaaatgggaaatgactctcaaggaagcagtggctaggagagaagcagtggaggagatatgcatatccgacgactcttcagtgacagaacctgatgcagagctggtgagggtgcatccgaagagttctttggctggaaggaagggctacagcacaagcgatggcaaaactttctcatatttggaagggaccaagtttcaccaggcggccaaggatatagcagaaattaatgccatgtggcccgttgcaacggaggccaatgagcaggtatgcatgtatatcctcggagaaagcatgagcagtattaggtcgaaatgccccgtcgaagagtcggaagcctccacaccacctagcacgctgccttgcttgtgcatccatgccatgactccagaaagagtacagcgcctaaaagcctcacgtccagaacaaattactgtgtgctcatcctttccattgccgaagtatagaatcactggtgtgcagaagatccaatgctcccagcctatattgttctcaccgaaagtgcctgcgtatattcatccaaggaagtatctcgtggaaacaccaccggtagacgagactccggagccatcggcagagaaccaatccacagaggggacacctgaacaaccaccacttataaccgaggatgagaccaggactagaacgcctgagccgatcatcatcgaagaggaagaagaggatagcataagtttgctgtcagatggcccgacccaccaggtgctgcaagtcgaggcagacattcacgggccgccctctgtatctagctcatcctggtccattcctcatgcatccgactttgatgtggacagtttatccatacttgacaccctggagggagctagcgtgaccagcggggcaacgtcagccgagactaactcttacttcgcaaagagtatggagtttctggcgcgaccggtgcctgcgcctcgaacagtattcaggaaccctccacatcccgctccgcgcacaagaacaccgtcacttgcacccagcagggcctgctcgagaaccagcctagtttccaccccgccaggcgtgaatagggtgatcactagagaggagctcgaggcgcttaccccgtcacgcactcctagcaggtcggtctcgagaaccagcctggtctccaacccgccaggcgtaaatagggtgattacaagagaggagtttgaggcgttcgtagcacaacaacaatgacggtttgatgcgggtgcatacatcttttcctccgacaccggtcaagggcatttacaacaaaaatcagtaaggcaaacggtgctatccgaagtggtgttggagaggaccgaattggagatttcgtatgccccgcgcctcgaccaagaaaaagaagaattactacgcaagaaattacagttaaatcccacacctgctaacagaagcagataccagtccaggaaggtggagaacatgaaagccataacagctagacgtattctgcaaggcctagggcattatttgaaggcagaaggaaaagtggagtgctaccgaaccctgcatcctgttcctttgtattcatctagtgtgaaccgtgccttttcaagccccaaggtcgcagtggaagcctgtaacgccatgttgaaagagaactttccgactgtggcttcttactgtattattccagagtacgatgcctatttggacatggttgacggagcttcatgctgcttagacactgccagtttttgccctgcaaagctgcgcagctttccaaagaaacactcctatttggaacccacaatacgatcggcagtgccttcagcgatccagaacacgctccagaacgtcctggcagctgccacaaaaagaaattgcaatgtcacgcaaatgagagaattgcccgtattggattcggcggcctttaatgtggaatgcttcaagaaatatgcgtgtaataatgaatattgggaaacgtttaaagaaaaccccatcaggcttactgaagaaaacgtggtaaattacattaccaaattaaaaggaccaaaagctgctgctctttttgcgaagacacataatttgaatatgttgcaggacataccaatggacaggtttgtaatggacttaaagagagacgtgaaagtgactccaggaacaaaacatactgaagaacggcccaaggtacaggtgatccaggctgccgatccgctagcaacagcgtatctgtgcggaatccaccgagagctggttaggagattaaatgcggtcctgcttccgaacattcatacactgtttgatatgtcggctgaagactttgacgctattatagccgagcacttccagcctggggattgtgttctggaaactgacatcgcgtcgtttgataaaagtgaggacgacgccatggctctgaccgcgttaatgattctggaagacttaggtgtggacgcagagctgttgacgctgattgaggcggctttcggcgaaatttcatcaatacatttgcccactaaaactaaatttaaattcggagccatgatgaaatctggaatgttcctcacactgtttgtgaacacagtcattaacattgtaatcgcaagcagagtgttgagagaacggctaaccggatcaccatgtgcagcattcattggagatgacaatatcgtgaaaggagtcaaatcggacaaattaatggcagacaggtgcgccacctggttgaatatggaagtcaagattatagatgctgtggtgggcgagaaagcgccttatttctgtggagggtttattttgtgtgactccgtgaccggcacagcgtgccgtgtggcagaccccctaaaaaggctgtttaagcttggcaaacctctggcagcagacgatgaacatgatgatgacaggagaagggcattgcatgaagagtcaacacgctggaaccgagtgggtattctttcagagctgtgcaaggcagtagaatcaaggtatgaaaccgtaggaacttccatcatagttatggccatgactactctagctagcagtgttaaatcattcagctacctgagaggggcccctataactctctacggctaacctgaatggactacgacatagtctagtccgccaagatgttcgtgttcctggtgctgctgcccctcgttagcagccagtgcgtgaatctgaccacccgcacccagctgccaccagcctacacaaacagcttcaccagaggagtgtattaccctgataaggtctttagatcctccgtcctgcattctacgcaggatctcttcttgccattcttcagcaacgtgacatggttccacgccatctctggcaccaacggcacaaagcgcttcgacaatcctgtgttgccgtttaacgacggcgtttacttcgccagcacagaaaagagcaacatcatccggggctggatcttcggcaccaccctggacagcaaaacccaaagcctgctcatcgtgaacaacgccaccaacgtggtgatcaaggtgtgcgagttccagttctgcaatgatccttttctgggcgtgtatcacaagaacaacaagagctggatggaaagcgagttcagagtgtattctagcgccaacaactgcacctttgagtacgtgtcccagccctttcttatggacctggaaggcaagcagggcaacttcaagaatctgagagaattcgtgttcaagaacattgatggctacttcaagatctacagcaagcacacccctatcaacctggttcgggacctgccacaaggcttcagcgccctggaacctctggtggacctgcctatcggcatcaacatcacacggttccaaaccctgcaccggagctacctgacccccggcgacagcagcagcggctggaccgccggcgctgccgcctattacgtgggctacctgcaacctagaaccttcctgctgaaatacaacgagaacggcacaatcaccgacgccgtggactgtgccctggaccccctgtctgagacaaagtgtaccctgaagtctttcaccgtggagaagggcatctaccagaccagcaacttccgggtgcagcctacagaatctatagtgcggttccctaacatcaccaacctgtgtccttttggcgaggtgttcaacgccactcggttcgcctctgtctacgcctggaaccggaaacggatctctaattgcgtggccgattacagcgtcctgtataactccgccagtttcagcacattcaagtgctacggcgtgtcacccaccaagctgaacgatctgtgcttcaccaatgtgtacgccgatagtttcgtgatccggggcgatgaggtgcggcagatcgcccctggacagacaggcaacatcgccgactacaactacaagctgcctgacgacttcacaggctgtgtgatcgcatggaacagcaacaacctggacagcaaggtgggcggaaactacaactacctgtacagactgttcagaaagtccaacctgaagcctttcgagagagatatatctaccgagatctaccaggccggcagcacaccctgtaatggagtgaaaggctttaactgctacttccctctgcaaagctatggatttcaacctacatatggggttggctaccagccttacagagtggtggtccttagcttcgagctgctccatgcccctgccaccgtgtgcggacctaagaagtccaccaacctggtgaaaaacaagtgcgtgaactttaattttaacggcctgaccggaacaggagtgctgacagaaagcaacaaaaagttcctgcctttccagcagttcggcagagacattgccgacaccacagatgctgttagagacccccagacgctggaaatcctggatatcaccccctgctcttttggcggcgtgagcgtgatcaccccaggcacaaacacaagcaaccaggtggctgtgctgtaccagggcgtgaactgtacagaggtccctgtggcaatccacgccgatcagctgacccctacatggcgggtgtactccactggatctaacgtgttccagacaagggccggatgcctcatcggcgctgagcacgtgaacaattcttacgagtgcgacatccctattggagcgggcatctgcgccagctaccagacacagaccaatagccctcagcaagccgctagcgtggcctcccagagcatcatcgcctacaccatgagcctgggagccgagaactctgtggcctacagcaacaacagcatcgctatccctaccaacttcaccatctctgtcaccaccgaaatcctgcccgtcagtatgaccaaaaccagcgtcgactgcaccatgtacatatgcggcgatagcaccgaatgcagcaacctgctgctgcagtatggctccttctgcacccaacttaacagagccctgactggcatcgccgtggagcaggacaagaatacccaggaggtgttcgcccaggtgaagcagatctacaagacacccccgatcaaggacttcggcggctttaatttctctcagatcctgccagacccatctaaaccctctaagcggagctttatcgaggacctgctgttcaacaaggtgactctggctgacgccggcttcatcaagcagtacggcgattgcctgggcgacattgctgctagagacctgatctgtgcccagaaattcaacggtcttactgtgctgcctcctctgctgacggatgagatgatcgcccagtacaccagcgccctgctggccggcaccatcacatccggctggacattcggcgccggcgcagccctgcagatcccttttgccatgcagatggcctaccggttcaacggaatcggagtgacacagaacgtgctctacgaaaatcagaagttgatcgccaaccagttcaacagcgccatcggcaagattcaggatagtctgagttccaccgccagcgccctgggaaagctgcaggacgtggtcaatcagaatgcccaagccctgaacaccctggtgaagcagctgagcagcaacttcggcgccatcagctctgtgctgaacgacatcctgagtagactggacaaggtggaagccgaagtgcagatcgacagattgatcaccggaagactgcaaagcctgcagacctacgtgacccagcagctgataagagctgctgaaatcagagccagcgctaatctggccgctaccaagatgagcgagtgcgttctgggccagtctaagagagtggacttctgcggaaaaggctaccacctgatgtcctttcctcagtctgccccccacggcgtggtgttcctgcacgtcacatacgtgcccgctcaagagaaaaacttcaccacggcccctgccatctgtcacgacggcaaggcccacttccccagagagggcgtgttcgtgagcaatggcacccactggtttgtgactcagagaaacttctacgagccacagattatcaccacagataacaccttcgtgtctggcaactgcgacgtggtgatcggcatcgtcaacaacacagtgtacgacccactgcaacctgagctggactcattcaaggaggaactggataagtacttcaagaatcacaccagccccgacgttgacctgggcgacatcagcggcattaacgcctctgtggtcaacatccagaaggaaatcgacagactgaatgaggtggccaagaatttgaacgagagcctgattgatctgcaggagctgggcaaatacgagcagtacatcaagtggccttggtacatctggctgggcttcatcgccgggctgatcgccatcgttatggtgacaatcatgctgtgttgcatgacaagctgttgtagctgcctgaaaggctgctgctcctgcggcagctgttgcaagtttgacgaagatgacagcgagcccgtgctgaaaggcgtcaagctgcactacacctgaggcgcgcccacccagcggccgcccgctacgccccaatgatccgaccagcaaaactcgatgtacttccgaggaactgatgtgcataatgcatcaggctggtacattagatccccgcttaccgcgggcaatatagcaacactaaaaactcgatgtacttccgaggaagcgcagtgcataatgctgcgcagtgttgccacataaccactatattaaccatttatctagcggacgccaaaaactcaatgtatttctgaggaagcgtggtgcataatgccacgcagcgtctgcataacttttattatttcttttattaatcaacaaaattttgtttttaacatttcaaaaaaaaaaaaaaaaaaaaaaaaaaaaaaaaaaaaagaagagcgtttaaacacgtgatatctggcctcatgggccttcctttcactgcccgctttccagtcgggaaacctgtcgtgccagctgcattaacatggtcatagctgtttccttgcgtattgggcgctctccgcttcctcgctcactgactcgctgcgctcggtcgttcgggtaaagcctggggtgcctaatgagcaaaaggccagcaaaaggccaggaaccgtaaaaaggccgcgttgctggcgtttttccataggctccgcccccctgacgagcatcacaaaaatcgacgctcaagtcagaggtggcgaaacccgacaggactataaagataccaggcgtttccccctggaagctccctcgtgcgctctcctgttccgaccctgccgcttaccggatacctgtccgcctttctcccttcgggaagcgtggcgctttctcatagctcacgctgtaggtatctcagttcggtgtaggtcgttcgctccaagctgggctgtgtgcacgaaccccccgttcagcccgaccgctgcgccttatccggtaactatcgtcttgagtccaacccggtaagacacgacttatcgccactggcagcagccactggtaacaggattagcagagcgaggtatgtaggcggtgctacagagttcttgaagtggtggcctaactacggctacactagaagaacagtatttggtatctgcgctctgctgaagccagttaccttcggaaaaagagttggtagctcttgatccggcaaacaaaccaccgctggtagcggtggtttttttgtttgcaggcagcagattacgcgcagaaaaaaaggatctcaagaagatcctttgatcttttctacggggtctgacgctcagtggaacgaaaactcacgttaagggattttggtcatgaatacacggtgcctgactgcgttagcaatttaactgtgataaactaccgcattaaagcttatcgatgataagctgtcaaacatgagaattcttagaaaaactcatcgagcatcaaatgaaactgcaatttattcatatcaggattatcaataccatatttttgaaaaagccgtttctgtaatgaaggagaaaactcaccgaggcagttccataggatggcaagatcctggtatcggtctgcgattccgactcgtccaacatcaatacaacctattaatttcccctcgtcaaaaataaggttatcaagtgagaaatcaccatgagtgacgactgaatccggtgagaatggcaaaagcttatgcatttctttccagacttgttcaacaggccagccattacgctcgtcatcaaaatcactcgcatcaaccaaaccgttattcattcgtgattgcgcctgagcgagacgaaatacgcgatcgctgttaaaaggacaattacaaacaggaatcgaatgcaaccggcgcaggaacactgccagcgcatcaacaatattttcacctgaatcaggatattcttctaatacctggaatgctgttttcccggggatcgcagtggtgagtaaccatgcatcatcaggagtacggataaaatgcttgatggtcggaagaggcataaattccgtcagccagtttagtctgaccatctcatctgtaacatcattggcaacgctacctttgccatgtttcagaaacaactctggcgcatcgggcttcccatacaatcgatagattgtcgcacctgattgcccgacattatcgcgagcccatttatacccatataaatcagcatccatgttggaatttaatcgcggcctcgagcaagacgtttcccgttgaatatggctcataacaccccttgtattactgtttatgtaagcagacagttttattgttcatgagcggatacatatttgaatgtatttagaaaaataaacaaataggggttccgcgcacatttccccgaaaagtgccacctaaattgtaagcgttaatattttgttaaaattcgcgttaaatttttgttaaatcagctcattttttaaccaataggccgaaatcggcaaaatcccttataaatcaaaagaatagaccgagatagggttgagtggccgctacagggcgctcccattcgccattcaggctgcgcaactgttgggaagggcgtttcggtgcgggcctcttcgctattacgccagctggcgaaagggggatgtgctgcaaggcgattaagttgggtaacgccagggttttcccagtcacacgcgtaatacgactcactatag

SEQ ID NO: 27 - DNA, 14005 bp, synthetic construct
  misc_feature 1..14005: note = Nucleotide sequence of construct Co80
  source 1..14005: mol_type = other DNA
ataggcggcgcatgagagaagcccagaccaattacctacccaaaatggagaaagttcacgttgacatcgaggaagacagcccattcctcagagctttgcagcggagcttcccgcagtttgaggtagaagccaagcaggtcactgataatgaccatgctaatgccagagcgttttcgcatctggcttcaaaactgatcgaaacggaggtggacccatccgacacgatccttgacattggaagtgcgcccgcccgcagaatgtattctaagcacaagtatcattgtatctgtccgatgagatgtgcggaagatccggacagattgtataagtatgcaactaagctgaagaaaaactgtaaggaaataactgataaggaattggacaagaaaatgaaggagctcgccgccgtcatgagcgaccctgacctggaaactgagactatgtgcctccacgacgacgagtcgtgtcgctacgaagggcaagtcgctgtttaccaggatgtatacgcggttgacggaccgacaagtctctatcaccaagccaataagggagttagagtcgcctactggataggctttgacaccaccccttttatgtttaagaacttggctggagcatatccatcatactctaccaactgggccgacgaaaccgtgttaacggctcgtaacataggcctatgcagctctgacgttatggagcggtcacgtagagggatgtccattcttagaaagaagtatttgaaaccatccaacaatgttctattctctgttggctcgaccatctaccacgagaagagggacttactgaggagctggcacctgccgtctgtatttcacttacgtggcaagcaaaattacacatgtcggtgtgagactatagttagttgcgacgggtacgtcgttaaaagaatagctatcagtccaggcctgtatgggaagccttcaggctatgctgctacgatgcaccgcgagggattcttgtgctgcaaagtgacagacacattgaacggggagagggtctcttttcccgtgtgcacgtatgtgccagctacattgtgtgaccaaatgactggcatactggcaacagatgtcagtgcggacgacgcgcaaaaactgctggttgggctcaaccagcgtatagtcgtcaacggtcgcacccagagaaacaccaataccatgaaaaattaccttttgcccgtagtggcccaggcatttgctaggtgggcaaaggaatataaggaagatcaagaagatgaaaggccactaggactacgagatagacagttagtcatggggtgttgttgggcttttagaaggcacaagataacatctatttataagcgcccggatacccaaaccatcatcaaagtgaacagcgatttccactcattcgtgctgcccaggataggcagtaacacattggagatcgggctgagaacaagaatcaggaaaatgttagaggagcacaaggagccgtcacctctcattaccgccgaggacgtacaagaagctaagtgcgcagccgatgaggctaaggaggtgcgtgaagccgaggagttgcgcgcagctctaccacctttggcagctgatgttgaggagcccactctggaagccgatgtcgacttgatgttacaagaggctggggccggctcagtggagacacctcgtggcttgataaaggttaccagctacgatggcgaggacaagatcggctcttacgctgtgctttctccgcaggctgtactcaagagtgaaaaattatcttgcatccaccctctcgctgaacaagtcatagtgataacacactctggccgaaaagggcgttatgccgtggaaccataccatggtaaagtagtggtgccagagggacatgcaatacccgtccaggactttcaagctctgagtgaaagtgccaccattgtgtacaacgaacgtgagttcgtaaacaggtacctgcaccatattgccacacatggaggagcgctgaacactgatgaagaatattacaaaactgtcaagcccagcgagcacgacggcgaatacctgtacgacatcgacaggaaacagtgcgtcaagaaagaactagtcactgggctagggctcacaggcgagctggtggatcctcccttccatgaattcgcctacgagagtctgagaacacgaccagccgctccttaccaagtaccaaccataggggtgtatggcgtgccaggatcaggcaagtctggcatcattaaaagcgcagtcaccaaaaaagatctagtggtgagcgccaagaaagaaaactgtgcagaaattataagggacgtcaagaaaatgaaagggctggacgtcaatgccagaactgtggactcagtgctcttgaatggatgcaaacaccccgtagagaccctgtatattgacgaagcttttgcttgtcatgcaggtactctcagagcgctcatagccattataagacctaaaaaggcagtgctctgcggggatcccaaacagtgcggtttttttaacatgatgtgcctgaaagtgcattttaaccacgagatttgcacacaagtcttccacaaaagcatctctcgccgttgcactaaatctgtgacttcggtcgtctcaaccttgttttacgacaaaaaaatgagaacgacgaatccgaaagagactaagattgtgattgacactaccggcagtaccaaacctaagcaggacgatctcattctcacttgtttcagagggtgggtgaagcagttgcaaatagattacaaaggcaacgaaataatgacggcagctgcctctcaagggctgacccgtaaaggtgtgtatgccgttcggtacaaggtgaatgaaaatcctctgtacgcacccacctcagaacatgtgaacgtcctactgacccgcacggaggaccgcatcgtgtggaaaacactagccggcgacccatggataaaaacactgactgccaagtaccctgggaatttcactgccacgatagaggagtggcaagcagagcatgatgccatcatgaggcacatcttggagagaccggaccctaccgacgtcttccagaataaggcaaacgtgtgttgggccaaggctttagtgccggtgctgaagaccgctggcatagacatgaccactgaacaatggaacactgtggattattttgaaacggacaaagctcactcagcagagatagtattgaaccaactatgcgtgaggttctttggactcgatctggactccggtctattttctgcacccactgttccgttatccattaggaataatcactgggataactccccgtcgcctaacatgtacgggctgaataaagaagtggtccgtcagctctctcgcaggtacccacaactgcctcgggcagttgccactggaagagtctatgacatgaacactggtacactgcgcaattatgatccgcgcataaacctagtacctgtaaacagaagactgcctcatgctttagtcctccaccataatgaacacccacagagtgacttttcttcattcgtcagcaaattgaagggcagaactgtcctggtggtcggggaaaagttgtccgtcccaggcaaaatggttgactggttgtcagaccggcctgaggctaccttcagagctcggctggatttaggcatcccaggtgatgtgcccaaatatgacataatatttgttaatgtgaggaccccatataaataccatcactatcagcagtgtgaagaccatgccattaagcttagcatgttgaccaagaaagcttgtctgcatctgaatcccggcggaacctgtgtcagcataggttatggttacgctgacagggccagcgaaagcatcattggtgctatagcgcggcagttcaagttttcccgggtatgcaaaccgaaatcctcacttgaagagacggaagttctgtttgtattcattgggtacgatcgcaaggcccgtacgcacaatccttacaagctttcatcaaccttgaccaacatttatacaggttccagactccacgaagccggatgtgcaccctcatatcatgtggtgcgaggggatattgccacggccaccgaaggagtgattataaatgctgctaacagcaaaggacaacctggcggaggggtgtgcggagcgctgtataagaaattcccggaaagcttcgatttacagccgatcgaagtaggaaaagcgcgactggtcaaaggtgcagctaaacatatcattcatgccgtaggaccaaacttcaacaaagtttcggaggttgaaggtgacaaacagttggcagaggcttatgagtccatcgctaagattgtcaacgataacaattacaagtcagtagcgattccactgttgtccaccggcatcttttccgggaacaaagatcgactaacccaatcattgaaccatttgctgacagctttagacaccactgatgcagatgtagccatatactgcagggacaagaaatgggaaatgactctcaaggaagcagtggctaggagagaagcagtggaggagatatgcatatccgacgactcttcagtgacagaacctgatgcagagctggtgagggtgcatccgaagagttctttggctggaaggaagggctacagcacaagcgatggcaaaactttctcatatttggaagggaccaagtttcaccaggcggccaaggatatagcagaaattaatgccatgtggcccgttgcaacggaggccaatgagcaggtatgcatgtatatcctcggagaaagcatgagcagtattaggtcgaaatgccccgtcgaagagtcggaagcctccacaccacctagcacgctgccttgcttgtgcatccatgccatgactccagaaagagtacagcgcctaaaagcctcacgtccagaacaaattactgtgtgctcatcctttccattgccgaagtatagaatcactggtgtgcagaagatccaatgctcccagcctatattgttctcaccgaaagtgcctgcgtatattcatccaaggaagtatctcgtggaaacaccaccggtagacgagactccggagccatcggcagagaaccaatccacagaggggacacctgaacaaccaccacttataaccgaggatgagaccaggactagaacgcctgagccgatcatcatcgaagaggaagaagaggatagcataagtttgctgtcagatggcccgacccaccaggtgctgcaagtcgaggcagacattcacgggccgccctctgtatctagctcatcctggtccattcctcatgcatccgactttgatgtggacagtttatccatacttgacaccctggagggagctagcgtgaccagcggggcaacgtcagccgagactaactcttacttcgcaaagagtatggagtttctggcgcgaccggtgcctgcgcctcgaacagtattcaggaaccctccacatcccgctccgcgcacaagaacaccgtcacttgcacccagcagggcctgctcgagaaccagcctagtttccaccccgccaggcgtgaatagggtgatcactagagaggagctcgaggcgcttaccccgtcacgcactcctagcaggtcggtctcgagaaccagcctggtctccaacccgccaggcgtaaatagggtgattacaagagaggagtttgaggcgttcgtagcacaacaacaatgacggtttgatgcgggtgcatacatcttttcctccgacaccggtcaagggcatttacaacaaaaatcagtaaggcaaacggtgctatccgaagtggtgttggagaggaccgaattggagatttcgtatgccccgcgcctcgaccaagaaaaagaagaattactacgcaagaaattacagttaaatcccacacctgctaacagaagcagataccagtccaggaaggtggagaacatgaaagccataacagctagacgtattctgcaaggcctagggcattatttgaaggcagaaggaaaagtggagtgctaccgaaccctgcatcctgttcctttgtattcatctagtgtgaaccgtgccttttcaagccccaaggtcgcagtggaagcctgtaacgccatgttgaaagagaactttccgactgtggcttcttactgtattattccagagtacgatgcctatttggacatggttgacggagcttcatgctgcttagacactgccagtttttgccctgcaaagctgcgcagctttccaaagaaacactcctatttggaacccacaatacgatcggcagtgccttcagcgatccagaacacgctccagaacgtcctggcagctgccacaaaaagaaattgcaatgtcacgcaaatgagagaattgcccgtattggattcggcggcctttaatgtggaatgcttcaagaaatatgcgtgtaataatgaatattgggaaacgtttaaagaaaaccccatcaggcttactgaagaaaacgtggtaaattacattaccaaattaaaaggaccaaaagctgctgctctttttgcgaagacacataatttgaatatgttgcaggacataccaatggacaggtttgtaatggacttaaagagagacgtgaaagtgactccaggaacaaaacatactgaagaacggcccaaggtacaggtgatccaggctgccgatccgctagcaacagcgtatctgtgcggaatccaccgagagctggttaggagattaaatgcggtcctgcttccgaacattcatacactgtttgatatgtcggctgaagactttgacgctattatagccgagcacttccagcctggggattgtgttctggaaactgacatcgcgtcgtttgataaaagtgaggacgacgccatggctctgaccgcgttaatgattctggaagacttaggtgtggacgcagagctgttgacgctgattgaggcggctttcggcgaaatttcatcaatacatttgcccactaaaactaaatttaaattcggagccatgatgaaatctggaatgttcctcacactgtttgtgaacacagtcattaacattgtaatcgcaagcagagtgttgagagaacggctaaccggatcaccatgtgcagcattcattggagatgacaatatcgtgaaaggagtcaaatcggacaaattaatggcagacaggtgcgccacctggttgaatatggaagtcaagattatagatgctgtggtgggcgagaaagcgccttatttctgtggagggtttattttgtgtgactccgtgaccggcacagcgtgccgtgtggcagaccccctaaaaaggctgtttaagcttggcaaacctctggcagcagacgatgaacatgatgatgacaggagaagggcattgcatgaagagtcaacacgctggaaccgagtgggtattctttcagagctgtgcaaggcagtagaatcaaggtatgaaaccgtaggaacttccatcatagttatggccatgactactctagctagcagtgttaaatcattcagctacctgagaggggcccctataactctctacggctaacctgaatggactacgacatagtctagtccgccaagatgttcgtgttcctggtgctgctgcccctcgttagcagccagtgcgtgaatctgaccacccgcacccagctgccaccagcctacacaaacagcttcaccagaggagtgtattaccctgataaggtctttagatcctccgtcctgcattctacgcaggatctcttcttgccattcttcagcaacgtgacatggttccacgccatctctggcaccaacggcacaaagcgcttcgacaatcctgtgttgccgtttaacgacggcgtttacttcgccagcacagaaaagagcaacatcatccggggctggatcttcggcaccaccctggacagcaaaacccaaagcctgctcatcgtgaacaacgccaccaacgtggtgatcaaggtgtgcgagttccagttctgcaatgatccttttctgggcgtgtatcacaagaacaacaagagctggatggaaagcgagttcagagtgtattctagcgccaacaactgcacctttgagtacgtgtcccagccctttcttatggacctggaaggcaagcagggcaacttcaagaatctgagagaattcgtgttcaagaacattgatggctacttcaagatctacagcaagcacacccctatcaacctggttcgggacctgccacaaggcttcagcgccctggaacctctggtggacctgcctatcggcatcaacatcacacggttccaaaccctgctggccctgcaccggagctacctgacccccggcgacagcagcagcggctggaccgccggcgctgccgcctattacgtgggctacctgcaacctagaaccttcctgctgaaatacaacgagaacggcacaatcaccgacgccgtggactgtgccctggaccccctgtctgagacaaagtgtaccctgaagtctttcaccgtggagaagggcatctaccagaccagcaacttccgggtgcagcctacagaatctatagtgcggttccctaacatcaccaacctgtgtccttttggcgaggtgttcaacgccactcggttcgcctctgtctacgcctggaaccggaaacggatctctaattgcgtggccgattacagcgtcctgtataactccgccagtttcagcacattcaagtgctacggcgtgtcacccaccaagctgaacgatctgtgcttcaccaatgtgtacgccgatagtttcgtgatccggggcgatgaggtgcggcagatcgcccctggacagacaggcaagatcgccgactacaactacaagctgcctgacgacttcacaggctgtgtgatcgcatggaacagcaacaacctggacagcaaggtgggcggaaactacaactacctgtacagactgttcagaaagtccaacctgaagcctttcgagagagatatatctaccgagatctaccaggccggcagcacaccctgtaatggagtggaaggctttaactgctacttccctctgcaaagctatggatttcaacctacatatggggttggctaccagccttacagagtggtggtccttagcttcgagctgctccatgcccctgccaccgtgtgcggacctaagaagtccaccaacctggtgaaaaacaagtgcgtgaactttaattttaacggcctgaccggaacaggagtgctgacagaaagcaacaaaaagttcctgcctttccagcagttcggcagagacattgacgacaccacagatgctgttagagacccccagacgctggaaatcctggatatcaccccctgctcttttggcggcgtgagcgtgatcaccccaggcacaaacacaagcaaccaggtggctgtgctgtaccagggcgtgaactgtacagaggtccctgtggcaatccacgccgatcagctgacccctacatggcgggtgtactccactggatctaacgtgttccagacaagggccggatgcctcatcggcgctgagcacgtgaacaattcttacgagtgcgacatccctattggagcgggcatctgcgccagctaccagacacagaccaatagccatcagcaagccgctagcgtggcctcccagagcatcatcgcctacaccatgagcctgggagccgagaactctgtggcctacagcaacaacagcatcgctatccctatcaacttcaccatctctgtcaccaccgaaatcctgcccgtcagtatgaccaaaaccagcgtcgactgcaccatgtacatatgcggcgatagcaccgaatgcagcaacctgctgctgcagtatggctccttctgcacccaacttaacagagccctgactggcatcgccgtggagcaggacaagaatacccaggaggtgttcgcccaggtgaagcagatctacaagacacccccgatcaaggacttcggcggctttaatttctctcagatcctgccagacccatctaaaccctctaagcggagctttatcgaggacctgctgttcaacaaggtgactctggctgacgccggcttcatcaagcagtacggcgattgcctgggcgacattgctgctagagacctgatctgtgcccagaaattcaacggtcttactgtgctgcctcctctgctgacggatgagatgatcgcccagtacaccagcgccctgctggccggcaccatcacatccggctggacattcggcgccggcgcagccctgcagatcccttttgccatgcagatggcctaccggttcaacggaatcggagtgacacagaacgtgctctacgaaaatcagaagttgatcgccaaccagttcaacagcgccatcggcaagattcaggatagtctgagttccaccgccagcgccctgggaaagctgcaggacgtggtcaatcagaatgcccaagccctgaacaccctggtgaagcagctgagcagcaacttcggcgccatcagctctgtgctgaacgacatcctggctagactggacaaggtggaagccgaagtgcagatcgacagattgatcaccggaagactgcaaagcctgcagacctacgtgacccagcagctgataagagctgctgaaatcagagccagcgctaatctggccgctaccaagatgagcgagtgcgttctgggccagtctaagagagtggacttctgcggaaaaggctaccacctgatgtcctttcctcagtctgccccccacggcgtggtgttcctgcacgtcacatacgtgcccgctcaagagaaaaacttcaccacggcccctgccatctgtcacgacggcaaggcccacttccccagagagggcgtgttcgtgagcaatggcacccactggtttgtgactcagagaaacttctacgagccacagattatcaccacacataacaccttcgtgtctggcaactgcgacgtggtgatcggcatcgtcaacaacacagtgtacgacccactgcaacctgagctggactcattcaaggaggaactggataagtacttcaagaatcacaccagccccgacgttgacctgggcgacatcagcggcattaacgcctctgtggtcaacatccagaaggaaatcgacagactgaatgaggtggccaagaatttgaacgagagcctgattgatctgcaggagctgggcaaatacgagcagtacatcaagtggccttggtacatctggctgggcttcatcgccgggctgatcgccatcgttatggtgacaatcatgctgtgttgcatgacaagctgttgtagctgcctgaaaggctgctgctcctgcggcagctgttgcaagtttgacgaagatgacagcgagcccgtgctgaaaggcgtcaagctgcactacacctgaggcgcgcccacccagcggccgcccgctacgccccaatgatccgaccagcaaaactcgatgtacttccgaggaactgatgtgcataatgcatcaggctggtacattagatccccgcttaccgcgggcaatatagcaacactaaaaactcgatgtacttccgaggaagcgcagtgcataatgctgcgcagtgttgccacataaccactatattaaccatttatctagcggacgccaaaaactcaatgtatttctgaggaagcgtggtgcataatgccacgcagcgtctgcataacttttattatttcttttattaatcaacaaaattttgtttttaacatttcaaaaaaaaaaaaaaaaaaaaaaaaaaaaaaaaaaaaagaagagcgtttaaacacgtgatatctggcctcatgggccttcctttcactgcccgctttccagtcgggaaacctgtcgtgccagctgcattaacatggtcatagctgtttccttgcgtattgggcgctctccgcttcctcgctcactgactcgctgcgctcggtcgttcgggtaaagcctggggtgcctaatgagcaaaaggccagcaaaaggccaggaaccgtaaaaaggccgcgttgctggcgtttttccataggctccgcccccctgacgagcatcacaaaaatcgacgctcaagtcagaggtggcgaaacccgacaggactataaagataccaggcgtttccccctggaagctccctcgtgcgctctcctgttccgaccctgccgcttaccggatacctgtccgcctttctcccttcgggaagcgtggcgctttctcatagctcacgctgtaggtatctcagttcggtgtaggtcgttcgctccaagctgggctgtgtgcacgaaccccccgttcagcccgaccgctgcgccttatccggtaactatcgtcttgagtccaacccggtaagacacgacttatcgccactggcagcagccactggtaacaggattagcagagcgaggtatgtaggcggtgctacagagttcttgaagtggtggcctaactacggctacactagaagaacagtatttggtatctgcgctctgctgaagccagttaccttcggaaaaagagttggtagctcttgatccggcaaacaaaccaccgctggtagcggtggtttttttgtttgcaggcagcagattacgcgcagaaaaaaaggatctcaagaagatcctttgatcttttctacggggtctgacgctcagtggaacgaaaactcacgttaagggattttggtcatgaatacacggtgcctgactgcgttagcaatttaactgtgataaactaccgcattaaagcttatcgatgataagctgtcaaacatgagaattcttagaaaaactcatcgagcatcaaatgaaactgcaatttattcatatcaggattatcaataccatatttttgaaaaagccgtttctgtaatgaaggagaaaactcaccgaggcagttccataggatggcaagatcctggtatcggtctgcgattccgactcgtccaacatcaatacaacctattaatttcccctcgtcaaaaataaggttatcaagtgagaaatcaccatgagtgacgactgaatccggtgagaatggcaaaagcttatgcatttctttccagacttgttcaacaggccagccattacgctcgtcatcaaaatcactcgcatcaaccaaaccgttattcattcgtgattgcgcctgagcgagacgaaatacgcgatcgctgttaaaaggacaattacaaacaggaatcgaatgcaaccggcgcaggaacactgccagcgcatcaacaatattttcacctgaatcaggatattcttctaatacctggaatgctgttttcccggggatcgcagtggtgagtaaccatgcatcatcaggagtacggataaaatgcttgatggtcggaagaggcataaattccgtcagccagtttagtctgaccatctcatctgtaacatcattggcaacgctacctttgccatgtttcagaaacaactctggcgcatcgggcttcccatacaatcgatagattgtcgcacctgattgcccgacattatcgcgagcccatttatacccatataaatcagcatccatgttggaatttaatcgcggcctcgagcaagacgtttcccgttgaatatggctcataacaccccttgtattactgtttatgtaagcagacagttttattgttcatgagcggatacatatttgaatgtatttagaaaaataaacaaataggggttccgcgcacatttccccgaaaagtgccacctaaattgtaagcgttaatattttgttaaaattcgcgttaaatttttgttaaatcagctcattttttaaccaataggccgaaatcggcaaaatcccttataaatcaaaagaatagaccgagatagggttgagtggccgctacagggcgctcccattcgccattcaggctgcgcaactgttgggaagggcgtttcggtgcgggcctcttcgctattacgccagctggcgaaagggggatgtgctgcaaggcgattaagttgggtaacgccagggttttcccagtcacacgcgtaatacgactcactatag

SEQ ID NO: 28 - DNA, 14005 bp, synthetic construct
  misc_feature 1..14005: note = Nucleotide sequence of construct Co81
  source 1..14005: mol_type = other DNA
ataggcggcgcatgagagaagcccagaccaattacctacccaaaatggagaaagttcacgttgacatcgaggaagacagcccattcctcagagctttgcagcggagcttcccgcagtttgaggtagaagccaagcaggtcactgataatgaccatgctaatgccagagcgttttcgcatctggcttcaaaactgatcgaaacggaggtggacccatccgacacgatccttgacattggaagtgcgcccgcccgcagaatgtattctaagcacaagtatcattgtatctgtccgatgagatgtgcggaagatccggacagattgtataagtatgcaactaagctgaagaaaaactgtaaggaaataactgataaggaattggacaagaaaatgaaggagctcgccgccgtcatgagcgaccctgacctggaaactgagactatgtgcctccacgacgacgagtcgtgtcgctacgaagggcaagtcgctgtttaccaggatgtatacgcggttgacggaccgacaagtctctatcaccaagccaataagggagttagagtcgcctactggataggctttgacaccaccccttttatgtttaagaacttggctggagcatatccatcatactctaccaactgggccgacgaaaccgtgttaacggctcgtaacataggcctatgcagctctgacgttatggagcggtcacgtagagggatgtccattcttagaaagaagtatttgaaaccatccaacaatgttctattctctgttggctcgaccatctaccacgagaagagggacttactgaggagctggcacctgccgtctgtatttcacttacgtggcaagcaaaattacacatgtcggtgtgagactatagttagttgcgacgggtacgtcgttaaaagaatagctatcagtccaggcctgtatgggaagccttcaggctatgctgctacgatgcaccgcgagggattcttgtgctgcaaagtgacagacacattgaacggggagagggtctcttttcccgtgtgcacgtatgtgccagctacattgtgtgaccaaatgactggcatactggcaacagatgtcagtgcggacgacgcgcaaaaactgctggttgggctcaaccagcgtatagtcgtcaacggtcgcacccagagaaacaccaataccatgaaaaattaccttttgcccgtagtggcccaggcatttgctaggtgggcaaaggaatataaggaagatcaagaagatgaaaggccactaggactacgagatagacagttagtcatggggtgttgttgggcttttagaaggcacaagataacatctatttataagcgcccggatacccaaaccatcatcaaagtgaacagcgatttccactcattcgtgctgcccaggataggcagtaacacattggagatcgggctgagaacaagaatcaggaaaatgttagaggagcacaaggagccgtcacctctcattaccgccgaggacgtacaagaagctaagtgcgcagccgatgaggctaaggaggtgcgtgaagccgaggagttgcgcgcagctctaccacctttggcagctgatgttgaggagcccactctggaagccgatgtcgacttgatgttacaagaggctggggccggctcagtggagacacctcgtggcttgataaaggttaccagctacgatggcgaggacaagatcggctcttacgctgtgctttctccgcaggctgtactcaagagtgaaaaattatcttgcatccaccctctcgctgaacaagtcatagtgataacacactctggccgaaaagggcgttatgccgtggaaccataccatggtaaagtagtggtgccagagggacatgcaatacccgtccaggactttcaagctctgagtgaaagtgccaccattgtgtacaacgaacgtgagttcgtaaacaggtacctgcaccatattgccacacatggaggagcgctgaacactgatgaagaatattacaaaactgtcaagcccagcgagcacgacggcgaatacctgtacgacatcgacaggaaacagtgcgtcaagaaagaactagtcactgggctagggctcacaggcgagctggtggatcctcccttccatgaattcgcctacgagagtctgagaacacgaccagccgctccttaccaagtaccaaccataggggtgtatggcgtgccaggatcaggcaagtctggcatcattaaaagcgcagtcaccaaaaaagatctagtggtgagcgccaagaaagaaaactgtgcagaaattataagggacgtcaagaaaatgaaagggctggacgtcaatgccagaactgtggactcagtgctcttgaatggatgcaaacaccccgtagagaccctgtatattgacgaagcttttgcttgtcatgcaggtactctcagagcgctcatagccattataagacctaaaaaggcagtgctctgcggggatcccaaacagtgcggtttttttaacatgatgtgcctgaaagtgcattttaaccacgagatttgcacacaagtcttccacaaaagcatctctcgccgttgcactaaatctgtgacttcggtcgtctcaaccttgttttacgacaaaaaaatgagaacgacgaatccgaaagagactaagattgtgattgacactaccggcagtaccaaacctaagcaggacgatctcattctcacttgtttcagagggtgggtgaagcagttgcaaatagattacaaaggcaacgaaataatgacggcagctgcctctcaagggctgacccgtaaaggtgtgtatgccgttcggtacaaggtgaatgaaaatcctctgtacgcacccacctcagaacatgtgaacgtcctactgacccgcacggaggaccgcatcgtgtggaaaacactagccggcgacccatggataaaaacactgactgccaagtaccctgggaatttcactgccacgatagaggagtggcaagcagagcatgatgccatcatgaggcacatcttggagagaccggaccctaccgacgtcttccagaataaggcaaacgtgtgttgggccaaggctttagtgccggtgctgaagaccgctggcatagacatgaccactgaacaatggaacactgtggattattttgaaacggacaaagctcactcagcagagatagtattgaaccaactatgcgtgaggttctttggactcgatctggactccggtctattttctgcacccactgttccgttatccattaggaataatcactgggataactccccgtcgcctaacatgtacgggctgaataaagaagtggtccgtcagctctctcgcaggtacccacaactgcctcgggcagttgccactggaagagtctatgacatgaacactggtacactgcgcaattatgatccgcgcataaacctagtacctgtaaacagaagactgcctcatgctttagtcctccaccataatgaacacccacagagtgacttttcttcattcgtcagcaaattgaagggcagaactgtcctggtggtcggggaaaagttgtccgtcccaggcaaaatggttgactggttgtcagaccggcctgaggctaccttcagagctcggctggatttaggcatcccaggtgatgtgcccaaatatgacataatatttgttaatgtgaggaccccatataaataccatcactatcagcagtgtgaagaccatgccattaagcttagcatgttgaccaagaaagcttgtctgcatctgaatcccggcggaacctgtgtcagcataggttatggttacgctgacagggccagcgaaagcatcattggtgctatagcgcggcagttcaagttttcccgggtatgcaaaccgaaatcctcacttgaagagacggaagttctgtttgtattcattgggtacgatcgcaaggcccgtacgcacaatccttacaagctttcatcaaccttgaccaacatttatacaggttccagactccacgaagccggatgtgcaccctcatatcatgtggtgcgaggggatattgccacggccaccgaaggagtgattataaatgctgctaacagcaaaggacaacctggcggaggggtgtgcggagcgctgtataagaaattcccggaaagcttcgatttacagccgatcgaagtaggaaaagcgcgactggtcaaaggtgcagctaaacatatcattcatgccgtaggaccaaacttcaacaaagtttcggaggttgaaggtgacaaacagttggcagaggcttatgagtccatcgctaagattgtcaacgataacaattacaagtcagtagcgattccactgttgtccaccggcatcttttccgggaacaaagatcgactaacccaatcattgaaccatttgctgacagctttagacaccactgatgcagatgtagccatatactgcagggacaagaaatgggaaatgactctcaaggaagcagtggctaggagagaagcagtggaggagatatgcatatccgacgactcttcagtgacagaacctgatgcagagctggtgagggtgcatccgaagagttctttggctggaaggaagggctacagcacaagcgatggcaaaactttctcatatttggaagggaccaagtttcaccaggcggccaaggatatagcagaaattaatgccatgtggcccgttgcaacggaggccaatgagcaggtatgcatgtatatcctcggagaaagcatgagcagtattaggtcgaaatgccccgtcgaagagtcggaagcctccacaccacctagcacgctgccttgcttgtgcatccatgccatgactccagaaagagtacagcgcctaaaagcctcacgtccagaacaaattactgtgtgctcatcctttccattgccgaagtatagaatcactggtgtgcagaagatccaatgctcccagcctatattgttctcaccgaaagtgcctgcgtatattcatccaaggaagtatctcgtggaaacaccaccggtagacgagactccggagccatcggcagagaaccaatccacagaggggacacctgaacaaccaccacttataaccgaggatgagaccaggactagaacgcctgagccgatcatcatcgaagaggaagaagaggatagcataagtttgctgtcagatggcccgacccaccaggtgctgcaagtcgaggcagacattcacgggccgccctctgtatctagctcatcctggtccattcctcatgcatccgactttgatgtggacagtttatccatacttgacaccctggagggagctagcgtgaccagcggggcaacgtcagccgagactaactcttacttcgcaaagagtatggagtttctggcgcgaccggtgcctgcgcctcgaacagtattcaggaaccctccacatcccgctccgcgcacaagaacaccgtcacttgcacccagcagggcctgctcgagaaccagcctagtttccaccccgccaggcgtgaatagggtgatcactagagaggagctcgaggcgcttaccccgtcacgcactcctagcaggtcggtctcgagaaccagcctggtctccaacccgccaggcgtaaatagggtgattacaagagaggagtttgaggcgttcgtagcacaacaacaatgacggtttgatgcgggtgcatacatcttttcctccgacaccggtcaagggcatttacaacaaaaatcagtaaggcaaacggtgctatccgaagtggtgttggagaggaccgaattggagatttcgtatgccccgcgcctcgaccaagaaaaagaagaattactacgcaagaaattacagttaaatcccacacctgctaacagaagcagataccagtccaggaaggtggagaacatgaaagccataacagctagacgtattctgcaaggcctagggcattatttgaaggcagaaggaaaagtggagtgctaccgaaccctgcatcctgttcctttgtattcatctagtgtgaaccgtgccttttcaagccccaaggtcgcagtggaagcctgtaacgccatgttgaaagagaactttccgactgtggcttcttactgtattattccagagtacgatgcctatttggacatggttgacggagcttcatgctgcttagacactgccagtttttgccctgcaaagctgcgcagctttccaaagaaacactcctatttggaacccacaatacgatcggcagtgccttcagcgatccagaacacgctccagaacgtcctggcagctgccacaaaaagaaattgcaatgtcacgcaaatgagagaattgcccgtattggattcggcggcctttaatgtggaatgcttcaagaaatatgcgtgtaataatgaatattgggaaacgtttaaagaaaaccccatcaggcttactgaagaaaacgtggtaaattacattaccaaattaaaaggaccaaaagctgctgctctttttgcgaagacacataatttgaatatgttgcaggacataccaatggacaggtttgtaatggacttaaagagagacgtgaaagtgactccaggaacaaaacatactgaagaacggcccaaggtacaggtgatccaggctgccgatccgctagcaacagcgtatctgtgcggaatccaccgagagctggttaggagattaaatgcggtcctgcttccgaacattcatacactgtttgatatgtcggctgaagactttgacgctattatagccgagcacttccagcctggggattgtgttctggaaactgacatcgcgtcgtttgataaaagtgaggacgacgccatggctctgaccgcgttaatgattctggaagacttaggtgtggacgcagagctgttgacgctgattgaggcggctttcggcgaaatttcatcaatacatttgcccactaaaactaaatttaaattcggagccatgatgaaatctggaatgttcctcacactgtttgtgaacacagtcattaacattgtaatcgcaagcagagtgttgagagaacggctaaccggatcaccatgtgcagcattcattggagatgacaatatcgtgaaaggagtcaaatcggacaaattaatggcagacaggtgcgccacctggttgaatatggaagtcaagattatagatgctgtggtgggcgagaaagcgccttatttctgtggagggtttattttgtgtgactccgtgaccggcacagcgtgccgtgtggcagaccccctaaaaaggctgtttaagcttggcaaacctctggcagcagacgatgaacatgatgatgacaggagaagggcattgcatgaagagtcaacacgctggaaccgagtgggtattctttcagagctgtgcaaggcagtagaatcaaggtatgaaaccgtaggaacttccatcatagttatggccatgactactctagctagcagtgttaaatcattcagctacctgagaggggcccctataactctctacggctaacctgaatggactacgacatagtctagtccgccaagatgttcgtgttcctggtgctgctgcccctcgttagcagccagtgcgtgaatttcaccacccgcacccagctgccaccagcctacacaaacagcttcaccagaggagtgtattaccctgataaggtctttagatcctccgtcctgcattctacgcaggatctcttcttgccattcttcagcaacgtgacatggttccacgccatccacgtttctggcaccaacggcacaaagcgcttcgccaatcctgtgttgccgtttaacgacggcgtttacttcgccagcacagaaaagagcaacatcatccggggctggatcttcggcaccaccctggacagcaaaacccaaagcctgctcatcgtgaacaacgccaccaacgtggtgatcaaggtgtgcgagttccagttctgcaatgatccttttctgggcgtgtactatcacaagaacaacaagagctggatggaaagcgagttcagagtgtattctagcgccaacaactgcacctttgagtacgtgtcccagccctttcttatggacctggaaggcaagcagggcaacttcaagaatctgagagaattcgtgttcaagaacattgatggctacttcaagatctacagcaagcacacccctatcaacctggttcggggcctgccacaaggcttcagcgccctggaacctctggtggacctgcctatcggcatcaacatcacacggttccaaaccctgcaccggagctacctgacccccggcgacagcagcagcggctggaccgccggcgctgccgcctattacgtgggctacctgcaacctagaaccttcctgctgaaatacaacgagaacggcacaatcaccgacgccgtggactgtgccctggaccccctgtctgagacaaagtgtaccctgaagtctttcaccgtggagaagggcatctaccagaccagcaacttccgggtgcagcctacagaatctatagtgcggttccctaacatcaccaacctgtgtccttttggcgaggtgttcaacgccactcggttcgcctctgtctacgcctggaaccggaaacggatctctaattgcgtggccgattacagcgtcctgtataactccgccagtttcagcacattcaagtgctacggcgtgtcacccaccaagctgaacgatctgtgcttcaccaatgtgtacgccgatagtttcgtgatccggggcgatgaggtgcggcagatcgcccctggacagacaggcaatatcgccgactacaactacaagctgcctgacgacttcacaggctgtgtgatcgcatggaacagcaacaacctggacagcaaggtgggcggaaactacaactacctgtacagactgttcagaaagtccaacctgaagcctttcgagagagatatatctaccgagatctaccaggccggcagcacaccctgtaatggagtgaaaggctttaactgctacttccctctgcaaagctatggatttcaacctacatatggggttggctaccagccttacagagtggtggtccttagcttcgagctgctccatgcccctgccaccgtgtgcggacctaagaagtccaccaacctggtgaaaaacaagtgcgtgaactttaattttaacggcctgaccggaacaggagtgctgacagaaagcaacaaaaagttcctgcctttccagcagttcggcagagacattgccgacaccacagatgctgttagagacccccagacgctggaaatcctggatatcaccccctgctcttttggcggcgtgagcgtgatcaccccaggcacaaacacaagcaaccaggtggctgtgctgtaccagggcgtgaactgtacagaggtccctgtggcaatccacgccgatcagctgacccctacatggcgggtgtactccactggatctaacgtgttccagacaagggccggatgcctcatcggcgctgagcacgtgaacaattcttacgagtgcgacatccctattggagcgggcatctgcgccagctaccagacacagaccaatagccctcagcaagccgctagcgtggcctcccagagcatcatcgcctacaccatgagcctgggagtcgagaactctgtggcctacagcaacaacagcatcgctatccctaccaacttcaccatctctgtcaccaccgaaatcctgcccgtcagtatgaccaaaaccagcgtcgactgcaccatgtacatatgcggcgatagcaccgaatgcagcaacctgctgctgcagtatggctccttctgcacccaacttaacagagccctgactggcatcgccgtggagcaggacaagaatacccaggaggtgttcgcccaggtgaagcagatctacaagacacccccgatcaaggacttcggcggctttaatttctctcagatcctgccagacccatctaaaccctctaagcggagctttatcgaggacctgctgttcaacaaggtgactctggctgacgccggcttcatcaagcagtacggcgattgcctgggcgacattgctgctagagacctgatctgtgcccagaaattcaacggtcttactgtgctgcctcctctgctgacggatgagatgatcgcccagtacaccagcgccctgctggccggcaccatcacatccggctggacattcggcgccggcgcagccctgcagatcccttttgccatgcagatggcctaccggttcaacggaatcggagtgacacagaacgtgctctacgaaaatcagaagttgatcgccaaccagttcaacagcgccatcggcaagattcaggatagtctgagttccaccgccagcgccctgggaaagctgcaggacgtggtcaatcagaatgcccaagccctgaacaccctggtgaagcagctgagcagcaacttcggcgccatcagctctgtgctgaacgacatcctgagtagactggacaaggtggaagccgaagtgcagatcgacagattgatcaccggaagactgcaaagcctgcagacctacgtgacccagcagctgataagagctgctgaaatcagagccagcgctaatctggccgctaccaagatgagcgagtgcgttctgggccagtctaagagagtggacttctgcggaaaaggctaccacctgatgtcctttcctcagtctgccccccacggcgtggtgttcctgcacgtcacatacgtgcccgctcaagagaaaaacttcaccacggcccctgccatctgtcacgacggcaaggcccacttccccagagagggcgtgttcgtgagcaatggcacccactggtttgtgactcagagaaacttctacgagccacagattatcaccacagataacaccttcgtgtctggcaactgcgacgtggtgatcggcatcgtcaacaacacagtgtacgacccactgcaacctgagctggactcattcaaggaggaactggataagtacttcaagaatcacaccagccccgacgttgacctgggcgacatcagcggcattaacgcctctgtggtcaacatccagaaggaaatcgacagactgaatgaggtggccaagaatttgaacgagagcctgattgatctgcaggagctgggcaaatacgagcagtacatcaagtggccttggtacatctggctgggcttcatcgccgggctgatcgccatcgttatggtgacaatcatgctgtgttgcatgacaagctgttgtagctgcctgaaaggctgctgctcctgcggcagctgttgcaagtttgacgaagatgacagcgagcccgtgctgaaaggcgtcaagctgcactacacctgaggcgcgcccacccagcggccgcccgctacgccccaatgatccgaccagcaaaactcgatgtacttccgaggaactgatgtgcataatgcatcaggctggtacattagatccccgcttaccgcgggcaatatagcaacactaaaaactcgatgtacttccgaggaagcgcagtgcataatgctgcgcagtgttgccacataaccactatattaaccatttatctagcggacgccaaaaactcaatgtatttctgaggaagcgtggtgcataatgccacgcagcgtctgcataacttttattatttcttttattaatcaacaaaattttgtttttaacatttcaaaaaaaaaaaaaaaaaaaaaaaaaaaaaaaaaaaaagaagagcgtttaaacacgtgatatctggcctcatgggccttcctttcactgcccgctttccagtcgggaaacctgtcgtgccagctgcattaacatggtcatagctgtttccttgcgtattgggcgctctccgcttcctcgctcactgactcgctgcgctcggtcgttcgggtaaagcctggggtgcctaatgagcaaaaggccagcaaaaggccaggaaccgtaaaaaggccgcgttgctggcgtttttccataggctccgcccccctgacgagcatcacaaaaatcgacgctcaagtcagaggtggcgaaacccgacaggactataaagataccaggcgtttccccctggaagctccctcgtgcgctctcctgttccgaccctgccgcttaccggatacctgtccgcctttctcccttcgggaagcgtggcgctttctcatagctcacgctgtaggtatctcagttcggtgtaggtcgttcgctccaagctgggctgtgtgcacgaaccccccgttcagcccgaccgctgcgccttatccggtaactatcgtcttgagtccaacccggtaagacacgacttatcgccactggcagcagccactggtaacaggattagcagagcgaggtatgtaggcggtgctacagagttcttgaagtggtggcctaactacggctacactagaagaacagtatttggtatctgcgctctgctgaagccagttaccttcggaaaaagagttggtagctcttgatccggcaaacaaaccaccgctggtagcggtggtttttttgtttgcaggcagcagattacgcgcagaaaaaaaggatctcaagaagatcctttgatcttttctacggggtctgacgctcagtggaacgaaaactcacgttaagggattttggtcatgaatacacggtgcctgactgcgttagcaatttaactgtgataaactaccgcattaaagcttatcgatgataagctgtcaaacatgagaattcttagaaaaactcatcgagcatcaaatgaaactgcaatttattcatatcaggattatcaataccatatttttgaaaaagccgtttctgtaatgaaggagaaaactcaccgaggcagttccataggatggcaagatcctggtatcggtctgcgattccgactcgtccaacatcaatacaacctattaatttcccctcgtcaaaaataaggttatcaagtgagaaatcaccatgagtgacgactgaatccggtgagaatggcaaaagcttatgcatttctttccagacttgttcaacaggccagccattacgctcgtcatcaaaatcactcgcatcaaccaaaccgttattcattcgtgattgcgcctgagcgagacgaaatacgcgatcgctgttaaaaggacaattacaaacaggaatcgaatgcaaccggcgcaggaacactgccagcgcatcaacaatattttcacctgaatcaggatattcttctaatacctggaatgctgttttcccggggatcgcagtggtgagtaaccatgcatcatcaggagtacggataaaatgcttgatggtcggaagaggcataaattccgtcagccagtttagtctgaccatctcatctgtaacatcattggcaacgctacctttgccatgtttcagaaacaactctggcgcatcgggcttcccatacaatcgatagattgtcgcacctgattgcccgacattatcgcgagcccatttatacccatataaatcagcatccatgttggaatttaatcgcggcctcgagcaagacgtttcccgttgaatatggctcataacaccccttgtattactgtttatgtaagcagacagttttattgttcatgagcggatacatatttgaatgtatttagaaaaataaacaaataggggttccgcgcacatttccccgaaaagtgccacctaaattgtaagcgttaatattttgttaaaattcgcgttaaatttttgttaaatcagctcattttttaaccaataggccgaaatcggcaaaatcccttataaatcaaaagaatagaccgagatagggttgagtggccgctacagggcgctcccattcgccattcaggctgcgcaactgttgggaagggcgtttcggtgcgggcctcttcgctattacgccagctggcgaaagggggatgtgctgcaaggcgattaagttgggtaacgccagggttttcccagtcacacgcgtaatacgactcactatag

SEQ ID NO: 29 - DNA, 45 bp, Venezuelan equine encephalitis virus
  source 1..45: mol_type = other DNA
gataggcggcgcatgagagaagcccagaccaattacctacccaaa

SEQ ID NO: 30 - DNA, 341 bp, Sindbis virus
  source 1..341: mol_type = other DNA
ggcgcgcccacccagcggccgcccgctacgccccaatgatccgaccagcaaaactcgatgtacttccgaggaactgatgtgcataatgcatcaggctggtacattagatccccgcttaccgcgggcaatatagcaacactaaaaactcgatgtacttccgaggaagcgcagtgcataatgctgcgcagtgttgccacataaccactatattaaccatttatctagcggacgccaaaaactcaatgtatttctgaggaagcgtggtgcataatgccacgcagcgtctgcataacttttattatttcttttattaatcaacaaaattttgtttttaacatttc

SEQ ID NO: 31 - DNA, 10 bp, synthetic construct
  misc_feature 1..10: note = GC-rich element
  source 1..10: mol_type = other DNA
ccccggcgcc

SEQ ID NO: 32 - skipped

SEQ ID NO: 33 - DNA, 20 bp, synthetic construct
  misc_feature 1..20: note = GC-rich element
  source 1..20: mol_type = other DNA
gcgccccgcggcgccccgcg

SEQ ID NO: 34 - DNA, 24 bp, synthetic construct
  misc_feature 1..24: note = Histone stem loop sequence
  source 1..24: mol_type = other DNA
caaaggctcttttcagagccacca

SEQ ID NO: 35-36 - skipped (2 entries)

SEQ ID NO: 37 - DNA, 36 bp, synthetic construct
  misc_feature 1..36: note = poly-a sequence
  source 1..36: mol_type = other DNA
aaaaaaaaaaaaaaaaaaaaaaaaaaaaaaaaaaaa